European Patent Specification EP 3 466 446 B1, published December 27, 2023. Title: Screening and iOrgans. Applicant: ADVANCED TELECOMMUNICATIONS RESEARCH INSTITUTE INTERNATIONAL. The sequence listing filed with the application follows.

SEQUENCE LISTING (2017 sequences)

SEQ ID NO: 1 - protein, 286 aa, Homo sapiens
MALVLILQLLTLWPLCHTDITPSVAIIVPPASYHPKPWLGAQPATVVTPGVNVTLRCRAPQPAWRFGLFKPGEIAPLLFRDVSSELAEFFLEEVTPAQGGSYRCCYRRPDWGPGVWSQPSDVLELLVTEELPRPSLVALPGPVVGPGANVSLRCAGRLRNMSFVLYREGVAAPLQYRHSAQPWADFTLLGARAPGTYSCYYHTPSAPYVLSQRSEVLVISWEGEGPEARPASSAPGMQAPGPPPSDPGAQAPSLSSFRPRGLVLQPLLPQTQDSWDPAPPPSDPGV

SEQ ID NO: 2 - protein, 459 aa, Artificial Sequence
  Oscar-Fc fusion
MALVLILQLLTLWPLCHTDITPSVAIIVPPASYHPKPWLGAQPATVVTPGVNVTLRCRAPQPAWRFGLFKPGEIAPLLFRDVSSELAEFFLEEVTPAQGGSYRCCYRRPDWGPGVWSQPSDVLELLVTEELPRPSLVALPGPVVGPGANVSLRCAGRLRNMSFVLYREGVAAPLQYRHSAQPWADFTLLGARAPGTYSCYYHTPSAPYVLSQRSEVLVISWEGEGPEARPASDKTHTCPPCPAPELLGGPSVFLFPPKPKDTLMISRTPEVTCVVVDVSHEDPEVKFNWYVDGVEVHNAKTKPREEQYNSTYRVVSVLTVLHQDWLNGKEYKCKVSNKALPAPIEKTISKAKGQPREPQVYTLPPSREEMTKNQVSLTCLVKGFYPSDIAVEWESNGQPENNYKTTPPVLDSDGSFFLYSKLTVDKSRWQQGNVFSCSVMHEALHNHYTQKSLSLSPGK

SEQ ID NO: 3 - protein, 271 aa, Mus musculus
MVLSLILQLSTLCELSLPWPACRADFTPTAPLASYPQPWLGAHPAAVVTPGINVTLTCRAPQSAWRFALFKSGLVTPLLLRDVSVELAEFFLEEVTPAQGGSYHCRYRKTDWGPGVWSQPSNVLELLVTDQLPRPSLVALPGPVVAPGANVSLRCAGRIPGMSFALYRVGVATPLQYIDSVQPWADFLLIGTHTPGTYCCYYHTPSAPYVLSQRSQPLVISFEGSGSLDYTQGNLIRLGLAGMVLICLGIIVTCDWHSRSSAFDGLLPQQN

SEQ ID NO: 4 - protein, 462 aa, Artificial Sequence
  Oscar-Fc fusion
MVLSLILQLSTLCELSLPWPACRADFTPTAPLASYPQPWLGAHPAAVVTPGINVTLTCRAPQSAWRFALFKSGLVTPLLLRDVSVELAEFFLEEVTPAQGGSYHCRYRKTDWGPGVWSQPSNVLELLVTDQLPRPSLVALPGPVVAPGANVSLRCAGRIPGMSFALYRVGVATPLQYIDSVQPWADFLLIGTHTPGTYCCYYHTPSAPYVLSQRSQPLVISFEGSGSLDYTQGNLDKTHTCPPCPAPELLGGPSVFLFPPKPKDTLMISRTPEVTCVVVDVSHEDPEVKFNWYVDGVEVHNAKTKPREEQYNSTYRVVSVLTVLHQDWLNGKEYKCKVSNKALPAPIEKTISKAKGQPREPQVYTLPPSREEMTKNQVSLTCLVKGFYPSDIAVEWESNGQPENNYKTTPPVLDSDGSFFLYSKLTVDKSRWQQGNVFSCSVMHEALHNHYTQKSLSLSPGK

SEQ ID NO: 5 - DNA, 1601 bp, Artificial Sequence
  Oscar-Fc
aagcttgccaccatggccctcgtgcttatcctccaacttctcacgctttggcctctgtgccacaccgacattactccgtctgttgcgataattgtccctcccgcctcttatcaccctaaaccttggctgggcgcacagccagctactgtggttactcctggggtgaacgtaacactgcgctgccgtgctcctcagcccgcctggagatttgggttgtttaagcccggagagatagcaccactgctgtttcgggatgtgtcctcagagctggctgagttcttcctggaagaggtcactcctgcccaaggaggcagctatcggtgctgttataggcggccggattggggacccggcgtttggtcccaaccatctgatgtgctcgaactgcttgtgacagaagagctgcccagacctagcttggtagccttgcccggtcctgtcgtcggacctggtgccaatgtttctcttcgatgtgccggaaggctgcgcaatatgtcctttgtactgtatagggagggagtagccgcacctctgcagtataggcatagcgctcagccctgggcggattttactctgcttggtgccagagcacccgggacctattcctgctactaccacactccttccgcaccctacgtcctgtcacagagatcagaagtgctcgtgatctcctgggagggagaaggcccagaagccgacaaaactcacacatgcccaccgtgcccaggtaagccagcccaggcctcgccctccagctcaaggcgggacaggtgccctagagtagcctgcatccagggacaggccccagccgggtgctgacacgtccacctccatctcttcctcagcacctgaactcctggggggaccgtcagtcttcctcttccccccaaaacccaaggacaccctcatgatctcccggacccctgaggtcacatgcgtggtggtggacgtgagccacgaagaccctgaggtcaagttcaactggtacgtggacggcgtggaggtgcataatgccaagacaaagccgcgggaggagcagtacaacagcacgtaccgtgtggtcagcgtcctcaccgtcctgcaccaggactggctgaatggcaaggagtacaagtgcaaggtctccaacaaagccctcccagcccccatcgagaaaaccatctccaaagccaaaggtgggacccgtggggtgcgagggccacatggacagaggccggctcggcccaccctctgccctgagagtgactgctgtaccaacctctgtccctacagggcagccccgagaaccacaggtgtacaccctgcccccatcccgggatgagctgaccaagaaccaggtcagcctgacctgcctggtcaaaggcttctatcccagcgacatcgccgtggagtgggagagcaatgggcagccggagaacaactacaagaccacgcctcccgtgctggactccgacggctccttcttcctctacagcaagctcaccgtggacaagagcaggtggcagcaggggaacgtcttctcatgctccgtgatgcatgaggctctgcacaaccactacacgcagaagagcctctccctgtctccgggtaaatgatctaga

SEQ ID NO: 6 - DNA, 21 bp, Artificial Sequence
  primer
aagaccttgagtagttgccca

SEQ ID NO: 7 - DNA, 21 bp, Artificial Sequence
  primer
tgctcgatcctacgtttgcag

SEQ ID NO: 8 - DNA, 20 bp, Artificial Sequence
  primer
aggagccatgactcgaaggt

SEQ ID NO: 9 - DNA, 21 bp, Artificial Sequence
  primer
gctcaccaggtagtgatgctt

SEQ ID NO: 10 - DNA, 20 bp, Artificial Sequence
  primer
accccagcatggaaacaaag

SEQ ID NO: 11 - DNA, 25 bp, Artificial Sequence
  primer
aagaatggtattgaagtcatctgtc

SEQ ID NO: 12 - DNA, 21 bp, Artificial Sequence
  primer
accccgtgaagaaaatcagaa

SEQ ID NO: 13 - DNA, 20 bp, Artificial Sequence
  primer
taacaggcggtcttggttgg

SEQ ID NO: 14 - DNA, 21 bp, Artificial Sequence
  primer
tggtggtcctgtttacagtgg

SEQ ID NO: 15 - DNA, 21 bp, Artificial Sequence
  primer
ttctgaagttcttcacggggt

SEQ ID NO: 16 - DNA, 24 bp, Artificial Sequence
  primer
cctacgaagactcaaattctcagc

SEQ ID NO: 17 - DNA, 19 bp, Artificial Sequence
  primer
gaggaccatggtggtgtcc

SEQ ID NO: 18 - DNA, 20 bp, Artificial Sequence
  primer
gctcggtgaccctggtcttt

SEQ ID NO: 19 - DNA, 20 bp, Artificial Sequence
  primer
aatgtgaggcgggtggaact

SEQ ID NO: 20 - DNA, 20 bp, Mus musculus
acagctggagtatcagcgac

SEQ ID NO: 21 - DNA, 20 bp, Mus musculus
gctcacagagagtcgacagc

SEQ ID NO: 22 - DNA, 146 bp, Artificial Sequence
  ssODN
gccaaggatccacacacaggggagggacagctcacagagagtcgacagctggagtatcagcctcagaagaactcgtcaagaagtcacgacaggaccatggtgggcactctccgtggagctgaggaaaaggttgaccctgccttttt

SEQ ID NO: 23 - DNA, 146 bp, Artificial Sequence
  ssODN
atagccctcagcccagccaaggatccacacacaggggagggacagctcacagagagtcgacctcagaagaactcgtcaagaagtcacagctggagtatcagcgacaggaccatggtgggcactctccgtggagctgaggaaaaggt

SEQ ID NO: 24 - DNA, 20 bp, Artificial Sequence
  primer
ctacttagcgacaacgtcct

SEQ ID NO: 25 - DNA, 20 bp, Artificial Sequence
  primer
gccttggggtttgaaggttt

SEQ ID NO: 26 - DNA, 20 bp, Artificial Sequence
  primer
cagaggctatgactgttcca

SEQ ID NO: 27 - DNA, 20 bp, Artificial Sequence
  primer
ggcagggtcaaccttttcct

SEQ ID NO: 28 - DNA, 20 bp, Artificial Sequence
  primer
agggacagctcacagagagt

SEQ ID NO: 29 - DNA, 20 bp, Artificial Sequence
  primer
gctcggtgaccctggtcttt

SEQ ID NO: 30 - DNA, 20 bp, Artificial Sequence
  primer
aatgtgaggcgggtggaact

SEQ ID NO: 31 - DNA, 20 bp, Artificial Sequence
  primer
cgggcatgagttttgcactg

SEQ ID NO: 32 - DNA, 21 bp, Artificial Sequence
  primer
tgggtatagtccaaggagcca

SEQ ID NO: 33 - DNA, 20 bp, Artificial Sequence
  primer
aggagccatgactcgaaggt

SEQ ID NO: 34 - DNA, 21 bp, Artificial Sequence
  primer
gctcaccaggtagtgatgctt

SEQ ID NO: 35 - DNA, 23 bp, Homo sapiens
caacacaaattagccgggcgtgg

SEQ ID NO: 36 - DNA, 23 bp, Homo sapiens
agctcaacatcggctcgtcctgg

SEQ ID NO: 37 - DNA, 23 bp, Homo sapiens
gtcactccggagcgacttctagg

SEQ ID NO: 38 - DNA, 23 bp, Homo sapiens
ccacgcaggtccgcaaagtcagg

SEQ ID NO: 39 - DNA, 23 bp, Homo sapiens
ggactattttgttccgccttagg

SEQ ID NO: 40 - DNA, 23 bp, Homo sapiens
gtctcgaacttcccgacctcagg

SEQ ID NO: 41 - DNA, 23 bp, Homo sapiens
gcgagggtctggcacgtaatagg

SEQ ID NO: 42 - DNA, 23 bp, Homo sapiens
cgccttaggtgggtcgcagcagg

SEQ ID NO: 43 - DNA, 23 bp, Homo sapiens
acctcgtgatccgcccgcctcgg

SEQ ID NO: 44 - DNA, 23 bp, Homo sapiens
aatcgcttgaactcgggagtcgg

SEQ ID NO: 45 - DNA, 23 bp, Homo sapiens
tcttggtctttcagtcggactgg

SEQ ID NO: 46 - DNA, 23 bp, Homo sapiens
cctgactttgcggacctgcgtgg

SEQ ID NO: 47 - DNA, 23 bp, Homo sapiens
tctcagcctagaagtcgctccgg

SEQ ID NO: 48 - DNA, 23 bp, Homo sapiens
cgcttgaactcgggagtcggagg

SEQ ID NO: 49 - DNA, 23 bp, Homo sapiens
ggagtgcaatggcgcgatctcgg

SEQ ID NO: 50 - DNA, 23 bp, Homo sapiens
atgttgagctgagacctcgaagg

SEQ ID NO: 51 - DNA, 23 bp, Homo sapiens
acaaccgcgcccggcctagaggg

SEQ ID NO: 52 - DNA, 23 bp, Homo sapiens
agactaaggagattccacgcagg

SEQ ID NO: 53 - DNA, 23 bp, Homo sapiens
aacaaccgcgcccggcctagagg

SEQ ID NO: 54 - DNA, 23 bp, Homo sapiens
ggatgagacctagcgcttccagg

SEQ ID NO: 55 - DNA, 23 bp, Homo sapiens
caaccgcgcccggcctagagggg

SEQ ID NO: 56 - DNA, 23 bp, Homo sapiens
tattttgttccgccttaggtggg

SEQ ID NO: 57 - DNA, 23 bp, Homo sapiens
gagaatggcgtgaacccgggagg

SEQ ID NO: 58 - DNA, 23 bp, Homo sapiens
aatgactaacctgtccttcgagg

SEQ ID NO: 59 - DNA, 23 bp, Homo sapiens
tagcccctctaggccgggcgcgg

SEQ ID NO: 60 - DNA, 23 bp, Homo sapiens
ggcgggcggatcacgaggtcagg

SEQ ID NO: 61 - DNA, 23 bp, Homo sapiens
cgctaggtctcatcccagatggg

SEQ ID NO: 62 - DNA, 23 bp, Homo sapiens
ctgctgcgacccacctaaggcgg

SEQ ID NO: 63 - DNA, 23 bp, Homo sapiens
cggctcgtcctggaagcgctagg

SEQ ID NO: 64 - DNA, 23 bp, Homo sapiens
cagaaagctcctaacccatctgg

SEQ ID NO: 65 - DNA, 23 bp, Homo sapiens
gggggttcagtcataacctgtgg

SEQ ID NO: 66 - DNA, 23 bp, Homo sapiens
ctattttgttccgccttaggtgg

SEQ ID NO: 67 - DNA, 23 bp, Homo sapiens
agcaggaggactagtcactccgg

SEQ ID NO: 68 - DNA, 23 bp, Homo sapiens
gagctgagacctcgaaggacagg

SEQ ID NO: 69 - DNA, 23 bp, Homo sapiens
cacaaattagccgggcgtggtgg

SEQ ID NO: 70 - DNA, 23 bp, Homo sapiens
gcgcccgtagtcccagctactgg

SEQ ID NO: 71 - DNA, 23 bp, Homo sapiens
ctgccaacatggcacagcgaggg

SEQ ID NO: 72 - DNA, 23 bp, Homo sapiens
aacatggcacagcgagggtctgg

SEQ ID NO: 73 - DNA, 23 bp, Homo sapiens
tcgaggtctcagctcaacatcgg

SEQ ID NO: 74 - DNA, 23 bp, Homo sapiens
gcgctaggtctcatcccagatgg

SEQ ID NO: 75 - DNA, 23 bp, Homo sapiens
gcaggagaatggcgtgaacccgg

SEQ ID NO: 76 - DNA, 23 bp, Homo sapiens
aaaattagcccctctaggccggg

SEQ ID NO: 77 - DNA, 23 bp, Homo sapiens
ggtctcatcccagatgggttagg

SEQ ID NO: 78 - DNA, 23 bp, Homo sapiens
aatggcgtgaacccgggaggcgg

SEQ ID NO: 79 - DNA, 23 bp, Homo sapiens
gaaaaattagccggctgtggagg

SEQ ID NO: 80 - DNA, 23 bp, Homo sapiens
caggagaatcgcttgaactcggg

SEQ ID NO: 81 - DNA, 23 bp, Homo sapiens
cgacttctaggctgagactaagg

SEQ ID NO: 82 - DNA, 23 bp, Homo sapiens
agaaagctcctaacccatctggg

SEQ ID NO: 83 - DNA, 23 bp, Homo sapiens
agtgatctgagctataatggcgg

SEQ ID NO: 84 - DNA, 23 bp, Homo sapiens
caggagaatggcgtgaacccggg

SEQ ID NO: 85 - DNA, 23 bp, Homo sapiens
aaagaaaaattagccggctgtgg

SEQ ID NO: 86 - DNA, 23 bp, Homo sapiens
aaaaattagcccctctaggccgg

SEQ ID NO: 87 - DNA, 23 bp, Homo sapiens
ctcctgctgcgacccacctaagg

SEQ ID NO: 88 - DNA, 23 bp, Homo sapiens
tcaggagatctagaccatcctgg

SEQ ID NO: 89 - DNA, 23 bp, Homo sapiens
caaggcgggtggatcacctgagg

SEQ ID NO: 90 - DNA, 23 bp, Homo sapiens
cctcgctgtgccatgttggcagg

SEQ ID NO: 91 - DNA, 23 bp, Homo sapiens
gtcatagccctatggcactgtgg

SEQ ID NO: 92 - DNA, 23 bp, Homo sapiens
aattagccgggcgtggtggtggg

SEQ ID NO: 93 - DNA, 23 bp, Homo sapiens
agacgggggtttctccatgttgg

SEQ ID NO: 94 - DNA, 23 bp, Homo sapiens
caggcgcgcgcctccacagccgg

SEQ ID NO: 95 - DNA, 23 bp, Homo sapiens
atgggttaggagctttctgcggg

SEQ ID NO: 96 - DNA, 23 bp, Homo sapiens
tcgatcaattaatcacagcaagg

SEQ ID NO: 97 - DNA, 23 bp, Homo sapiens
gaacaaagatggagccgtggagg

SEQ ID NO: 98 - DNA, 23 bp, Homo sapiens
ttaagtgatctgagctataatgg

SEQ ID NO: 99 - DNA, 23 bp, Homo sapiens
cccttgctgtgattgattgatgg

SEQ ID NO: 100 - DNA, 23 bp, Homo sapiens
cttaggtgggtcgcagcaggagg

SEQ ID NO: 101 - DNA, 23 bp, Homo sapiens
acagtatcacaccaagagcctgg

SEQ ID NO: 102 - DNA, 23 bp, Homo sapiens
agaccctcgctgtgccatgttgg

SEQ ID NO: 103 - DNA, 23 bp, Homo sapiens
cctgccaacatggcacagcgagg

SEQ ID NO: 104 - DNA, 23 bp, Homo sapiens
gatcacttaagaaactgacctgg

SEQ ID NO: 105 - DNA, 23 bp, Homo sapiens
cttaagaaactgacctggtctgg

SEQ ID NO: 106 - DNA, 23 bp, Homo sapiens
ccgactgaaagaccaagaccagg

SEQ ID NO: 107 - DNA, 23 bp, Homo sapiens
tctagaaacaaatactagtcagg

SEQ ID NO: 108 - DNA, 23 bp, Homo sapiens
attagcacctgttaagtgccagg

SEQ ID NO: 109 - DNA, 23 bp, Homo sapiens
ggcactgtggaaaaattagcagg

SEQ ID NO: 110 - DNA, 23 bp, Homo sapiens
aaactgacctggtctgggccagg

SEQ ID NO: 111 - DNA, 23 bp, Homo sapiens
gccttagcctccccagtagctgg

SEQ ID NO: 112 - DNA, 23 bp, Homo sapiens
tccatcaatcaatcacagcaagg

SEQ ID NO: 113 - DNA, 23 bp, Homo sapiens
cgatcaattaatcacagcaaggg

SEQ ID NO: 114 - DNA, 23 bp, Homo sapiens
cctggtcttggtctttcagtcgg

SEQ ID NO: 115 - DNA, 23 bp, Homo sapiens
ctgctgcttgagagcagtaacgg

SEQ ID NO: 116 - DNA, 23 bp, Homo sapiens
tttcaatcacagcaagggcctgg

SEQ ID NO: 117 - DNA, 23 bp, Homo sapiens
caggctgctcttgaactcttggg

SEQ ID NO: 118 - DNA, 23 bp, Homo sapiens
agatggagccgtggaggtaaagg

SEQ ID NO: 119 - DNA, 23 bp, Homo sapiens
gctactggggaggctaaggcagg

SEQ ID NO: 120 - DNA, 23 bp, Homo sapiens
aaattagccgggcgtggtggtgg

SEQ ID NO: 121 - DNA, 23 bp, Homo sapiens
gcctcagcctcctgaatagctgg

SEQ ID NO: 122 - DNA, 23 bp, Homo sapiens
aatcaatcacagcaagggcctgg

SEQ ID NO: 123 - DNA, 23 bp, Homo sapiens
gatgggttaggagctttctgcgg

SEQ ID NO: 124 - DNA, 23 bp, Homo sapiens
ttcttttttaggagagacggggg

SEQ ID NO: 125 - DNA, 23 bp, Homo sapiens
gcactgtggaaaaattagcaggg

SEQ ID NO: 126 - DNA, 23 bp, Homo sapiens
agaaacaaatactagtcaggagg

SEQ ID NO: 127 - DNA, 23 bp, Homo sapiens
cgtagtcccagctactggggagg

SEQ ID NO: 128 - DNA, 23 bp, Homo sapiens
aacaaatactagtcaggaggtgg

SEQ ID NO: 129 - DNA, 23 bp, Homo sapiens
ttaagaaactgacctggtctggg

SEQ ID NO: 130 - DNA, 23 bp, Homo sapiens
ccttagcctccccagtagctggg

SEQ ID NO: 131 - DNA, 23 bp, Homo sapiens
agataaaaattagcccctctagg

SEQ ID NO: 132 - DNA, 23 bp, Homo sapiens
ccatcaatcaatcacagcaaggg

SEQ ID NO: 133 - DNA, 23 bp, Homo sapiens
gaggtaaaggaagtggtgtcagg

SEQ ID NO: 134 - DNA, 23 bp, Homo sapiens
cactgcaagctccgcctcccggg

SEQ ID NO: 135 - DNA, 23 bp, Homo sapiens
taattgatcgattgatagattgg

SEQ ID NO: 136 - DNA, 23 bp, Homo sapiens
aaatacaacacaaattagccggg

SEQ ID NO: 137 - DNA, 23 bp, Homo sapiens
tccctctgtgcctgccaacatgg

SEQ ID NO: 138 - DNA, 23 bp, Homo sapiens
gttaaataaatgaacaccacagg

SEQ ID NO: 139 - DNA, 23 bp, Homo sapiens
gttagtcattcaccttctcccgg

SEQ ID NO: 140 - DNA, 23 bp, Homo sapiens
caccgcgcctggcccagaccagg

SEQ ID NO: 141 - DNA, 23 bp, Homo sapiens
gttagtcattcaccttctcccgg

SEQ ID NO: 142 - DNA, 23 bp, Homo sapiens
aaaagaaactgacctggtcttgg

SEQ ID NO: 143 - DNA, 23 bp, Homo sapiens
gcaagagtctggcacataatagg

SEQ ID NO: 144 - DNA, 23 bp, Homo sapiens
aagaaactgagcccgggagaagg

SEQ ID NO: 145 - DNA, 23 bp, Homo sapiens
caagcgcaagcctgactttgcgg

SEQ ID NO: 146 - DNA, 23 bp, Homo sapiens
ctggtctgggccaggcgcggtgg

SEQ ID NO: 147 - DNA, 23 bp, Homo sapiens
aatcaatgacagcaagagtctgg

SEQ ID NO: 148 - DNA, 23 bp, Homo sapiens
ccaggctgctcttgaactcttgg

SEQ ID NO: 149 - DNA, 23 bp, Homo sapiens
ttagtcattcaccttctcccggg

SEQ ID NO: 150 - DNA, 23 bp, Homo sapiens
tcactgcaagctccgcctcccgg

SEQ ID NO: 151 - DNA, 23 bp, Homo sapiens
aaatactagtcaggaggtggagg

SEQ ID NO: 152 - DNA, 23 bp, Homo sapiens
ctatctttcaatcacagcaaggg

SEQ ID NO: 153 - DNA, 23 bp, Homo sapiens
caagagttcaagagcagcctggg

SEQ ID NO: 154 - DNA, 23 bp, Homo sapiens
gccatgttggcaggcacagaggg

SEQ ID NO: 155 - DNA, 23 bp, Homo sapiens
tgccatgttggcaggcacagagg

SEQ ID NO: 156 - DNA, 23 bp, Homo sapiens
acagacgaagaaactgagcccgg

SEQ ID NO: 157 - DNA, 23 bp, Homo sapiens
tctatctttcaatcacagcaagg

SEQ ID NO: 158 - DNA, 23 bp, Homo sapiens
ccaagagttcaagagcagcctgg

SEQ ID NO: 159 - DNA, 23 bp, Homo sapiens
cccagctactggggaggctaagg

SEQ ID NO: 160 - DNA, 23 bp, Homo sapiens
tttcttttttaggagagacgggg

SEQ ID NO: 161 - DNA, 23 bp, Homo sapiens
actgtggaaaaattagcaggggg

SEQ ID NO: 162 - DNA, 23 bp, Homo sapiens
tgtaatcccagctattcaggagg

SEQ ID NO: 163 - DNA, 23 bp, Homo sapiens
caccacttcctttacctccacgg

SEQ ID NO: 164 - DNA, 23 bp, Homo sapiens
cgcccgtagtcccagctactggg

SEQ ID NO: 165 - DNA, 23 bp, Homo sapiens
cactgtggaaaaattagcagggg

SEQ ID NO: 166 - DNA, 23 bp, Homo sapiens
ccaagagcctggcacataatagg

SEQ ID NO: 167 - DNA, 23 bp, Homo sapiens
gccgaggcgggcggatcacgagg

SEQ ID NO: 168 - DNA, 23 bp, Homo sapiens
caggcgtgaacaaccgcgcccgg

SEQ ID NO: 169 - DNA, 23 bp, Homo sapiens
attaacaccaattatgtgccagg

SEQ ID NO: 170 - DNA, 23 bp, Homo sapiens
gcaagggcctggcacataattgg

SEQ ID NO: 171 - DNA, 23 bp, Homo sapiens
cctcagcctcctgaatagctggg

SEQ ID NO: 172 - DNA, 23 bp, Homo sapiens
atggtctcactctatcacccagg

SEQ ID NO: 173 - DNA, 23 bp, Homo sapiens
agccgtggaggtaaaggaagtgg

SEQ ID NO: 174 - DNA, 23 bp, Homo sapiens
gcctgtaatcccagctattcagg

SEQ ID NO: 175 - DNA, 23 bp, Homo sapiens
gcaagggcctggcacttaacagg

SEQ ID NO: 176 - DNA, 23 bp, Homo sapiens
gcaggagaatcgcttgaactcgg

SEQ ID NO: 177 - DNA, 23 bp, Homo sapiens
gacctggtctgggccaggcgcgg

SEQ ID NO: 178 - DNA, 23 bp, Homo sapiens
ctagaccatcctggctaacatgg

SEQ ID NO: 179 - DNA, 23 bp, Homo sapiens
gtgattgaaagatagatagatgg

SEQ ID NO: 180 - DNA, 23 bp, Homo sapiens
cagacgaagaaactgagcccggg

SEQ ID NO: 181 - DNA, 23 bp, Homo sapiens
aaaatacaacacaaattagccgg

SEQ ID NO: 182 - DNA, 23 bp, Homo sapiens
gcgggtggatcacctgaggtcgg

SEQ ID NO: 183 - DNA, 23 bp, Homo sapiens
cctattatgtgccaggctcttgg

SEQ ID NO: 184 - DNA, 23 bp, Homo sapiens
tcctgaatagctgggattacagg

SEQ ID NO: 185 - DNA, 23 bp, Homo sapiens
gcccgtagtcccagctactgggg

SEQ ID NO: 186 - DNA, 23 bp, Homo sapiens
ctcaggtgatccacccgccttgg

SEQ ID NO: 187 - DNA, 23 bp, Homo sapiens
aattaatcacagcaagggcctgg

SEQ ID NO: 188 - DNA, 23 bp, Homo sapiens
ttttcttttttaggagagacggg

SEQ ID NO: 189 - DNA, 23 bp, Homo sapiens
taatttttccacagtgccatagg

SEQ ID NO: 190 - DNA, 23 bp, Homo sapiens
ttgtatttttaagtagagacagg

SEQ ID NO: 191 - DNA, 23 bp, Homo sapiens
aatttttccacagtgccataggg

SEQ ID NO: 192 - DNA, 23 bp, Homo sapiens
cgggtggatcacctgaggtcggg

SEQ ID NO: 193 - DNA, 23 bp, Homo sapiens
actagtcaggaggtggaggcagg

SEQ ID NO: 194 - DNA, 23 bp, Homo sapiens
ttcatacataaactataaaatgg

SEQ ID NO: 195 - DNA, 23 bp, Homo sapiens
gggaggctaaggcaggagaatgg

SEQ ID NO: 196 - DNA, 23 bp, Homo sapiens
tgagtctagctctgtcgcccagg

SEQ ID NO: 197 - DNA, 23 bp, Homo sapiens
ctttgggaggccgaggcgggcgg

SEQ ID NO: 198 - DNA, 23 bp, Homo sapiens
caaaaaaaaagaaactgacctgg

SEQ ID NO: 199 - DNA, 23 bp, Homo sapiens
cgggcgcccaccaccacgcccgg

SEQ ID NO: 200 - DNA, 23 bp, Homo sapiens
ccggctaatttttcttttttagg

SEQ ID NO: 201 - DNA, 23 bp, Homo sapiens
tcatacataaactataaaatggg

SEQ ID NO: 202 - DNA, 23 bp, Homo sapiens
ttgaaagatagatagatggatgg

SEQ ID NO: 203 - DNA, 23 bp, Homo sapiens
cccagctattcaggaggctgagg

SEQ ID NO: 204 - DNA, 23 bp, Homo sapiens
tgtatttttaagtagagacaggg

SEQ ID NO: 205 - DNA, 23 bp, Homo sapiens
cctaaaaaagaaaaattagccgg

SEQ ID NO: 206 - DNA, 23 bp, Homo sapiens
catacataaactataaaatgggg

SEQ ID NO: 207 - DNA, 23 bp, Homo sapiens
atttgcacctattatgtgccagg

SEQ ID NO: 208 - DNA, 23 bp, Homo sapiens
agtttcttcgtctgtaaaatggg

SEQ ID NO: 209 - DNA, 23 bp, Homo sapiens
cgcgccattgcactccagcctgg

SEQ ID NO: 210 - DNA, 23 bp, Homo sapiens
gcgccattgcactccagcctggg

SEQ ID NO: 211 - DNA, 23 bp, Homo sapiens
ctttgggaggccaaggcgggtgg

SEQ ID NO: 212 - DNA, 23 bp, Homo sapiens
gctattcaggaggctgaggcagg

SEQ ID NO: 213 - DNA, 23 bp, Homo sapiens
tttttcttttttaggagagacgg

SEQ ID NO: 214 - DNA, 23 bp, Homo sapiens
aagatagatagatggatggatgg

SEQ ID NO: 215 - DNA, 23 bp, Homo sapiens
tatttatttattttttagacagg

SEQ ID NO: 216 - DNA, 23 bp, Homo sapiens
agggtttcaccatgttagccagg

SEQ ID NO: 217 - DNA, 23 bp, Homo sapiens
ctccccagtagctgggactacgg

SEQ ID NO: 218 - DNA, 23 bp, Homo sapiens
gcactttgggaggccgaggcggg

SEQ ID NO: 219 - DNA, 23 bp, Homo sapiens
ggagtgcagtggtgtgatctcgg

SEQ ID NO: 220 - DNA, 23 bp, Homo sapiens
cagtttcttcgtctgtaaaatgg

SEQ ID NO: 221 - DNA, 23 bp, Homo sapiens
tccccagtagctgggactacggg

SEQ ID NO: 222 - DNA, 23 bp, Homo sapiens
tttcaccatgttagccaggatgg

SEQ ID NO: 223 - DNA, 23 bp, Homo sapiens
ggggtttctccatgttggtcagg

SEQ ID NO: 224 - DNA, 23 bp, Homo sapiens
agtcaggaggtggaggcaggagg

SEQ ID NO: 225 - DNA, 23 bp, Homo sapiens
agcactttgggaggccgaggcgg

SEQ ID NO: 226 - DNA, 23 bp, Homo sapiens
tctagctctgtcgcccaggctgg

SEQ ID NO: 227 - DNA, 23 bp, Homo sapiens
agggtctcgctctgttgcccagg

SEQ ID NO: 228 - DNA, 23 bp, Homo sapiens
atttatttattttttagacaggg

SEQ ID NO: 229 - DNA, 23 bp, Homo sapiens
tgtgccactgcactccagcctgg

SEQ ID NO: 230 - DNA, 23 bp, Homo sapiens
ggagtctcgctctgtcgcccagg

SEQ ID NO: 231 - DNA, 23 bp, Homo sapiens
cacaccactgcactccagcctgg

SEQ ID NO: 232 - DNA, 23 bp, Homo sapiens
tttctccatgttggtcaggctgg

SEQ ID NO: 233 - DNA, 23 bp, Homo sapiens
tctcactctatcacccaggctgg

SEQ ID NO: 234 - DNA, 23 bp, Homo sapiens
cccagcactttgggaggccgagg

SEQ ID NO: 235 - DNA, 23 bp, Homo sapiens
cagtttctttttttttgagacgg

SEQ ID NO: 236 - DNA, 23 bp, Homo sapiens
cgagaccagcctgaccaacatgg

SEQ ID NO: 237 - DNA, 23 bp, Homo sapiens
tcgcccaggctggagtgcaatgg

SEQ ID NO: 238 - DNA, 23 bp, Homo sapiens
gcctcggcctcccaaagtgctgg

SEQ ID NO: 239 - DNA, 23 bp, Homo sapiens
tctcgctctgtcgcccaggctgg

SEQ ID NO: 240 - DNA, 23 bp, Homo sapiens
acaccactgcactccagcctggg

SEQ ID NO: 241 - DNA, 23 bp, Homo sapiens
gtgccactgcactccagcctggg

SEQ ID NO: 242 - DNA, 23 bp, Homo sapiens
cctcggcctcccaaagtgctggg

SEQ ID NO: 243 - DNA, 23 bp, Homo sapiens
gcactttgggaggccaaggcggg

SEQ ID NO: 244 - DNA, 23 bp, Homo sapiens
cccagcactttgggaggccaagg

SEQ ID NO: 245 - DNA, 23 bp, Homo sapiens
tcgcccaggctggagtgcagtgg

SEQ ID NO: 246 - DNA, 23 bp, Homo sapiens
agcactttgggaggccaaggcgg

SEQ ID NO: 247 - DNA, 23 bp, Homo sapiens
gccttggcctcccaaagtgctgg

SEQ ID NO: 248 - DNA, 23 bp, Homo sapiens
attagcacctattatgtgccagg

SEQ ID NO: 249 - DNA, 23 bp, Homo sapiens
cgcctgtaatcccagcactttgg

SEQ ID NO: 250 - DNA, 23 bp, Homo sapiens
ccttggcctcccaaagtgctggg

SEQ ID NO: 251 - DNA, 23 bp, Homo sapiens
cgcctgtaatcccagcactttgg

SEQ ID NO: 252 - DNA, 23 bp, Homo sapiens
tcacccaggctggagtgcagtgg

SEQ ID NO: 253 - DNA, 23 bp, Homo sapiens
tgtaatcccagcactttgggagg

SEQ ID NO: 254 - DNA, 23 bp, Homo sapiens
gcctgtaatcccagcactttggg

SEQ ID NO: 255 - DNA, 23 bp, Homo sapiens
tgtaatcccagcactttgggagg

SEQ ID NO: 256 - DNA, 23 bp, Homo sapiens
gcctgtaatcccagcactttggg

SEQ ID NO: 257 - DNA, 23 bp, Homo sapiens
caggcgtgagccaccgcgcctgg

SEQ ID NO: 258 - DNA, 23 bp, Homo sapiens
tcccaaagtgctgggattacagg

SEQ ID NO: 259 - DNA, 23 bp, Homo sapiens
atttacggaagagagtatcgagg

SEQ ID NO: 260 - DNA, 23 bp, Homo sapiens
tacggaagagagtatcgaggtgg

SEQ ID NO: 261 - DNA, 23 bp, Homo sapiens
gggcagatacccgctagagctgg

SEQ ID NO: 262 - DNA, 23 bp, Homo sapiens
cggaagagagtatcgaggtgggg

SEQ ID NO: 263 - DNA, 23 bp, Homo sapiens
tagcgggtatctgcccaccatgg

SEQ ID NO: 264 - DNA, 23 bp, Homo sapiens
acggaagagagtatcgaggtggg

SEQ ID NO: 265 - DNA, 23 bp, Homo sapiens
gatactctcttccgtaaatgagg

SEQ ID NO: 266 - DNA, 23 bp, Homo sapiens
tcttccgtaaatgaggatctggg

SEQ ID NO: 267 - DNA, 23 bp, Homo sapiens
ctcttccgtaaatgaggatctgg

SEQ ID NO: 268 - DNA, 23 bp, Homo sapiens
cgtaaatgaggatctgggtctgg

SEQ ID NO: 269 - DNA, 23 bp, Homo sapiens
gtgactgtgtcatagccctatgg

SEQ ID NO: 270 - DNA, 23 bp, Homo sapiens
gtatcgaggtgggggcctgtggg

SEQ ID NO: 271 - DNA, 23 bp, Homo sapiens
gtcatagccctatggcactgtgg

SEQ ID NO: 272 - DNA, 23 bp, Homo sapiens
gctatgacacagtcacccacagg

SEQ ID NO: 273 - DNA, 23 bp, Homo sapiens
gagagggtgcgaccaagccctgg

SEQ ID NO: 274 - DNA, 23 bp, Homo sapiens
ggcactgtggaaaaattagcagg

SEQ ID NO: 275 - DNA, 23 bp, Homo sapiens
ggaagagagtatcgaggtggggg

SEQ ID NO: 276 - DNA, 23 bp, Homo sapiens
tacccgctagagctggagccagg

SEQ ID NO: 277 - DNA, 23 bp, Homo sapiens
cagacccagatcctcatttacgg

SEQ ID NO: 278 - DNA, 23 bp, Homo sapiens
agtatcgaggtgggggcctgtgg

SEQ ID NO: 279 - DNA, 23 bp, Homo sapiens
gcactgtggaaaaattagcaggg

SEQ ID NO: 280 - DNA, 23 bp, Homo sapiens
cagctggaggatcagcaccaggg

SEQ ID NO: 281 - DNA, 23 bp, Homo sapiens
gcagctggaggatcagcaccagg

SEQ ID NO: 282 - DNA, 23 bp, Homo sapiens
actcacagagggtcagcagctgg

SEQ ID NO: 283 - DNA, 23 bp, Homo sapiens
aagaaaggggtgactcacagagg

SEQ ID NO: 284 - DNA, 23 bp, Homo sapiens
gtatctgcccaccatggccctgg

SEQ ID NO: 285 - DNA, 23 bp, Homo sapiens
tgttgcctcatttcctgggaggg

SEQ ID NO: 286 - DNA, 23 bp, Homo sapiens
atgttgcctcatttcctgggagg

SEQ ID NO: 287 - DNA, 23 bp, Homo sapiens
actgtggaaaaattagcaggggg

SEQ ID NO: 288 - DNA, 23 bp, Homo sapiens
ctgatgttgcctcatttcctggg

SEQ ID NO: 289 - DNA, 23 bp, Homo sapiens
agccctggctccagctctagcgg

SEQ ID NO: 290 - DNA, 23 bp, Homo sapiens
atcagcaccagggccatggtggg

SEQ ID NO: 291 - DNA, 23 bp, Homo sapiens
acccgctagagctggagccaggg

SEQ ID NO: 292 - DNA, 23 bp, Homo sapiens
cactgtggaaaaattagcagggg

SEQ ID NO: 293 - DNA, 23 bp, Homo sapiens
tctgatgttgcctcatttcctgg

SEQ ID NO: 294 - DNA, 23 bp, Homo sapiens
agaaaggggtgactcacagaggg

SEQ ID NO: 295 - DNA, 23 bp, Homo sapiens
gttgcctcatttcctgggagggg

SEQ ID NO: 296 - DNA, 23 bp, Homo sapiens
ctctcccctcccaggaaatgagg

SEQ ID NO: 297 - DNA, 23 bp, Homo sapiens
gaggatcagcaccagggccatgg

SEQ ID NO: 298 - DNA, 23 bp, Homo sapiens
cacagagggtcagcagctggagg

SEQ ID NO: 299 - DNA, 23 bp, Homo sapiens
taatttttccacagtgccatagg

SEQ ID NO: 300 - DNA, 23 bp, Homo sapiens
aatttttccacagtgccataggg

SEQ ID NO: 301 - DNA, 23 bp, Homo sapiens
gccctggctccagctctagcggg

SEQ ID NO: 302 - DNA, 23 bp, Homo sapiens
ctcatttcctgggaggggagagg

SEQ ID NO: 303 - DNA, 23 bp, Homo sapiens
gatcagcaccagggccatggtgg

SEQ ID NO: 304 - DNA, 23 bp, Homo sapiens
tcatttcctgggaggggagaggg

SEQ ID NO: 305 - DNA, 23 bp, Homo sapiens
ctagagctggagccagggcttgg

SEQ ID NO: 306 - DNA, 23 bp, Homo sapiens
gtcgcaccctctcccctcccagg

SEQ ID NO: 307 - DNA, 23 bp, Homo sapiens
cacacagacatcactccgtctgg

SEQ ID NO: 308 - DNA, 23 bp, Homo sapiens
ctagtccctcaacctcctacagg

SEQ ID NO: 309 - DNA, 23 bp, Homo sapiens
tagtccctcaacctcctacaggg

SEQ ID NO: 310 - DNA, 23 bp, Homo sapiens
tggggtggctactcaccagacgg

SEQ ID NO: 311 - DNA, 23 bp, Homo sapiens
agaggccctgtaggaggttgagg

SEQ ID NO: 312 - DNA, 23 bp, Homo sapiens
tgacacagaggccctgtaggagg

SEQ ID NO: 313 - DNA, 23 bp, Homo sapiens
gaggccctgtaggaggttgaggg

SEQ ID NO: 314 - DNA, 23 bp, Homo sapiens
gtgatgtctgtgtgacacagagg

SEQ ID NO: 315 - DNA, 23 bp, Homo sapiens
gtgtgacacagaggccctgtagg

SEQ ID NO: 316 - DNA, 23 bp, Homo sapiens
ctcacctataatggccactaagg

SEQ ID NO: 317 - DNA, 23 bp, Homo sapiens
cacctataatggccactaagggg

SEQ ID NO: 318 - DNA, 23 bp, Homo sapiens
tcacctataatggccactaaggg

SEQ ID NO: 319 - DNA, 23 bp, Homo sapiens
ttccccttagtggccattatagg

SEQ ID NO: 320 - DNA, 23 bp, Homo sapiens
tcttcagtactcacctataatgg

SEQ ID NO: 321 - DNA, 23 bp, Homo sapiens
ataggtgagtactgaagaccagg

SEQ ID NO: 322 - DNA, 23 bp, Homo sapiens
tcttttctcattccccttagtgg

SEQ ID NO: 323 - DNA, 23 bp, Homo sapiens
tgcgttcagacttcttcggtagg

SEQ ID NO: 324 - DNA, 23 bp, Homo sapiens
ttcagacttcttcggtaggtggg

SEQ ID NO: 325 - DNA, 23 bp, Homo sapiens
tacttgaaccctagagtcggagg

SEQ ID NO: 326 - DNA, 23 bp, Homo sapiens
gtttctcctctcacgagttcagg

SEQ ID NO: 327 - DNA, 23 bp, Homo sapiens
gttcagacttcttcggtaggtgg

SEQ ID NO: 328 - DNA, 23 bp, Homo sapiens
gagcattcgctatattgcccagg

SEQ ID NO: 329 - DNA, 23 bp, Homo sapiens
gcggtctccctatgttgagcagg

SEQ ID NO: 330 - DNA, 23 bp, Homo sapiens
aactgcagcctccgactctaggg

SEQ ID NO: 331 - DNA, 23 bp, Homo sapiens
gcctcagcctccgtagtagctgg

SEQ ID NO: 332 - DNA, 23 bp, Homo sapiens
cagattcctgaactcgtgagagg

SEQ ID NO: 333 - DNA, 23 bp, Homo sapiens
caagctagcactaccacgcctgg

SEQ ID NO: 334 - DNA, 23 bp, Homo sapiens
tgtagtcccagctactacggagg

SEQ ID NO: 335 - DNA, 23 bp, Homo sapiens
gaactcgctgttgggcgcagcgg

SEQ ID NO: 336 - DNA, 23 bp, Homo sapiens
cttcttcggtaggtgggcaatgg

SEQ ID NO: 337 - DNA, 23 bp, Homo sapiens
agagaggggtttcgccatgttgg

SEQ ID NO: 338 - DNA, 23 bp, Homo sapiens
ggggtttcaccacattagccagg

SEQ ID NO: 339 - DNA, 23 bp, Homo sapiens
ctcacctataatggccactaagg

SEQ ID NO: 340 - DNA, 23 bp, Homo sapiens
aggtcagatcgagatcatcctgg

SEQ ID NO: 341 - DNA, 23 bp, Homo sapiens
taactgcagcctccgactctagg

SEQ ID NO: 342 - DNA, 23 bp, Homo sapiens
cacctataatggccactaagggg

SEQ ID NO: 343 - DNA, 23 bp, Homo sapiens
tcacctataatggccactaaggg

SEQ ID NO: 344 - DNA, 23 bp, Homo sapiens
taaaaataagggtcgggtgaggg

SEQ ID NO: 345 - DNA, 23 bp, Homo sapiens
ccccctcccatataagaatctgg

SEQ ID NO: 346 - DNA, 23 bp, Homo sapiens
cctcagcctccgtagtagctggg

SEQ ID NO: 347 - DNA, 23 bp, Homo sapiens
ccccatctcattggtaacccagg

SEQ ID NO: 348 - DNA, 23 bp, Homo sapiens
ttccccttagtggccattatagg

SEQ ID NO: 349 - DNA, 23 bp, Homo sapiens
gcaggttggtcttaaactactgg

SEQ ID NO: 350 - DNA, 23 bp, Homo sapiens
cccagattcttatatgggagggg

SEQ ID NO: 351 - DNA, 23 bp, Homo sapiens
ggactcccagattcttatatggg

SEQ ID NO: 352 - DNA, 23 bp, Homo sapiens
ctctcacgagttcaggaatctgg

SEQ ID NO: 353 - DNA, 23 bp, Homo sapiens
ctcccagattcttatatgggagg

SEQ ID NO: 354 - DNA, 23 bp, Homo sapiens
cccctcccatataagaatctggg

SEQ ID NO: 355 - DNA, 23 bp, Homo sapiens
cacacagacatcactccgtctgg

SEQ ID NO: 356 - DNA, 23 bp, Homo sapiens
aggaaggctgttgggtccggtgg

SEQ ID NO: 357 - DNA, 23 bp, Homo sapiens
actctacgatcattgttccctgg

SEQ ID NO: 358 - DNA, 23 bp, Homo sapiens
tttgaaaagaactcgctgttggg

SEQ ID NO: 359 - DNA, 23 bp, Homo sapiens
tctccctatgttgagcaggttgg

SEQ ID NO: 360 - DNA, 23 bp, Homo sapiens
tctcacgagttcaggaatctggg

SEQ ID NO: 361 - DNA, 23 bp, Homo sapiens
ggatcttgggctgggcgcaatgg

SEQ ID NO: 362 - DNA, 23 bp, Homo sapiens
gcagaggcgggcggatcacaagg

SEQ ID NO: 363 - DNA, 23 bp, Homo sapiens
gagccgaggcccagcactttggg

SEQ ID NO: 364 - DNA, 23 bp, Homo sapiens
cgagatcatcctggctaatgtgg

SEQ ID NO: 365 - DNA, 23 bp, Homo sapiens
ttttgaaaagaactcgctgttgg

SEQ ID NO: 366 - DNA, 23 bp, Homo sapiens
ggtctgcgttcagacttcttcgg

SEQ ID NO: 367 - DNA, 23 bp, Homo sapiens
gcctgggcaaccaagagttcagg

SEQ ID NO: 368 - DNA, 23 bp, Homo sapiens
ctagtccctcaacctcctacagg

SEQ ID NO: 369 - DNA, 23 bp, Homo sapiens
cacagggtctttaattaatctgg

SEQ ID NO: 370 - DNA, 23 bp, Homo sapiens
caaaaattatccgggcattgtgg

SEQ ID NO: 371 - DNA, 23 bp, Homo sapiens
agtctgaacgcagacccctctgg

SEQ ID NO: 372 - DNA, 23 bp, Homo sapiens
agaccaacctgctcaacataggg

SEQ ID NO: 373 - DNA, 23 bp, Homo sapiens
aattacttgaaccctagagtcgg

SEQ ID NO: 374 - DNA, 23 bp, Homo sapiens
ctccatggtggcatgcactttgg

SEQ ID NO: 375 - DNA, 23 bp, Homo sapiens
agaacacagattcccgaaagagg

SEQ ID NO: 376 - DNA, 23 bp, Homo sapiens
aaaaataagggtcgggtgagggg

SEQ ID NO: 377 - DNA, 23 bp, Homo sapiens
tcccagattcttatatgggaggg

SEQ ID NO: 378 - DNA, 23 bp, Homo sapiens
tccatggtggcatgcactttggg

SEQ ID NO: 379 - DNA, 23 bp, Homo sapiens
ctgaataaacggggctgcctggg

SEQ ID NO: 380 - DNA, 23 bp, Homo sapiens
cagaccagcctgaccaacatggg

SEQ ID NO: 381 - DNA, 23 bp, Homo sapiens
ataaaaataagggtcgggtgagg

SEQ ID NO: 382 - DNA, 23 bp, Homo sapiens
aggactcccagattcttatatgg

SEQ ID NO: 383 - DNA, 23 bp, Homo sapiens
acgatcattgttccctggaaagg

SEQ ID NO: 384 - DNA, 23 bp, Homo sapiens
gttctcttgctttaggacccagg

SEQ ID NO: 385 - DNA, 23 bp, Homo sapiens
ctgcccctctgatttgcacctgg

SEQ ID NO: 386 - DNA, 23 bp, Homo sapiens
attagagttctggctgggcgtgg

SEQ ID NO: 387 - DNA, 23 bp, Homo sapiens
aagaccaacctgctcaacatagg

SEQ ID NO: 388 - DNA, 23 bp, Homo sapiens
tcttcagtactcacctataatgg

SEQ ID NO: 389 - DNA, 23 bp, Homo sapiens
tcctgggttaccaatgagatggg

SEQ ID NO: 390 - DNA, 23 bp, Homo sapiens
tagtccctcaacctcctacaggg

SEQ ID NO: 391 - DNA, 23 bp, Homo sapiens
cttaagccctgtactgtgccagg

SEQ ID NO: 392 - DNA, 23 bp, Homo sapiens
cctgggttaccaatgagatgggg

SEQ ID NO: 393 - DNA, 23 bp, Homo sapiens
aaaggggcagtaattgtccaagg

SEQ ID NO: 394 - DNA, 23 bp, Homo sapiens
tgtttgagcccaagagattgagg

SEQ ID NO: 395 - DNA, 23 bp, Homo sapiens
tggggtggctactcaccagacgg

SEQ ID NO: 396 - DNA, 23 bp, Homo sapiens
tgaatacgatggtgaaactgagg

SEQ ID NO: 397 - DNA, 23 bp, Homo sapiens
tctcattgtgtcacccgggctgg

SEQ ID NO: 398 - DNA, 23 bp, Homo sapiens
gcttgtagttccagctgtttggg

SEQ ID NO: 399 - DNA, 23 bp, Homo sapiens
atacaaagattagcctggtgtgg

SEQ ID NO: 400 - DNA, 23 bp, Homo sapiens
agcttgtagttccagctgtttgg

SEQ ID NO: 401 - DNA, 23 bp, Homo sapiens
acaggtatctctggttcttgagg

SEQ ID NO: 402 - DNA, 23 bp, Homo sapiens
tcccaaagtgcatgccaccatgg

SEQ ID NO: 403 - DNA, 23 bp, Homo sapiens
caggctactcttgaactcttggg

SEQ ID NO: 404 - DNA, 23 bp, Homo sapiens
aatcaagccttgttaaaaccagg

SEQ ID NO: 405 - DNA, 23 bp, Homo sapiens
tgctttaggacccaggggtctgg

SEQ ID NO: 406 - DNA, 23 bp, Homo sapiens
tcacccgggctggagtacggtgg

SEQ ID NO: 407 - DNA, 23 bp, Homo sapiens
gggcttaagaaataggatcttgg

SEQ ID NO: 408 - DNA, 23 bp, Homo sapiens
agcttgtaaacttagcactttgg

SEQ ID NO: 409 - DNA, 23 bp, Homo sapiens
agagccaccgtactccagcccgg

SEQ ID NO: 410 - DNA, 23 bp, Homo sapiens
aaatttctgcctactgagacagg

SEQ ID NO: 411 - DNA, 23 bp, Homo sapiens
ttcctgggttaccaatgagatgg

SEQ ID NO: 412 - DNA, 23 bp, Homo sapiens
tgaaactgaggtcctagcttagg

SEQ ID NO: 413 - DNA, 23 bp, Homo sapiens
tcacatataaatgaatacgatgg

SEQ ID NO: 414 - DNA, 23 bp, Homo sapiens
gatttgatgagatctcacagcgg

SEQ ID NO: 415 - DNA, 23 bp, Homo sapiens
gaggtggggacaggtatctctgg

SEQ ID NO: 416 - DNA, 23 bp, Homo sapiens
cctggaaaggtggagttcaaggg

SEQ ID NO: 417 - DNA, 23 bp, Homo sapiens
ccatgttggtcaggctggtctgg

SEQ ID NO: 418 - DNA, 23 bp, Homo sapiens
atggtggcatgcactttgggagg

SEQ ID NO: 419 - DNA, 23 bp, Homo sapiens
agttgccaaaacttgctatttgg

SEQ ID NO: 420 - DNA, 23 bp, Homo sapiens
agttcaagggcctgaactcttgg

SEQ ID NO: 421 - DNA, 23 bp, Homo sapiens
agcaagctgtgacttgttctagg

SEQ ID NO: 422 - DNA, 23 bp, Homo sapiens
tgtggccagccccatctcattgg

SEQ ID NO: 423 - DNA, 23 bp, Homo sapiens
ggcttaagaaataggatcttggg

SEQ ID NO: 424 - DNA, 23 bp, Homo sapiens
ccagtttctctctgtcgcccagg

SEQ ID NO: 425 - DNA, 23 bp, Homo sapiens
ccagattcttatatgggaggggg

SEQ ID NO: 426 - DNA, 23 bp, Homo sapiens
atcacacaaattaagagtacagg

SEQ ID NO: 427 - DNA, 23 bp, Homo sapiens
actgaataaacggggctgcctgg

SEQ ID NO: 428 - DNA, 23 bp, Homo sapiens
taagaaataggatcttgggctgg

SEQ ID NO: 429 - DNA, 23 bp, Homo sapiens
ggttaccaatgagatggggctgg

SEQ ID NO: 430 - DNA, 23 bp, Homo sapiens
gcgcagcggctcatgcctgtggg

SEQ ID NO: 431 - DNA, 23 bp, Homo sapiens
gaacgcagacccctctggcctgg

SEQ ID NO: 432 - DNA, 23 bp, Homo sapiens
ctgaggcagaggcctaagctagg

SEQ ID NO: 433 - DNA, 23 bp, Homo sapiens
cagtacagggcttaagaaatagg

SEQ ID NO: 434 - DNA, 23 bp, Homo sapiens
cactgcagcctcaatctcttggg

SEQ ID NO: 435 - DNA, 23 bp, Homo sapiens
caagagttcaagagtagcctggg

SEQ ID NO: 436 - DNA, 23 bp, Homo sapiens
aaaataagggtcgggtgaggggg

SEQ ID NO: 437 - DNA, 23 bp, Homo sapiens
tacaggaaggctgttgggtccgg

SEQ ID NO: 438 - DNA, 23 bp, Homo sapiens
gtatctctggttcttgaggcagg

SEQ ID NO: 439 - DNA, 23 bp, Homo sapiens
cccagctactacggaggctgagg

SEQ ID NO: 440 - DNA, 23 bp, Homo sapiens
caagtgcccgccaccacaccagg

SEQ ID NO: 441 - DNA, 23 bp, Homo sapiens
acagaaaaattagccaggcgtgg

SEQ ID NO: 442 - DNA, 23 bp, Homo sapiens
ggtcttgaactcctgtcctcagg

SEQ ID NO: 443 - DNA, 23 bp, Homo sapiens
gcaaccacctcctgggttcaagg

SEQ ID NO: 444 - DNA, 23 bp, Homo sapiens
gattagcctggtgtggtggcggg

SEQ ID NO: 445 - DNA, 23 bp, Homo sapiens
ccaagagttcaagagtagcctgg

SEQ ID NO: 446 - DNA, 23 bp, Homo sapiens
caaggtgggtgcatcacctgagg

SEQ ID NO: 447 - DNA, 23 bp, Homo sapiens
ataggtgagtactgaagaccagg

SEQ ID NO: 448 - DNA, 23 bp, Homo sapiens
agacaccctgcagggggaccagg

SEQ ID NO: 449 - DNA, 23 bp, Homo sapiens
acagagtgagaactccatggtgg

SEQ ID NO: 450 - DNA, 23 bp, Homo sapiens
taaaaccaggtgcaaatcagagg

SEQ ID NO: 451 - DNA, 23 bp, Homo sapiens
ggtcttgaactcctgacctcagg

SEQ ID NO: 452 - DNA, 23 bp, Homo sapiens
gcttgtaaacttagcactttggg

SEQ ID NO: 453 - DNA, 23 bp, Homo sapiens
gagatggggctggccacaaaggg

SEQ ID NO: 454 - DNA, 23 bp, Homo sapiens
ctggaggattgtctgagcccagg

SEQ ID NO: 455 - DNA, 23 bp, Homo sapiens
cccccttttcccagggaatcagg

SEQ ID NO: 456 - DNA, 23 bp, Homo sapiens
caggcacatgccactacaccagg

SEQ ID NO: 457 - DNA, 23 bp, Homo sapiens
aaaaaattagcctggtgtagtgg

SEQ ID NO: 458 - DNA, 23 bp, Homo sapiens
ttctcttgctttaggacccaggg

SEQ ID NO: 459 - DNA, 23 bp, Homo sapiens
tgagatggggctggccacaaagg

SEQ ID NO: 460 - DNA, 23 bp, Homo sapiens
tctcttgctttaggacccagggg

SEQ ID NO: 461 - DNA, 23 bp, Homo sapiens
tcactgcagctttgaattcctgg

SEQ ID NO: 462 - DNA, 23 bp, Homo sapiens
tactcagcatcccaaacagctgg

SEQ ID NO: 463 - DNA, 23 bp, Homo sapiens
ggctcactgcaaccacctcctgg

SEQ ID NO: 464 - DNA, 23 bp, Homo sapiens
ggcagcaggtttgggattctagg

SEQ ID NO: 465 - DNA, 23 bp, Homo sapiens
gctcatgcctgtgggagccgagg

SEQ ID NO: 466 - DNA, 23 bp, Homo sapiens
ccttgaactccacctttccaggg

SEQ ID NO: 467 - DNA, 23 bp, Homo sapiens
ccgaggcccagcactttgggagg

SEQ ID NO: 468 - DNA, 23 bp, Homo sapiens
cacaaattaagagtacaggaagg

SEQ ID NO: 469 - DNA, 23 bp, Homo sapiens
agcggcccattttacagagaagg

SEQ ID NO: 470 - DNA, 23 bp, Homo sapiens
agaggccctgtaggaggttgagg

SEQ ID NO: 471 - DNA, 23 bp, Homo sapiens
aaggatatctgggatgggattgg

SEQ ID NO: 472 - DNA, 23 bp, Homo sapiens
tggggtctcattgtgtcacccgg

SEQ ID NO: 473 - DNA, 23 bp, Homo sapiens
ggagccgaggcccagcactttgg

SEQ ID NO: 474 - DNA, 23 bp, Homo sapiens
ctctccctgattttacaaacagg

SEQ ID NO: 475 - DNA, 23 bp, Homo sapiens
cacagattcccgaaagaggaagg

SEQ ID NO: 476 - DNA, 23 bp, Homo sapiens
caaagattagcctggtgtggtgg

SEQ ID NO: 477 - DNA, 23 bp, Homo sapiens
aagagtacaggaaggctgttggg

SEQ ID NO: 478 - DNA, 23 bp, Homo sapiens
tttaaaattagagttctggctgg

SEQ ID NO: 479 - DNA, 23 bp, Homo sapiens
tgggtgcatcacctgaggtcagg

SEQ ID NO: 480 - DNA, 23 bp, Homo sapiens
gttcaaataaagaacagggctgg

SEQ ID NO: 481 - DNA, 23 bp, Homo sapiens
gcctgtggtcccaggtactcagg

SEQ ID NO: 482 - DNA, 23 bp, Homo sapiens
gaaactgtgtttacaaactgtgg

SEQ ID NO: 483 - DNA, 23 bp, Homo sapiens
aggatatctgggatgggattggg

SEQ ID NO: 484 - DNA, 23 bp, Homo sapiens
agctggggggactgaataaacgg

SEQ ID NO: 485 - DNA, 23 bp, Homo sapiens
ttaaaattagagttctggctggg

SEQ ID NO: 486 - DNA, 23 bp, Homo sapiens
tgtctcagtaggcagaaatttgg

SEQ ID NO: 487 - DNA, 23 bp, Homo sapiens
tgacacagaggccctgtaggagg

SEQ ID NO: 488 - DNA, 23 bp, Homo sapiens
gcaacagagtgagaactccatgg

SEQ ID NO: 489 - DNA, 23 bp, Homo sapiens
gagctgggaactcagattcctgg

SEQ ID NO: 490 - DNA, 23 bp, Homo sapiens
cccttgaactccacctttccagg

SEQ ID NO: 491 - DNA, 23 bp, Homo sapiens
catgtgcaaaaccctgagcctgg

SEQ ID NO: 492 - DNA, 23 bp, Homo sapiens
cactgcagctttgaattcctggg

SEQ ID NO: 493 - DNA, 23 bp, Homo sapiens
atttgcacctggttttaacaagg

SEQ ID NO: 494 - DNA, 23 bp, Homo sapiens
agctgtttgggatgctgagtagg

SEQ ID NO: 495 - DNA, 23 bp, Homo sapiens
tggtccccctgcagggtgtctgg

SEQ ID NO: 496 - DNA, 23 bp, Homo sapiens
tcttggttgcccaggccagaggg

SEQ ID NO: 497 - DNA, 23 bp, Homo sapiens
ggtccccctgcagggtgtctggg

SEQ ID NO: 498 - DNA, 23 bp, Homo sapiens
gggattttaccatgttggtcagg

SEQ ID NO: 499 - DNA, 23 bp, Homo sapiens
gaggccctgtaggaggttgaggg

SEQ ID NO: 500 - DNA, 23 bp, Homo sapiens
cctgggcgacagagagaaactgg

SEQ ID NO: 501 - DNA, 23 bp, Homo sapiens
ccctggaaaggtggagttcaagg

SEQ ID NO: 502 - DNA, 23 bp, Homo sapiens
ccctgagcctggcacagtacagg

SEQ ID NO: 503 - DNA, 23 bp, Homo sapiens
agaatcccaaacctgctgcctgg

SEQ ID NO: 504 - DNA, 23 bp, Homo sapiens
aacgcagacccctctggcctggg

SEQ ID NO: 505 - DNA, 23 bp, Homo sapiens
tttctgcctactgagacaggagg

SEQ ID NO: 506 - DNA, 23 bp, Homo sapiens
tctaggttcaaataaagaacagg

SEQ ID NO: 507 - DNA, 23 bp, Homo sapiens
taagagtacaggaaggctgttgg

SEQ ID NO: 508 - DNA, 23 bp, Homo sapiens
gtgacttgttctaggtcatatgg

SEQ ID NO: 509 - DNA, 23 bp, Homo sapiens
gggaggaaaataaggatatctgg

SEQ ID NO: 510 - DNA, 23 bp, Homo sapiens
gctttaggacccaggggtctggg

SEQ ID NO: 511 - DNA, 23 bp, Homo sapiens
agctgggaactcagattcctggg

SEQ ID NO: 512 - DNA, 23 bp, Homo sapiens
aagaaataggatcttgggctggg

SEQ ID NO: 513 - DNA, 23 bp, Homo sapiens
ttgggaaatggtatgaggtaggg

SEQ ID NO: 514 - DNA, 23 bp, Homo sapiens
tgtaaacttagcactttgggagg

SEQ ID NO: 515 - DNA, 23 bp, Homo sapiens
ggtgtagtggcatgtgcctgtgg

SEQ ID NO: 516 - DNA, 23 bp, Homo sapiens
caggtgcaaatcagaggggcagg

SEQ ID NO: 517 - DNA, 23 bp, Homo sapiens
actcacagagggtcagcagctgg

SEQ ID NO: 518 - DNA, 23 bp, Homo sapiens
aagaaaggggtgactcacagagg

SEQ ID NO: 519 - DNA, 23 bp, Homo sapiens
ttcccagctcctatctcctctgg

SEQ ID NO: 520 - DNA, 23 bp, Homo sapiens
tggagacccagacaccctgcagg

SEQ ID NO: 521 - DNA, 23 bp, Homo sapiens
gagccaccgtactccagcccggg

SEQ ID NO: 522 - DNA, 23 bp, Homo sapiens
cctgggtcctcgggcctcctggg

SEQ ID NO: 523 - DNA, 23 bp, Homo sapiens
agattagcctggtgtggtggcgg

SEQ ID NO: 524 - DNA, 23 bp, Homo sapiens
agagttctggctgggcgtggtgg

SEQ ID NO: 525 - DNA, 23 bp, Homo sapiens
tgtttgtaatcccaacactttgg

SEQ ID NO: 526 - DNA, 23 bp, Homo sapiens
tgctgggcctcggctcccacagg

SEQ ID NO: 527 - DNA, 23 bp, Homo sapiens
tcctgagtacctgggaccacagg

SEQ ID NO: 528 - DNA, 23 bp, Homo sapiens
gttcttttcaaaaccctttgtgg

SEQ ID NO: 529 - DNA, 23 bp, Homo sapiens
gggaaggaggaaaatcaccttgg

SEQ ID NO: 530 - DNA, 23 bp, Homo sapiens
gctcactgcaaccacctcctggg

SEQ ID NO: 531 - DNA, 23 bp, Homo sapiens
gctactacggaggctgaggcagg

SEQ ID NO: 532 - DNA, 23 bp, Homo sapiens
cttggttgcccaggccagagggg

SEQ ID NO: 533 - DNA, 23 bp, Homo sapiens
ctgaagaccaggaacttctgagg

SEQ ID NO: 534 - DNA, 23 bp, Homo sapiens
cgggtggatcacctgaggacagg

SEQ ID NO: 535 - DNA, 23 bp, Homo sapiens
tttgggaaatggtatgaggtagg

SEQ ID NO: 536 - DNA, 23 bp, Homo sapiens
tcccagaggagataggagctggg

SEQ ID NO: 537 - DNA, 23 bp, Homo sapiens
gtgatgtctgtgtgacacagagg

SEQ ID NO: 538 - DNA, 23 bp, Homo sapiens
ggaggaaaataaggatatctggg

SEQ ID NO: 539 - DNA, 23 bp, Homo sapiens
cttttccaaatagcaagttttgg

SEQ ID NO: 540 - DNA, 23 bp, Homo sapiens
attccctgggaaaagggggctgg

SEQ ID NO: 541 - DNA, 23 bp, Homo sapiens
agccaggactcctgattccctgg

SEQ ID NO: 542 - DNA, 23 bp, Homo sapiens
aaaataaggatatctgggatggg

SEQ ID NO: 543 - DNA, 23 bp, Homo sapiens
tcaaataaagaacagggctgggg

SEQ ID NO: 544 - DNA, 23 bp, Homo sapiens
gtgtgacacagaggccctgtagg

SEQ ID NO: 545 - DNA, 23 bp, Homo sapiens
ggtctggaactcctgacctcagg

SEQ ID NO: 546 - DNA, 23 bp, Homo sapiens
ctgctgcctggtccccctgcagg

SEQ ID NO: 547 - DNA, 23 bp, Homo sapiens
cgaggcgggtggatcacctgagg

SEQ ID NO: 548 - DNA, 23 bp, Homo sapiens
aaaccaggtgcaaatcagagggg

SEQ ID NO: 549 - DNA, 23 bp, Homo sapiens
aaacacagtttcaaaaggtcagg

SEQ ID NO: 550 - DNA, 23 bp, Homo sapiens
tttcatcttctggggctcccagg

SEQ ID NO: 551 - DNA, 23 bp, Homo sapiens
ttcccagaggagataggagctgg

SEQ ID NO: 552 - DNA, 23 bp, Homo sapiens
tgggagccccagaagatgaaagg

SEQ ID NO: 553 - DNA, 23 bp, Homo sapiens
tcttttctcattccccttagtgg

SEQ ID NO: 554 - DNA, 23 bp, Homo sapiens
tatttgtcttggggtaaggaagg

SEQ ID NO: 555 - DNA, 23 bp, Homo sapiens
gtttgtaatcccaacactttggg

SEQ ID NO: 556 - DNA, 23 bp, Homo sapiens
gcctgggtcctcgggcctcctgg

SEQ ID NO: 557 - DNA, 23 bp, Homo sapiens
caggtgcgtcccaccacacccgg

SEQ ID NO: 558 - DNA, 23 bp, Homo sapiens
atcattgttccctggaaaggtgg

SEQ ID NO: 559 - DNA, 23 bp, Homo sapiens
aatgaataaaaataagggtcggg

SEQ ID NO: 560 - DNA, 23 bp, Homo sapiens
aaaaccaggtgcaaatcagaggg

SEQ ID NO: 561 - DNA, 23 bp, Homo sapiens
tttaagtaatgagatgggagggg

SEQ ID NO: 562 - DNA, 23 bp, Homo sapiens
ttcaaataaagaacagggctggg

SEQ ID NO: 563 - DNA, 23 bp, Homo sapiens
tgaggcagagggatcacctgagg

SEQ ID NO: 564 - DNA, 23 bp, Homo sapiens
tcactgcagcctcaatctcttgg

SEQ ID NO: 565 - DNA, 23 bp, Homo sapiens
gagacccagacaccctgcagggg

SEQ ID NO: 566 - DNA, 23 bp, Homo sapiens
gaaaataaggatatctgggatgg

SEQ ID NO: 567 - DNA, 23 bp, Homo sapiens
ctgcctactgagacaggaggagg

SEQ ID NO: 568 - DNA, 23 bp, Homo sapiens
cctgagcctggcacagtacaggg

SEQ ID NO: 569 - DNA, 23 bp, Homo sapiens
caggagaatcacttgaacctggg

SEQ ID NO: 570 - DNA, 23 bp, Homo sapiens
acctcagcctcctgagtacctgg

SEQ ID NO: 571 - DNA, 23 bp, Homo sapiens
aatatatttgtcttggggtaagg

SEQ ID NO: 572 - DNA, 23 bp, Homo sapiens
tcttgaggcaggaagaggtcagg

SEQ ID NO: 573 - DNA, 23 bp, Homo sapiens
tcccagggaatcaggagtcctgg

SEQ ID NO: 574 - DNA, 23 bp, Homo sapiens
gtgtcacccgggctggagtacgg

SEQ ID NO: 575 - DNA, 23 bp, Homo sapiens
gggagccccagaagatgaaaggg

SEQ ID NO: 576 - DNA, 23 bp, Homo sapiens
gcctctgcctcagaagttcctgg

SEQ ID NO: 577 - DNA, 23 bp, Homo sapiens
ctcttggttgcccaggccagagg

SEQ ID NO: 578 - DNA, 23 bp, Homo sapiens
ctcttagctcctgagagaagagg

SEQ ID NO: 579 - DNA, 23 bp, Homo sapiens
ctccctcctcctgtctcagtagg

SEQ ID NO: 580 - DNA, 23 bp, Homo sapiens
ctcaggtgatgcacccaccttgg

SEQ ID NO: 581 - DNA, 23 bp, Homo sapiens
cctcccaaagtgctgggcctcgg

SEQ ID NO: 582 - DNA, 23 bp, Homo sapiens
cccaggaggcccgaggacccagg

SEQ ID NO: 583 - DNA, 23 bp, Homo sapiens
ccaggctactcttgaactcttgg

SEQ ID NO: 584 - DNA, 23 bp, Homo sapiens
caggcacacaccacaatgcccgg

SEQ ID NO: 585 - DNA, 23 bp, Homo sapiens
caacaaaaggagagtggatgggg

SEQ ID NO: 586 - DNA, 23 bp, Homo sapiens
attcttatatgggagggggatgg

SEQ ID NO: 587 - DNA, 23 bp, Homo sapiens
agaaaggggtgactcacagaggg

SEQ ID NO: 588 - DNA, 23 bp, Homo sapiens
tttttaagtaatgagatgggagg

SEQ ID NO: 589 - DNA, 23 bp, Homo sapiens
tgcctactgagacaggaggaggg

SEQ ID NO: 590 - DNA, 23 bp, Homo sapiens
tctcatttcccagaggagatagg

SEQ ID NO: 591 - DNA, 23 bp, Homo sapiens
gggggaccaggcagcaggtttgg

SEQ ID NO: 592 - DNA, 23 bp, Homo sapiens
gctatttaaaattagagttctgg

SEQ ID NO: 593 - DNA, 23 bp, Homo sapiens
cctgattccctgggaaaaggggg

SEQ ID NO: 594 - DNA, 23 bp, Homo sapiens
caggagaatcccttgaacccagg

SEQ ID NO: 595 - DNA, 23 bp, Homo sapiens
cagagggatcacctgaggtcagg

SEQ ID NO: 596 - DNA, 23 bp, Homo sapiens
agattcccgaaagaggaaggagg

SEQ ID NO: 597 - DNA, 23 bp, Homo sapiens
cttagcactttgggaggccgagg

SEQ ID NO: 598 - DNA, 23 bp, Homo sapiens
accaggaacttctgaggcagagg

SEQ ID NO: 599 - DNA, 23 bp, Homo sapiens
tcctgattccctgggaaaagggg

SEQ ID NO: 600 - DNA, 23 bp, Homo sapiens
tcccagctcctatctcctctggg

SEQ ID NO: 601 - DNA, 23 bp, Homo sapiens
gccaggactcctgattccctggg

SEQ ID NO: 602 - DNA, 23 bp, Homo sapiens
catcttctggggctcccaggagg

SEQ ID NO: 603 - DNA, 23 bp, Homo sapiens
aaaaattagccgggtgtggtggg

SEQ ID NO: 604 - DNA, 23 bp, Homo sapiens
ttgttttgggaaatggtatgagg

SEQ ID NO: 605 - DNA, 23 bp, Homo sapiens
ttccctgggaaaagggggctggg

SEQ ID NO: 606 - DNA, 23 bp, Homo sapiens
tgctgcctggtccccctgcaggg

SEQ ID NO: 607 - DNA, 23 bp, Homo sapiens
tcccgaaagaggaaggaggtggg

SEQ ID NO: 608 - DNA, 23 bp, Homo sapiens
gcctgaactcttggttgcccagg

SEQ ID NO: 609 - DNA, 23 bp, Homo sapiens
attaatctggaagttgttttggg

SEQ ID NO: 610 - DNA, 23 bp, Homo sapiens
atgctaaaagacaaaactagagg

SEQ ID NO: 611 - DNA, 23 bp, Homo sapiens
actcctgattccctgggaaaagg

SEQ ID NO: 612 - DNA, 23 bp, Homo sapiens
acggggctgcctgggtcctcggg

SEQ ID NO: 613 - DNA, 23 bp, Homo sapiens
aattaatctggaagttgttttgg

SEQ ID NO: 614 - DNA, 23 bp, Homo sapiens
ttaagtaatgagatgggaggggg

SEQ ID NO: 615 - DNA, 23 bp, Homo sapiens
gagatgggattttaccatgttgg

SEQ ID NO: 616 - DNA, 23 bp, Homo sapiens
ctcctgattccctgggaaaaggg

SEQ ID NO: 617 - DNA, 23 bp, Homo sapiens
caaccacctcctgggttcaaggg

SEQ ID NO: 618 - DNA, 23 bp, Homo sapiens
agtttcctgtttgtaaaatcagg

SEQ ID NO: 619 - DNA, 23 bp, Homo sapiens
aaaaaaaaattagccgggtgtgg

SEQ ID NO: 620 - DNA, 23 bp, Homo sapiens
tggggctcccaggaggcccgagg

SEQ ID NO: 621 - DNA, 23 bp, Homo sapiens
tcttagctcctgagagaagaggg

SEQ ID NO: 622 - DNA, 23 bp, Homo sapiens
tagaggacaaatgatagtactgg

SEQ ID NO: 623 - DNA, 23 bp, Homo sapiens
taataaaattacagagttctggg

SEQ ID NO: 624 - DNA, 23 bp, Homo sapiens
gcatgcactttgggaggctgagg

SEQ ID NO: 625 - DNA, 23 bp, Homo sapiens
gagacagggtttccccatgttgg

SEQ ID NO: 626 - DNA, 23 bp, Homo sapiens
cgaggtgggaggattgcttgagg

SEQ ID NO: 627 - DNA, 23 bp, Homo sapiens
ataagattctcatttcccagagg

SEQ ID NO: 628 - DNA, 23 bp, Homo sapiens
aacggggctgcctgggtcctcgg

SEQ ID NO: 629 - DNA, 23 bp, Homo sapiens
aaaaaattagccgggtgtggtgg

SEQ ID NO: 630 - DNA, 23 bp, Homo sapiens
ggagacccagacaccctgcaggg

SEQ ID NO: 631 - DNA, 23 bp, Homo sapiens
gcaccactgcactccggcctggg

SEQ ID NO: 632 - DNA, 23 bp, Homo sapiens
ccaacttccctttcatcttctgg

SEQ ID NO: 633 - DNA, 23 bp, Homo sapiens
atgggagggggatggaagccagg

SEQ ID NO: 634 - DNA, 23 bp, Homo sapiens
agtcacccctttcttctccctgg

SEQ ID NO: 635 - DNA, 23 bp, Homo sapiens
aatctgtgttctcttgctttagg

SEQ ID NO: 636 - DNA, 23 bp, Homo sapiens
aacttccctttcatcttctgggg

SEQ ID NO: 637 - DNA, 23 bp, Homo sapiens
tgtcagcaacaaaaggagagtgg

SEQ ID NO: 638 - DNA, 23 bp, Homo sapiens
gttcccagcccccttttcccagg

SEQ ID NO: 639 - DNA, 23 bp, Homo sapiens
ggagtgcagtggtgcaatctcgg

SEQ ID NO: 640 - DNA, 23 bp, Homo sapiens
ctaggttcaaataaagaacaggg

SEQ ID NO: 641 - DNA, 23 bp, Homo sapiens
atactatattgcaaatattctgg

SEQ ID NO: 642 - DNA, 23 bp, Homo sapiens
agacccagacaccctgcaggggg

SEQ ID NO: 643 - DNA, 23 bp, Homo sapiens
aaaggggtgtcagcaacaaaagg

SEQ ID NO: 644 - DNA, 23 bp, Homo sapiens
ttgctcaggcaggagtgcagtgg

SEQ ID NO: 645 - DNA, 23 bp, Homo sapiens
taaaaatacaaagattagcctgg

SEQ ID NO: 646 - DNA, 23 bp, Homo sapiens
ggggaccaggcagcaggtttggg

SEQ ID NO: 647 - DNA, 23 bp, Homo sapiens
gcaggaagaggtcaggagacagg

SEQ ID NO: 648 - DNA, 23 bp, Homo sapiens
gagaatcacttgaacctgggagg

SEQ ID NO: 649 - DNA, 23 bp, Homo sapiens
ctggttcttgaggcaggaagagg

SEQ ID NO: 650 - DNA, 23 bp, Homo sapiens
cacagagggtcagcagctggagg

SEQ ID NO: 651 - DNA, 23 bp, Homo sapiens
caacttccctttcatcttctggg

SEQ ID NO: 652 - DNA, 23 bp, Homo sapiens
aaaatctgagtaattggaaaagg

SEQ ID NO: 653 - DNA, 23 bp, Homo sapiens
ttcccagcccccttttcccaggg

SEQ ID NO: 654 - DNA, 23 bp, Homo sapiens
tggcatgtgcctgtggtcccagg

SEQ ID NO: 655 - DNA, 23 bp, Homo sapiens
ggggtctcattgtgtcacccggg

SEQ ID NO: 656 - DNA, 23 bp, Homo sapiens
gggctggggcccagacccctggg

SEQ ID NO: 657 - DNA, 23 bp, Homo sapiens
ctcaggtgatccacccgcctcgg

SEQ ID NO: 658 - DNA, 23 bp, Homo sapiens
cagaagatgaaagggaagttggg

SEQ ID NO: 659 - DNA, 23 bp, Homo sapiens
cacttgaacctgggaggcagagg

SEQ ID NO: 660 - DNA, 23 bp, Homo sapiens
caaaataaaatctgagtaattgg

SEQ ID NO: 661 - DNA, 23 bp, Homo sapiens
tgggttcctggctggggttgggg

SEQ ID NO: 662 - DNA, 23 bp, Homo sapiens
gcctcagcctcccaaagtgttgg

SEQ ID NO: 663 - DNA, 23 bp, Homo sapiens
ctggaagttgttttgggaaatgg

SEQ ID NO: 664 - DNA, 23 bp, Homo sapiens
cccgaaagaggaaggaggtgggg

SEQ ID NO: 665 - DNA, 23 bp, Homo sapiens
caaaaggagagtggatggggtgg

SEQ ID NO: 666 - DNA, 23 bp, Homo sapiens
ataataaaattacagagttctgg

SEQ ID NO: 667 - DNA, 23 bp, Homo sapiens
agcaacaaaaggagagtggatgg

SEQ ID NO: 668 - DNA, 23 bp, Homo sapiens
tccccacctccttcctctttcgg

SEQ ID NO: 669 - DNA, 23 bp, Homo sapiens
gcaacaaaaggagagtggatggg

SEQ ID NO: 670 - DNA, 23 bp, Homo sapiens
cttctccctgggttcctggctgg

SEQ ID NO: 671 - DNA, 23 bp, Homo sapiens
agggtttccccatgttggtcagg

SEQ ID NO: 672 - DNA, 23 bp, Homo sapiens
agggctggggcccagacccctgg

SEQ ID NO: 673 - DNA, 23 bp, Homo sapiens
ttgtaaaatcagggagagactgg

SEQ ID NO: 674 - DNA, 23 bp, Homo sapiens
gtttcctgtttgtaaaatcaggg

SEQ ID NO: 675 - DNA, 23 bp, Homo sapiens
ctttcttctccctgggttcctgg

SEQ ID NO: 676 - DNA, 23 bp, Homo sapiens
ctgcagggggaccaggcagcagg

SEQ ID NO: 677 - DNA, 23 bp, Homo sapiens
caagagaatcgcttgaacccagg

SEQ ID NO: 678 - DNA, 23 bp, Homo sapiens
acaacttaagaaatttgaagtgg

SEQ ID NO: 679 - DNA, 23 bp, Homo sapiens
aaaaaaaagtctgggtgtggtgg

SEQ ID NO: 680 - DNA, 23 bp, Homo sapiens
tttgtaaacacagtttcaaaagg

SEQ ID NO: 681 - DNA, 23 bp, Homo sapiens
tcctgagagaagagggaaatggg

SEQ ID NO: 682 - DNA, 23 bp, Homo sapiens
gggaaaagggggctgggaacagg

SEQ ID NO: 683 - DNA, 23 bp, Homo sapiens
ggcgcagcggctcatgcctgtgg

SEQ ID NO: 684 - DNA, 23 bp, Homo sapiens
ggaaactgaggctaagaaagggg

SEQ ID NO: 685 - DNA, 23 bp, Homo sapiens
gcctcagcctcctgagtagctgg

SEQ ID NO: 686 - DNA, 23 bp, Homo sapiens
gatgaaagggaagttggggaagg

SEQ ID NO: 687 - DNA, 23 bp, Homo sapiens
agtaatgagatgggagggggcgg

SEQ ID NO: 688 - DNA, 23 bp, Homo sapiens
ttatttttaagtaatgagatggg

SEQ ID NO: 689 - DNA, 23 bp, Homo sapiens
tactgcaacctctgcctcctggg

SEQ ID NO: 690 - DNA, 23 bp, Homo sapiens
ccccatttccctcttctctcagg

SEQ ID NO: 691 - DNA, 23 bp, Homo sapiens
caaccccagccaggaacccaggg

SEQ ID NO: 692 - DNA, 23 bp, Homo sapiens
aggaaactgaggctaagaaaggg

SEQ ID NO: 693 - DNA, 23 bp, Homo sapiens
aatcccttgaacccaggaggtgg

SEQ ID NO: 694 - DNA, 23 bp, Homo sapiens
aaatctgagtaattggaaaaggg

SEQ ID NO: 695 - DNA, 23 bp, Homo sapiens
aaaagtattcaaaaaactatagg

SEQ ID NO: 696 - DNA, 23 bp, Homo sapiens
tcctgagtagctgggattacagg

SEQ ID NO: 697 - DNA, 23 bp, Homo sapiens
gcctctgcctcccaaagtgctgg

SEQ ID NO: 698 - DNA, 23 bp, Homo sapiens
cctgagagaagagggaaatgggg

SEQ ID NO: 699 - DNA, 23 bp, Homo sapiens
ccctgtactgtgccaggctcagg

SEQ ID NO: 700 - DNA, 23 bp, Homo sapiens
ctttgggaggcagaggcgggcgg

SEQ ID NO: 701 - DNA, 23 bp, Homo sapiens
ctactgagacaggaggagggagg

SEQ ID NO: 702 - DNA, 23 bp, Homo sapiens
ccagaagatgaaagggaagttgg

SEQ ID NO: 703 - DNA, 23 bp, Homo sapiens
caggaagaggtcaggagacaggg

SEQ ID NO: 704 - DNA, 23 bp, Homo sapiens
ataggaaaatatatttgtcttgg

SEQ ID NO: 705 - DNA, 23 bp, Homo sapiens
aggaaaatatatttgtcttgggg

SEQ ID NO: 706 - DNA, 23 bp, Homo sapiens
ttctccctgggttcctggctggg

SEQ ID NO: 707 - DNA, 23 bp, Homo sapiens
taggaaaatatatttgtcttggg

SEQ ID NO: 708 - DNA, 23 bp, Homo sapiens
ggaaaagggggctgggaacaggg

SEQ ID NO: 709 - DNA, 23 bp, Homo sapiens
ctttgggaggccgaggcgggtgg

SEQ ID NO: 710 - DNA, 23 bp, Homo sapiens
cctcagcctcctgagtacctggg

SEQ ID NO: 711 - DNA, 23 bp, Homo sapiens
cctcagcctcccaaagtgttggg

SEQ ID NO: 712 - DNA, 23 bp, Homo sapiens
ccaaccccagccaggaacccagg

SEQ ID NO: 713 - DNA, 23 bp, Homo sapiens
caggaacccagggagaagaaagg

SEQ ID NO: 714 - DNA, 23 bp, Homo sapiens
caggaaactgaggctaagaaagg

SEQ ID NO: 715 - DNA, 23 bp, Homo sapiens
cacaccactacactccagcctgg

SEQ ID NO: 716 - DNA, 23 bp, Homo sapiens
attatttttaagtaatgagatgg

SEQ ID NO: 717 - DNA, 23 bp, Homo sapiens
ttttaagtaatgagatgggaggg

SEQ ID NO: 718 - DNA, 23 bp, Homo sapiens
ttcccgaaagaggaaggaggtgg

SEQ ID NO: 719 - DNA, 23 bp, Homo sapiens
tgcaccactgcactccggcctgg

SEQ ID NO: 720 - DNA, 23 bp, Homo sapiens
gagaatcgcttgaacccaggagg

SEQ ID NO: 721 - DNA, 23 bp, Homo sapiens
gaagaggtcaggagacagggagg

SEQ ID NO: 722 - DNA, 23 bp, Homo sapiens
atataaaataaaaagttgtatgg

SEQ ID NO: 723 - DNA, 23 bp, Homo sapiens
agaagatgaaagggaagttgggg

SEQ ID NO: 724 - DNA, 23 bp, Homo sapiens
tttctctctgtcgcccaggccgg

SEQ ID NO: 725 - DNA, 23 bp, Homo sapiens
ttactgcaacctctgcctcctgg

SEQ ID NO: 726 - DNA, 23 bp, Homo sapiens
gtcacccctttcttctccctggg

SEQ ID NO: 727 - DNA, 23 bp, Homo sapiens
ggggtttcgccatgttggtcagg

SEQ ID NO: 728 - DNA, 23 bp, Homo sapiens
gagaatcccttgaacccaggagg

SEQ ID NO: 729 - DNA, 23 bp, Homo sapiens
ctcctgagagaagagggaaatgg

SEQ ID NO: 730 - DNA, 23 bp, Homo sapiens
ctaaggggaatgagaaaagaagg

SEQ ID NO: 731 - DNA, 23 bp, Homo sapiens
tttctgtttttagtagagatggg

SEQ ID NO: 732 - DNA, 23 bp, Homo sapiens
tcgcccaggctggagtgtagtgg

SEQ ID NO: 733 - DNA, 23 bp, Homo sapiens
gggttcctggctggggttggggg

SEQ ID NO: 734 - DNA, 23 bp, Homo sapiens
gcactttgggaggcagaggcggg

SEQ ID NO: 735 - DNA, 23 bp, Homo sapiens
ccccacctccttcctctttcggg

SEQ ID NO: 736 - DNA, 23 bp, Homo sapiens
caattactcagattttattttgg

SEQ ID NO: 737 - DNA, 23 bp, Homo sapiens
attttacaaacaggaaactgagg

SEQ ID NO: 738 - DNA, 23 bp, Homo sapiens
acttgtagtcccagctactacgg

SEQ ID NO: 739 - DNA, 23 bp, Homo sapiens
aaaaaaaaaaagtctgggtgtgg

SEQ ID NO: 740 - DNA, 23 bp, Homo sapiens
tgtaatcccagctactcaggagg

SEQ ID NO: 741 - DNA, 23 bp, Homo sapiens
tggagggagggaggaaaataagg

SEQ ID NO: 742 - DNA, 23 bp, Homo sapiens
taaaaatacaaaaattatccggg

SEQ ID NO: 743 - DNA, 23 bp, Homo sapiens
ggggaatgagaaaagaaggaagg

SEQ ID NO: 744 - DNA, 23 bp, Homo sapiens
aggaacccagggagaagaaaggg

SEQ ID NO: 745 - DNA, 23 bp, Homo sapiens
acaccactacactccagcctggg

SEQ ID NO: 746 - DNA, 23 bp, Homo sapiens
ttttattcatttttagagatggg

SEQ ID NO: 747 - DNA, 23 bp, Homo sapiens
tctccctgggttcctggctgggg

SEQ ID NO: 748 - DNA, 23 bp, Homo sapiens
tactgagacaggaggagggaggg

SEQ ID NO: 749 - DNA, 23 bp, Homo sapiens
cactgcaacctctgcctcccagg

SEQ ID NO: 750 - DNA, 23 bp, Homo sapiens
agcactttgggaggcagaggcgg

SEQ ID NO: 751 - DNA, 23 bp, Homo sapiens
aaatgaataaaaataagggtcgg

SEQ ID NO: 752 - DNA, 23 bp, Homo sapiens
tcctgagtagctgggactacagg

SEQ ID NO: 753 - DNA, 23 bp, Homo sapiens
cccagcactttgggaggcagagg

SEQ ID NO: 754 - DNA, 23 bp, Homo sapiens
tttattcatttttagagatgggg

SEQ ID NO: 755 - DNA, 23 bp, Homo sapiens
ggaacccagggagaagaaagggg

SEQ ID NO: 756 - DNA, 23 bp, Homo sapiens
gcaggagaatcacttgaacctgg

SEQ ID NO: 757 - DNA, 23 bp, Homo sapiens
gagattgcaccactgcactccgg

SEQ ID NO: 758 - DNA, 23 bp, Homo sapiens
ctttgggaggctgaggcagaggg

SEQ ID NO: 759 - DNA, 23 bp, Homo sapiens
aagaggaaggaggtggggacagg

SEQ ID NO: 760 - DNA, 23 bp, Homo sapiens
ctgggttcctggctggggttggg

SEQ ID NO: 761 - DNA, 23 bp, Homo sapiens
cctgggttcctggctggggttgg

SEQ ID NO: 762 - DNA, 23 bp, Homo sapiens
tatttggaaaagaaaaatgttgg

SEQ ID NO: 763 - DNA, 23 bp, Homo sapiens
taaaaacagaaaaattagccagg

SEQ ID NO: 764 - DNA, 23 bp, Homo sapiens
ctttgggaggccgaggtgggagg

SEQ ID NO: 765 - DNA, 23 bp, Homo sapiens
ctcaagcaatcctcccacctcgg

SEQ ID NO: 766 - DNA, 23 bp, Homo sapiens
ttttaccatgttggtcaggctgg

SEQ ID NO: 767 - DNA, 23 bp, Homo sapiens
tcgcccaggccggagtgcagtgg

SEQ ID NO: 768 - DNA, 23 bp, Homo sapiens
ctaaaaatacaaaaattatccgg

SEQ ID NO: 769 - DNA, 23 bp, Homo sapiens
cccaggtactcaggaggctgagg

SEQ ID NO: 770 - DNA, 23 bp, Homo sapiens
catttccttctctgtaaaatggg

SEQ ID NO: 771 - DNA, 23 bp, Homo sapiens
aggtactcaggaggctgaggtgg

SEQ ID NO: 772 - DNA, 23 bp, Homo sapiens
aagaaggaaggaatggagggagg

SEQ ID NO: 773 - DNA, 23 bp, Homo sapiens
tactcaggaggctgaggtggagg

SEQ ID NO: 774 - DNA, 23 bp, Homo sapiens
gtttaaaaaaaaagaaacacagg

SEQ ID NO: 775 - DNA, 23 bp, Homo sapiens
gcactttgggaggccgaggcggg

SEQ ID NO: 776 - DNA, 23 bp, Homo sapiens
ctttgggaggctgaggctggagg

SEQ ID NO: 777 - DNA, 23 bp, Homo sapiens
cctctgcctcccaaagtgctggg

SEQ ID NO: 778 - DNA, 23 bp, Homo sapiens
agtgctgggattacagacgttgg

SEQ ID NO: 779 - DNA, 23 bp, Homo sapiens
tttttattcatttttagagatgg

SEQ ID NO: 780 - DNA, 23 bp, Homo sapiens
gggggcagagagagaggcaatgg

SEQ ID NO: 781 - DNA, 23 bp, Homo sapiens
gcgccactgcactccagcctggg

SEQ ID NO: 782 - DNA, 23 bp, Homo sapiens
cgcgccactgcactccagcctgg

SEQ ID NO: 783 - DNA, 23 bp, Homo sapiens
cccaacactttgggaggctgagg

SEQ ID NO: 784 - DNA, 23 bp, Homo sapiens
agaaaagaaggaaggaatggagg

SEQ ID NO: 785 - DNA, 23 bp, Homo sapiens
actttgggaggctgaggcagagg

SEQ ID NO: 786 - DNA, 23 bp, Homo sapiens
acctcggcctcccaaagtgctgg

SEQ ID NO: 787 - DNA, 23 bp, Homo sapiens
tttccccatgttggtcaggctgg

SEQ ID NO: 788 - DNA, 23 bp, Homo sapiens
ggattacagctgtgagccaccgg

SEQ ID NO: 789 - DNA, 23 bp, Homo sapiens
ggagtcttgcactgtcacccagg

SEQ ID NO: 790 - DNA, 23 bp, Homo sapiens
gaaagggaagttggggaaggagg

SEQ ID NO: 791 - DNA, 23 bp, Homo sapiens
ccattttacagagaaggaaatgg

SEQ ID NO: 792 - DNA, 23 bp, Homo sapiens
ccatttccttctctgtaaaatgg

SEQ ID NO: 793 - DNA, 23 bp, Homo sapiens
ccagaccagcctgaccaacatgg

SEQ ID NO: 794 - DNA, 23 bp, Homo sapiens
agggtcttgctctgttgctcagg

SEQ ID NO: 795 - DNA, 23 bp, Homo sapiens
tctaaaaatgaataaaaataagg

SEQ ID NO: 796 - DNA, 23 bp, Homo sapiens
gctactcaggaggctgaggcagg

SEQ ID NO: 797 - DNA, 23 bp, Homo sapiens
cgcttgaacccaggaggcagagg

SEQ ID NO: 798 - DNA, 23 bp, Homo sapiens
cccagctactcaggaggctgagg

SEQ ID NO: 799 - DNA, 23 bp, Homo sapiens
caagaccagcctgaccaacatgg

SEQ ID NO: 800 - DNA, 23 bp, Homo sapiens
agcactttgggaggccgaggtgg

SEQ ID NO: 801 - DNA, 23 bp, Homo sapiens
agcactttgggaggccgaggcgg

SEQ ID NO: 802 - DNA, 23 bp, Homo sapiens
ttttttttttagtagagacgggg

SEQ ID NO: 803 - DNA, 23 bp, Homo sapiens
tcttgcactgtcacccaggctgg

SEQ ID NO: 804 - DNA, 23 bp, Homo sapiens
cctcagcctcctgagtagctggg

SEQ ID NO: 805 - DNA, 23 bp, Homo sapiens
acctgtaatcccagctactcagg

SEQ ID NO: 806 - DNA, 23 bp, Homo sapiens
acaaacaaaaaaaactcttttgg

SEQ ID NO: 807 - DNA, 23 bp, Homo sapiens
tttcgccatgttggtcaggctgg

SEQ ID NO: 808 - DNA, 23 bp, Homo sapiens
tctttgtatttttagtagagagg

SEQ ID NO: 809 - DNA, 23 bp, Homo sapiens
ggggttgggggcagagagagagg

SEQ ID NO: 810 - DNA, 23 bp, Homo sapiens
cagctgtaatcccagcactttgg

SEQ ID NO: 811 - DNA, 23 bp, Homo sapiens
atgagaaaagaaggaaggaatgg

SEQ ID NO: 812 - DNA, 23 bp, Homo sapiens
agaccagcctgaccaacatgggg

SEQ ID NO: 813 - DNA, 23 bp, Homo sapiens
tttttttttttagtagagacggg

SEQ ID NO: 814 - DNA, 23 bp, Homo sapiens
gcctgtagtcccagctactcagg

SEQ ID NO: 815 - DNA, 23 bp, Homo sapiens
gcactttgggaggctgaggctgg

SEQ ID NO: 816 - DNA, 23 bp, Homo sapiens
gcactttgggaggccaaggtggg

SEQ ID NO: 817 - DNA, 23 bp, Homo sapiens
gaaaagaaggaaggaatggaggg

SEQ ID NO: 818 - DNA, 23 bp, Homo sapiens
ctctgcccccaaccccagccagg

SEQ ID NO: 819 - DNA, 23 bp, Homo sapiens
cgtctgtaatcccagcactttgg

SEQ ID NO: 820 - DNA, 23 bp, Homo sapiens
ttttctgtttttagtagagatgg

SEQ ID NO: 821 - DNA, 23 bp, Homo sapiens
tttaaaaaaaaagaaacacaggg

SEQ ID NO: 822 - DNA, 23 bp, Homo sapiens
tgtaatcccaacactttgggagg

SEQ ID NO: 823 - DNA, 23 bp, Homo sapiens
tcttgctctgttgctcaggcagg

SEQ ID NO: 824 - DNA, 23 bp, Homo sapiens
ctaaaaatgaataaaaataaggg

SEQ ID NO: 825 - DNA, 23 bp, Homo sapiens
cccagcactttgggaggccgagg

SEQ ID NO: 826 - DNA, 23 bp, Homo sapiens
agagtctcactctgtcgcccagg

SEQ ID NO: 827 - DNA, 23 bp, Homo sapiens
agaaggaaggaatggagggaggg

SEQ ID NO: 828 - DNA, 23 bp, Homo sapiens
tgtggtcccaggtactcaggagg

SEQ ID NO: 829 - DNA, 23 bp, Homo sapiens
gcctcggcctcccaaagtgctgg

SEQ ID NO: 830 - DNA, 23 bp, Homo sapiens
catgccactgcactccagcctgg

SEQ ID NO: 831 - DNA, 23 bp, Homo sapiens
agctgtaatcccagcactttggg

SEQ ID NO: 832 - DNA, 23 bp, Homo sapiens
taaaaaaaaaaaaattagcctgg

SEQ ID NO: 833 - DNA, 23 bp, Homo sapiens
cctttttttttttttgtctgagg

SEQ ID NO: 834 - DNA, 23 bp, Homo sapiens
cctcggcctcccaaagtgctggg

SEQ ID NO: 835 - DNA, 23 bp, Homo sapiens
atgccactgcactccagcctggg

SEQ ID NO: 836 - DNA, 23 bp, Homo sapiens
accttggcctcccaaagtgctgg

SEQ ID NO: 837 - DNA, 23 bp, Homo sapiens
tttgtatttttagtagagagggg

SEQ ID NO: 838 - DNA, 23 bp, Homo sapiens
gtctgtaatcccagcactttggg

SEQ ID NO: 839 - DNA, 23 bp, Homo sapiens
cccagcactttgggaggccaagg

SEQ ID NO: 840 - DNA, 23 bp, Homo sapiens
cacctgtaatcccagcactttgg

SEQ ID NO: 841 - DNA, 23 bp, Homo sapiens
ttgtttgtttgtttttgaagtgg

SEQ ID NO: 842 - DNA, 23 bp, Homo sapiens
ttgcccaggctggagtgcagtgg

SEQ ID NO: 843 - DNA, 23 bp, Homo sapiens
tctcactctgtcgcccaggctgg

SEQ ID NO: 844 - DNA, 23 bp, Homo sapiens
agcactttgggaggccaaggtgg

SEQ ID NO: 845 - DNA, 23 bp, Homo sapiens
ttttttttttttagtagagacgg

SEQ ID NO: 846 - DNA, 23 bp, Homo sapiens
ttgtatttttagtagagacaggg

SEQ ID NO: 847 - DNA, 23 bp, Homo sapiens
tgtagtcccagctactcaggagg

SEQ ID NO: 848 - DNA, 23 bp, Homo sapiens
tcacccaggctggagtgcagtgg

SEQ ID NO: 849 - DNA, 23 bp, Homo sapiens
ccttggcctcccaaagtgctggg

SEQ ID NO: 850 - DNA, 23 bp, Homo sapiens
cctcagacaaaaaaaaaaaaagg

SEQ ID NO: 851 - DNA, 23 bp, Homo sapiens
aggaaggaatggagggagggagg

SEQ ID NO: 852 - DNA, 23 bp, Homo sapiens
aataaataaataaaataaatagg

SEQ ID NO: 853 - DNA, 23 bp, Homo sapiens
aaaaaaaaaaaaaattagccggg

SEQ ID NO: 854 - DNA, 23 bp, Homo sapiens
tgtaatcccagcactttgggagg

SEQ ID NO: 855 - DNA, 23 bp, Homo sapiens
tctcactctgttgcccaggctgg

SEQ ID NO: 856 - DNA, 23 bp, Homo sapiens
acctgtaatcccagcactttggg

SEQ ID NO: 857 - DNA, 23 bp, Homo sapiens
aaaaaaaaaaaaaaattagccgg

SEQ ID NO: 858 - DNA, 23 bp, Homo sapiens
tttgtatttttagtagagacagg

SEQ ID NO: 859 - DNA, 23 bp, Homo sapiens
tcccaaagtgctgggattacagg

SEQ ID NO: 860 - DNA, 23 bp, Homo sapiens
ctttgtatttttagtagagaggg

SEQ ID NO: 861 - DNA, 23 bp, Homo sapiens
tttttttttttttttgaggcagg

SEQ ID NO: 862 - DNA, 23 bp, Homo sapiens
ttttttttttttttgaggcaggg

SEQ ID NO: 863 - DNA, 23 bp, Homo sapiens
tttttttttttttttttttgagg

SEQ ID NO: 864 - DNA, 23 bp, Homo sapiens
aaaaaaaaaaaaaaaagtctggg

SEQ ID NO: 865 - DNA, 23 bp, Homo sapiens
aaaaaaaaaaaaaaaaagtctgg

SEQ ID NO: 866 - DNA, 23 bp, Homo sapiens
ctcacctataatggccactaagg

SEQ ID NO: 867 - DNA, 23 bp, Homo sapiens
cacctataatggccactaagggg

SEQ ID NO: 868 - DNA, 23 bp, Homo sapiens
tcacctataatggccactaaggg

SEQ ID NO: 869 - DNA, 23 bp, Homo sapiens
ttccccttagtggccattatagg

SEQ ID NO: 870 - DNA, 23 bp, Homo sapiens
cacacagacatcactccgtctgg

SEQ ID NO: 871 - DNA, 23 bp, Homo sapiens
tcttcagtactcacctataatgg

SEQ ID NO: 872 - DNA, 23 bp, Homo sapiens
tggggtggctactcaccagacgg

SEQ ID NO: 873 - DNA, 23 bp, Homo sapiens
tgaatacgatggtgaaactgagg

SEQ ID NO: 874 - DNA, 23 bp, Homo sapiens
tgaaactgaggtcctagcttagg

SEQ ID NO: 875 - DNA, 23 bp, Homo sapiens
tcacatataaatgaatacgatgg

SEQ ID NO: 876 - DNA, 23 bp, Homo sapiens
agcaagctgtgacttgttctagg

SEQ ID NO: 877 - DNA, 23 bp, Homo sapiens
ctgaggcagaggcctaagctagg

SEQ ID NO: 878 - DNA, 23 bp, Homo sapiens
ataggtgagtactgaagaccagg

SEQ ID NO: 879 - DNA, 23 bp, Homo sapiens
aaggatatctgggatgggattgg

SEQ ID NO: 880 - DNA, 23 bp, Homo sapiens
aggatatctgggatgggattggg

SEQ ID NO: 881 - DNA, 23 bp, Homo sapiens
gtgacttgttctaggtcatatgg

SEQ ID NO: 882 - DNA, 23 bp, Homo sapiens
gggaggaaaataaggatatctgg

SEQ ID NO: 883 - DNA, 23 bp, Homo sapiens
ctgaagaccaggaacttctgagg

SEQ ID NO: 884 - DNA, 23 bp, Homo sapiens
aaaataaggatatctgggatggg

SEQ ID NO: 885 - DNA, 23 bp, Homo sapiens
ggaggaaaataaggatatctggg

SEQ ID NO: 886 - DNA, 23 bp, Homo sapiens
tcttttctcattccccttagtgg

SEQ ID NO: 887 - DNA, 23 bp, Homo sapiens
gaaaataaggatatctgggatgg

SEQ ID NO: 888 - DNA, 23 bp, Homo sapiens
caacaaaaggagagtggatgggg

SEQ ID NO: 889 - DNA, 23 bp, Homo sapiens
gcctctgcctcagaagttcctgg

SEQ ID NO: 890 - DNA, 23 bp, Homo sapiens
accaggaacttctgaggcagagg

SEQ ID NO: 891 - DNA, 23 bp, Homo sapiens
tgtcagcaacaaaaggagagtgg

SEQ ID NO: 892 - DNA, 23 bp, Homo sapiens
aaaggggtgtcagcaacaaaagg

SEQ ID NO: 893 - DNA, 23 bp, Homo sapiens
aaaatctgagtaattggaaaagg

SEQ ID NO: 894 - DNA, 23 bp, Homo sapiens
caaaataaaatctgagtaattgg

SEQ ID NO: 895 - DNA, 23 bp, Homo sapiens
agcaacaaaaggagagtggatgg

SEQ ID NO: 896 - DNA, 23 bp, Homo sapiens
caaaaggagagtggatggggtgg

SEQ ID NO: 897 - DNA, 23 bp, Homo sapiens
gcaacaaaaggagagtggatggg

SEQ ID NO: 898 - DNA, 23 bp, Homo sapiens
aaatctgagtaattggaaaaggg

SEQ ID NO: 899 - DNA, 23 bp, Homo sapiens
ctaaggggaatgagaaaagaagg

SEQ ID NO: 900 - DNA, 23 bp, Homo sapiens
caattactcagattttattttgg

SEQ ID NO: 901 - DNA, 23 bp, Homo sapiens
tggagggagggaggaaaataagg

SEQ ID NO: 902 - DNA, 23 bp, Homo sapiens
ggggaatgagaaaagaaggaagg

SEQ ID NO: 903 - DNA, 23 bp, Homo sapiens
aagaaggaaggaatggagggagg

SEQ ID NO: 904 - DNA, 23 bp, Homo sapiens
agaaaagaaggaaggaatggagg

SEQ ID NO: 905 - DNA, 23 bp, Homo sapiens
atgagaaaagaaggaaggaatgg

SEQ ID NO: 906 - DNA, 23 bp, Homo sapiens
gaaaagaaggaaggaatggaggg

SEQ ID NO: 907 - DNA, 23 bp, Homo sapiens
agaaggaaggaatggagggaggg

SEQ ID NO: 908 - DNA, 23 bp, Homo sapiens
aggaaggaatggagggagggagg

SEQ ID NO: 909 - DNA, 23 bp, Homo sapiens
tacttgaaccctagagtcggagg

SEQ ID NO: 910 - DNA, 23 bp, Homo sapiens
gagcattcgctatattgcccagg

SEQ ID NO: 911 - DNA, 23 bp, Homo sapiens
gcggtctccctatgttgagcagg

SEQ ID NO: 912 - DNA, 23 bp, Homo sapiens
aactgcagcctccgactctaggg

SEQ ID NO: 913 - DNA, 23 bp, Homo sapiens
caagctagcactaccacgcctgg

SEQ ID NO: 914 - DNA, 23 bp, Homo sapiens
ctcacctataatggccactaagg

SEQ ID NO: 915 - DNA, 23 bp, Homo sapiens
ggggtttcaccacattagccagg

SEQ ID NO: 916 - DNA, 23 bp, Homo sapiens
aggtcagatcgagatcatcctgg

SEQ ID NO: 917 - DNA, 23 bp, Homo sapiens
ctcacctataatggccactaagg

SEQ ID NO: 918 - DNA, 23 bp, Homo sapiens
cacctataatggccactaagggg

SEQ ID NO: 919 - DNA, 23 bp, Homo sapiens
taactgcagcctccgactctagg

SEQ ID NO: 920 - DNA, 23 bp, Homo sapiens
tcacctataatggccactaaggg

SEQ ID NO: 921 - DNA, 23 bp, Homo sapiens
taaaaataagggtcgggtgaggg

SEQ ID NO: 922 - DNA, 23 bp, Homo sapiens
ttccccttagtggccattatagg

SEQ ID NO: 923 - DNA, 23 bp, Homo sapiens
gcaggttggtcttaaactactgg

SEQ ID NO: 924 - DNA, 23 bp, Homo sapiens
aggaaggctgttgggtccggtgg

SEQ ID NO: 925 - DNA, 23 bp, Homo sapiens
tctccctatgttgagcaggttgg

SEQ ID NO: 926 - DNA, 23 bp, Homo sapiens
cgagatcatcctggctaatgtgg

SEQ ID NO: 927 - DNA, 23 bp, Homo sapiens
ggatcttgggctgggcgcaatgg

SEQ ID NO: 928 - DNA, 23 bp, Homo sapiens
gcagaggcgggcggatcacaagg

SEQ ID NO: 929 - DNA, 23 bp, Homo sapiens
agaccaacctgctcaacataggg

SEQ ID NO: 930 - DNA, 23 bp, Homo sapiens
caaaaattatccgggcattgtgg

SEQ ID NO: 931 - DNA, 23 bp, Homo sapiens
aattacttgaaccctagagtcgg

SEQ ID NO: 932 - DNA, 23 bp, Homo sapiens
cacagggtctttaattaatctgg

SEQ ID NO: 933 - DNA, 23 bp, Homo sapiens
ctccatggtggcatgcactttgg

SEQ ID NO: 934 - DNA, 23 bp, Homo sapiens
aaaaataagggtcgggtgagggg

SEQ ID NO: 935 - DNA, 23 bp, Homo sapiens
ctgaataaacggggctgcctggg

SEQ ID NO: 936 - DNA, 23 bp, Homo sapiens
tccatggtggcatgcactttggg

SEQ ID NO: 937 - DNA, 23 bp, Homo sapiens
ataaaaataagggtcgggtgagg

SEQ ID NO: 938 - DNA, 23 bp, Homo sapiens
cagaccagcctgaccaacatggg

SEQ ID NO: 939 - DNA, 23 bp, Homo sapiens
aagaccaacctgctcaacatagg

SEQ ID NO: 940 - DNA, 23 bp, Homo sapiens
ctgcccctctgatttgcacctgg

SEQ ID NO: 941 - DNA, 23 bp, Homo sapiens
attagagttctggctgggcgtgg

SEQ ID NO: 942 - DNA, 23 bp, Homo sapiens
tcttcagtactcacctataatgg

SEQ ID NO: 943 - DNA, 23 bp, Homo sapiens
aaaggggcagtaattgtccaagg

SEQ ID NO: 944 - DNA, 23 bp, Homo sapiens
cttaagccctgtactgtgccagg

SEQ ID NO: 945 - DNA, 23 bp, Homo sapiens
tcttcagtactcacctataatgg

SEQ ID NO: 946 - DNA, 23 bp, Homo sapiens
tgtttgagcccaagagattgagg

SEQ ID NO: 947 - DNA, 23 bp, Homo sapiens
tgaatacgatggtgaaactgagg

SEQ ID NO: 948 - DNA, 23 bp, Homo sapiens
tctcattgtgtcacccgggctgg

SEQ ID NO: 949 - DNA, 23 bp, Homo sapiens
gcttgtagttccagctgtttggg

SEQ ID NO: 950 - DNA, 23 bp, Homo sapiens
agcttgtagttccagctgtttgg

SEQ ID NO: 951 - DNA, 23 bp, Homo sapiens
caggctactcttgaactcttggg

SEQ ID NO: 952 - DNA, 23 bp, Homo sapiens
aatcaagccttgttaaaaccagg

SEQ ID NO: 953 - DNA, 23 bp, Homo sapiens
tcccaaagtgcatgccaccatgg

SEQ ID NO: 954 - DNA, 23 bp, Homo sapiens
agcttgtaaacttagcactttgg

SEQ ID NO: 955 - DNA, 23 bp, Homo sapiens
gggcttaagaaataggatcttgg

SEQ ID NO: 956 - DNA, 23 bp, Homo sapiens
agagccaccgtactccagcccgg

SEQ ID NO: 957 - DNA, 23 bp, Homo sapiens
tcacccgggctggagtacggtgg

SEQ ID NO: 958 - DNA, 23 bp, Homo sapiens
gatttgatgagatctcacagcgg

SEQ ID NO: 959 - DNA, 23 bp, Homo sapiens
tgaaactgaggtcctagcttagg

SEQ ID NO: 960 - DNA, 23 bp, Homo sapiens
tcacatataaatgaatacgatgg

SEQ ID NO: 961 - DNA, 23 bp, Homo sapiens
agcaagctgtgacttgttctagg

SEQ ID NO: 962 - DNA, 23 bp, Homo sapiens
atggtggcatgcactttgggagg

SEQ ID NO: 963 - DNA, 23 bp, Homo sapiens
ccatgttggtcaggctggtctgg

SEQ ID NO: 964 - DNA, 23 bp, Homo sapiens
agttgccaaaacttgctatttgg

SEQ ID NO: 965 - DNA, 23 bp, Homo sapiens
ggcttaagaaataggatcttggg

SEQ ID NO: 966 - DNA, 23 bp, Homo sapiens
ccagtttctctctgtcgcccagg

SEQ ID NO: 967 - DNA, 23 bp, Homo sapiens
actgaataaacggggctgcctgg

SEQ ID NO: 968 - DNA, 23 bp, Homo sapiens
atcacacaaattaagagtacagg

SEQ ID NO: 969 - DNA, 23 bp, Homo sapiens
caagagttcaagagtagcctggg

SEQ ID NO: 970 - DNA, 23 bp, Homo sapiens
cactgcagcctcaatctcttggg

SEQ ID NO: 971 - DNA, 23 bp, Homo sapiens
taagaaataggatcttgggctgg

SEQ ID NO: 972 - DNA, 23 bp, Homo sapiens
cagtacagggcttaagaaatagg

SEQ ID NO: 973 - DNA, 23 bp, Homo sapiens
ctgaggcagaggcctaagctagg

SEQ ID NO: 974 - DNA, 23 bp, Homo sapiens
aaaataagggtcgggtgaggggg

SEQ ID NO: 975 - DNA, 23 bp, Homo sapiens
tacaggaaggctgttgggtccgg

SEQ ID NO: 976 - DNA, 23 bp, Homo sapiens
acagaaaaattagccaggcgtgg

SEQ ID NO: 977 - DNA, 23 bp, Homo sapiens
ataggtgagtactgaagaccagg

SEQ ID NO: 978 - DNA, 23 bp, Homo sapiens
ccaagagttcaagagtagcctgg

SEQ ID NO: 979 - DNA, 23 bp, Homo sapiens
acagagtgagaactccatggtgg

SEQ ID NO: 980 - DNA, 23 bp, Homo sapiens
gcaaccacctcctgggttcaagg

SEQ ID NO: 981 - DNA, 23 bp, Homo sapiens
caaggtgggtgcatcacctgagg

SEQ ID NO: 982 - DNA, 23 bp, Homo sapiens
aaaaaattagcctggtgtagtgg

SEQ ID NO: 983 - DNA, 23 bp, Homo sapiens
caggcacatgccactacaccagg

SEQ ID NO: 984 - DNA, 23 bp, Homo sapiens
gcttgtaaacttagcactttggg

SEQ ID NO: 985 - DNA, 23 bp, Homo sapiens
taaaaccaggtgcaaatcagagg

SEQ ID NO: 986 - DNA, 23 bp, Homo sapiens
ctggaggattgtctgagcccagg

SEQ ID NO: 987 - DNA, 23 bp, Homo sapiens
ggtcttgaactcctgacctcagg

SEQ ID NO: 988 - DNA, 23 bp, Homo sapiens
agcggcccattttacagagaagg

SEQ ID NO: 989 - DNA, 23 bp, Homo sapiens
tcactgcagctttgaattcctgg

SEQ ID NO: 990 - DNA, 23 bp, Homo sapiens
ggctcactgcaaccacctcctgg

SEQ ID NO: 991 - DNA, 23 bp, Homo sapiens
cacaaattaagagtacaggaagg

SEQ ID NO: 992 - DNA, 23 bp, Homo sapiens
tactcagcatcccaaacagctgg

SEQ ID NO: 993 - DNA, 23 bp, Homo sapiens
ctctccctgattttacaaacagg

SEQ ID NO: 994 - DNA, 23 bp, Homo sapiens
tggggtctcattgtgtcacccgg

SEQ ID NO: 995 - DNA, 23 bp, Homo sapiens
aagagtacaggaaggctgttggg

SEQ ID NO: 996 - DNA, 23 bp, Homo sapiens
gcctgtggtcccaggtactcagg

SEQ ID NO: 997 - DNA, 23 bp, Homo sapiens
gaaactgtgtttacaaactgtgg

SEQ ID NO: 998 - DNA, 23 bp, Homo sapiens
agctggggggactgaataaacgg

SEQ ID NO: 999 - DNA, 23 bp, Homo sapiens
tgggtgcatcacctgaggtcagg

SEQ ID NO: 1000 - DNA, 23 bp, Homo sapiens
tttaaaattagagttctggctgg

SEQ ID NO: 1001 - DNA, 23 bp, Homo sapiens
atttgcacctggttttaacaagg

SEQ ID NO: 1002 - DNA, 23 bp, Homo sapiens
catgtgcaaaaccctgagcctgg

SEQ ID NO: 1003 - DNA, 23 bp, Homo sapiens
gcaacagagtgagaactccatgg

SEQ ID NO: 1004 - DNA, 23 bp, Homo sapiens
cactgcagctttgaattcctggg

SEQ ID NO: 1005 - DNA, 23 bp, Homo sapiens
agctgtttgggatgctgagtagg

SEQ ID NO: 1006 - DNA, 23 bp, Homo sapiens
ttaaaattagagttctggctggg

SEQ ID NO: 1007 - DNA, 23 bp, Homo sapiens
ccctgagcctggcacagtacagg

SEQ ID NO: 1008 - DNA, 23 bp, Homo sapiens
cctgggcgacagagagaaactgg

SEQ ID NO: 1009 - DNA, 23 bp, Homo sapiens
gggattttaccatgttggtcagg

SEQ ID NO: 1010 - DNA, 23 bp, Homo sapiens
gtgacttgttctaggtcatatgg

SEQ ID NO: 1011 - DNA, 23 bp, Homo sapiens
aagaaataggatcttgggctggg

SEQ ID NO: 1012 - DNA, 23 bp, Homo sapiens
taagagtacaggaaggctgttgg

SEQ ID NO: 1013 - DNA, 23 bp, Homo sapiens
ggtgtagtggcatgtgcctgtgg

SEQ ID NO: 1014 - DNA, 23 bp, Homo sapiens
tgtaaacttagcactttgggagg

SEQ ID NO: 1015 - DNA, 23 bp, Homo sapiens
caggtgcaaatcagaggggcagg

SEQ ID NO: 1016 - DNA, 23 bp, Homo sapiens
ttgggaaatggtatgaggtaggg

SEQ ID NO: 1017 - DNA, 23 bp, Homo sapiens
cctgggtcctcgggcctcctggg

SEQ ID NO: 1018 - DNA, 23 bp, Homo sapiens
gagccaccgtactccagcccggg

SEQ ID NO: 1019 - DNA, 23 bp, Homo sapiens
agagttctggctgggcgtggtgg

SEQ ID NO: 1020 - DNA, 23 bp, Homo sapiens
ctgaagaccaggaacttctgagg

SEQ ID NO: 1021 - DNA, 23 bp, Homo sapiens
tcctgagtacctgggaccacagg

SEQ ID NO: 1022 - DNA, 23 bp, Homo sapiens
gggaaggaggaaaatcaccttgg

SEQ ID NO: 1023 - DNA, 23 bp, Homo sapiens
tgtttgtaatcccaacactttgg

SEQ ID NO: 1024 - DNA, 23 bp, Homo sapiens
gctcactgcaaccacctcctggg

SEQ ID NO: 1025 - DNA, 23 bp, Homo sapiens
tttgggaaatggtatgaggtagg

SEQ ID NO: 1026 - DNA, 23 bp, Homo sapiens
cttttccaaatagcaagttttgg

SEQ ID NO: 1027 - DNA, 23 bp, Homo sapiens
aaacacagtttcaaaaggtcagg

SEQ ID NO: 1028 - DNA, 23 bp, Homo sapiens
aaaccaggtgcaaatcagagggg

SEQ ID NO: 1029 - DNA, 23 bp, Homo sapiens
ggtctggaactcctgacctcagg

SEQ ID NO: 1030 - DNA, 23 bp, Homo sapiens
aaaaccaggtgcaaatcagaggg

SEQ ID NO: 1031 - DNA, 23 bp, Homo sapiens
tgggagccccagaagatgaaagg

SEQ ID NO: 1032 - DNA, 23 bp, Homo sapiens
tttcatcttctggggctcccagg

SEQ ID NO: 1033 - DNA, 23 bp, Homo sapiens
gcctgggtcctcgggcctcctgg

SEQ ID NO: 1034 - DNA, 23 bp, Homo sapiens
caggtgcgtcccaccacacccgg

SEQ ID NO: 1035 - DNA, 23 bp, Homo sapiens
gtttgtaatcccaacactttggg

SEQ ID NO: 1036 - DNA, 23 bp, Homo sapiens
aatgaataaaaataagggtcggg

SEQ ID NO: 1037 - DNA, 23 bp, Homo sapiens
tatttgtcttggggtaaggaagg

SEQ ID NO: 1038 - DNA, 23 bp, Homo sapiens
acctcagcctcctgagtacctgg

SEQ ID NO: 1039 - DNA, 23 bp, Homo sapiens
tcactgcagcctcaatctcttgg

SEQ ID NO: 1040 - DNA, 23 bp, Homo sapiens
tttaagtaatgagatgggagggg

SEQ ID NO: 1041 - DNA, 23 bp, Homo sapiens
cctgagcctggcacagtacaggg

SEQ ID NO: 1042 - DNA, 23 bp, Homo sapiens
tgaggcagagggatcacctgagg

SEQ ID NO: 1043 - DNA, 23 bp, Homo sapiens
aatatatttgtcttggggtaagg

SEQ ID NO: 1044 - DNA, 23 bp, Homo sapiens
gcctctgcctcagaagttcctgg

SEQ ID NO: 1045 - DNA, 23 bp, Homo sapiens
ccaggctactcttgaactcttgg

SEQ ID NO: 1046 - DNA, 23 bp, Homo sapiens
cccaggaggcccgaggacccagg

SEQ ID NO: 1047 - DNA, 23 bp, Homo sapiens
gggagccccagaagatgaaaggg

SEQ ID NO: 1048 - DNA, 23 bp, Homo sapiens
gtgtcacccgggctggagtacgg

SEQ ID NO: 1049 - DNA, 23 bp, Homo sapiens
caggcacacaccacaatgcccgg

SEQ ID NO: 1050 - DNA, 23 bp, Homo sapiens
ctcaggtgatgcacccaccttgg

SEQ ID NO: 1051 - DNA, 23 bp, Homo sapiens
tttttaagtaatgagatgggagg

SEQ ID NO: 1052 - DNA, 23 bp, Homo sapiens
cagagggatcacctgaggtcagg

SEQ ID NO: 1053 - DNA, 23 bp, Homo sapiens
caggagaatcccttgaacccagg

SEQ ID NO: 1054 - DNA, 23 bp, Homo sapiens
gctatttaaaattagagttctgg

SEQ ID NO: 1055 - DNA, 23 bp, Homo sapiens
accaggaacttctgaggcagagg

SEQ ID NO: 1056 - DNA, 23 bp, Homo sapiens
cttagcactttgggaggccgagg

SEQ ID NO: 1057 - DNA, 23 bp, Homo sapiens
catcttctggggctcccaggagg

SEQ ID NO: 1058 - DNA, 23 bp, Homo sapiens
aaaaattagccgggtgtggtggg

SEQ ID NO: 1059 - DNA, 23 bp, Homo sapiens
acggggctgcctgggtcctcggg

SEQ ID NO: 1060 - DNA, 23 bp, Homo sapiens
atgctaaaagacaaaactagagg

SEQ ID NO: 1061 - DNA, 23 bp, Homo sapiens
aattaatctggaagttgttttgg

SEQ ID NO: 1062 - DNA, 23 bp, Homo sapiens
ttgttttgggaaatggtatgagg

SEQ ID NO: 1063 - DNA, 23 bp, Homo sapiens
attaatctggaagttgttttggg

SEQ ID NO: 1064 - DNA, 23 bp, Homo sapiens
ttaagtaatgagatgggaggggg

SEQ ID NO: 1065 - DNA, 23 bp, Homo sapiens
agtttcctgtttgtaaaatcagg

SEQ ID NO: 1066 - DNA, 23 bp, Homo sapiens
aaaaaaaaattagccgggtgtgg

SEQ ID NO: 1067 - DNA, 23 bp, Homo sapiens
caaccacctcctgggttcaaggg

SEQ ID NO: 1068 - DNA, 23 bp, Homo sapiens
gagatgggattttaccatgttgg

SEQ ID NO: 1069 - DNA, 23 bp, Homo sapiens
taataaaattacagagttctggg

SEQ ID NO: 1070 - DNA, 23 bp, Homo sapiens
cgaggtgggaggattgcttgagg

SEQ ID NO: 1071 - DNA, 23 bp, Homo sapiens
aacggggctgcctgggtcctcgg

SEQ ID NO: 1072 - DNA, 23 bp, Homo sapiens
tggggctcccaggaggcccgagg

SEQ ID NO: 1073 - DNA, 23 bp, Homo sapiens
aaaaaattagccgggtgtggtgg

SEQ ID NO: 1074 - DNA, 23 bp, Homo sapiens
gcatgcactttgggaggctgagg

SEQ ID NO: 1075 - DNA, 23 bp, Homo sapiens
gagacagggtttccccatgttgg

SEQ ID NO: 1076 - DNA, 23 bp, Homo sapiens
tagaggacaaatgatagtactgg

SEQ ID NO: 1077 - DNA, 23 bp, Homo sapiens
aacttccctttcatcttctgggg

SEQ ID NO: 1078 - DNA, 23 bp, Homo sapiens
ccaacttccctttcatcttctgg

SEQ ID NO: 1079 - DNA, 23 bp, Homo sapiens
gcaccactgcactccggcctggg

SEQ ID NO: 1080 - DNA, 23 bp, Homo sapiens
ggagtgcagtggtgcaatctcgg

SEQ ID NO: 1081 - DNA, 23 bp, Homo sapiens
atactatattgcaaatattctgg

SEQ ID NO: 1082 - DNA, 23 bp, Homo sapiens
ttgctcaggcaggagtgcagtgg

SEQ ID NO: 1083 - DNA, 23 bp, Homo sapiens
caacttccctttcatcttctggg

SEQ ID NO: 1084 - DNA, 23 bp, Homo sapiens
tggcatgtgcctgtggtcccagg

SEQ ID NO: 1085 - DNA, 23 bp, Homo sapiens
cagaagatgaaagggaagttggg

SEQ ID NO: 1086 - DNA, 23 bp, Homo sapiens
ggggtctcattgtgtcacccggg

SEQ ID NO: 1087 - DNA, 23 bp, Homo sapiens
ataataaaattacagagttctgg

SEQ ID NO: 1088 - DNA, 23 bp, Homo sapiens
gcctcagcctcccaaagtgttgg

SEQ ID NO: 1089 - DNA, 23 bp, Homo sapiens
ctggaagttgttttgggaaatgg

SEQ ID NO: 1090 - DNA, 23 bp, Homo sapiens
agggtttccccatgttggtcagg

SEQ ID NO: 1091 - DNA, 23 bp, Homo sapiens
aaaaaaaagtctgggtgtggtgg

SEQ ID NO: 1092 - DNA, 23 bp, Homo sapiens
gtttcctgtttgtaaaatcaggg

SEQ ID NO: 1093 - DNA, 23 bp, Homo sapiens
ttgtaaaatcagggagagactgg

SEQ ID NO: 1094 - DNA, 23 bp, Homo sapiens
caagagaatcgcttgaacccagg

SEQ ID NO: 1095 - DNA, 23 bp, Homo sapiens
acaacttaagaaatttgaagtgg

SEQ ID NO: 1096 - DNA, 23 bp, Homo sapiens
agtaatgagatgggagggggcgg

SEQ ID NO: 1097 - DNA, 23 bp, Homo sapiens
tttgtaaacacagtttcaaaagg

SEQ ID NO: 1098 - DNA, 23 bp, Homo sapiens
gatgaaagggaagttggggaagg

SEQ ID NO: 1099 - DNA, 23 bp, Homo sapiens
ggaaactgaggctaagaaagggg

SEQ ID NO: 1100 - DNA, 23 bp, Homo sapiens
gcctcagcctcctgagtagctgg

SEQ ID NO: 1101 - DNA, 23 bp, Homo sapiens
ttatttttaagtaatgagatggg

SEQ ID NO: 1102 - DNA, 23 bp, Homo sapiens
aggaaactgaggctaagaaaggg

SEQ ID NO: 1103 - DNA, 23 bp, Homo sapiens
tactgcaacctctgcctcctggg

SEQ ID NO: 1104 - DNA, 23 bp, Homo sapiens
aatcccttgaacccaggaggtgg

SEQ ID NO: 1105 - DNA, 23 bp, Homo sapiens
aaaagtattcaaaaaactatagg

SEQ ID NO: 1106 - DNA, 23 bp, Homo sapiens
tcctgagtagctgggattacagg

SEQ ID NO: 1107 - DNA, 23 bp, Homo sapiens
ccctgtactgtgccaggctcagg

SEQ ID NO: 1108 - DNA, 23 bp, Homo sapiens
gcctctgcctcccaaagtgctgg

SEQ ID NO: 1109 - DNA, 23 bp, Homo sapiens
ccagaagatgaaagggaagttgg

SEQ ID NO: 1110 - DNA, 23 bp, Homo sapiens
ctttgggaggcagaggcgggcgg

SEQ ID NO: 1111 - DNA, 23 bp, Homo sapiens
ataggaaaatatatttgtcttgg

SEQ ID NO: 1112 - DNA, 23 bp, Homo sapiens
aggaaaatatatttgtcttgggg

SEQ ID NO: 1113 - DNA, 23 bp, Homo sapiens
cctcagcctcctgagtacctggg

SEQ ID NO: 1114 - DNA, 23 bp, Homo sapiens
attatttttaagtaatgagatgg

SEQ ID NO: 1115 - DNA, 23 bp, Homo sapiens
caggaaactgaggctaagaaagg

SEQ ID NO: 1116 - DNA, 23 bp, Homo sapiens
cctcagcctcccaaagtgttggg

SEQ ID NO: 1117 - DNA, 23 bp, Homo sapiens
taggaaaatatatttgtcttggg

SEQ ID NO: 1118 - DNA, 23 bp, Homo sapiens
ttttaagtaatgagatgggaggg

SEQ ID NO: 1119 - DNA, 23 bp, Homo sapiens
agaagatgaaagggaagttgggg

SEQ ID NO: 1120 - DNA, 23 bp, Homo sapiens
gagaatcgcttgaacccaggagg

SEQ ID NO: 1121 - DNA, 23 bp, Homo sapiens
tgcaccactgcactccggcctgg

SEQ ID NO: 1122 - DNA, 23 bp, Homo sapiens
atataaaataaaaagttgtatgg

SEQ ID NO: 1123 - DNA, 23 bp, Homo sapiens
ttactgcaacctctgcctcctgg

SEQ ID NO: 1124 - DNA, 23 bp, Homo sapiens
gagaatcccttgaacccaggagg

SEQ ID NO: 1125 - DNA, 23 bp, Homo sapiens
tttctctctgtcgcccaggccgg

SEQ ID NO: 1126 - DNA, 23 bp, Homo sapiens
aaaaaaaaaaagtctgggtgtgg

SEQ ID NO: 1127 - DNA, 23 bp, Homo sapiens
attttacaaacaggaaactgagg

SEQ ID NO: 1128 - DNA, 23 bp, Homo sapiens
gcactttgggaggcagaggcggg

SEQ ID NO: 1129 - DNA, 23 bp, Homo sapiens
tttctgtttttagtagagatggg

SEQ ID NO: 1130 - DNA, 23 bp, Homo sapiens
tgtaatcccagctactcaggagg

SEQ ID NO: 1131 - DNA, 23 bp, Homo sapiens
taaaaatacaaaaattatccggg

SEQ ID NO: 1132 - DNA, 23 bp, Homo sapiens
agcactttgggaggcagaggcgg

SEQ ID NO: 1133 - DNA, 23 bp, Homo sapiens
ttttattcatttttagagatggg

SEQ ID NO: 1134 - DNA, 23 bp, Homo sapiens
aaatgaataaaaataagggtcgg

SEQ ID NO: 1135 - DNA, 23 bp, Homo sapiens
cccagcactttgggaggcagagg

SEQ ID NO: 1136 - DNA, 23 bp, Homo sapiens
tcctgagtagctgggactacagg

SEQ ID NO: 1137 - DNA, 23 bp, Homo sapiens
tttattcatttttagagatgggg

SEQ ID NO: 1138 - DNA, 23 bp, Homo sapiens
ctttgggaggctgaggcagaggg

SEQ ID NO: 1139 - DNA, 23 bp, Homo sapiens
gagattgcaccactgcactccgg

SEQ ID NO: 1140 - DNA, 23 bp, Homo sapiens
ctttgggaggccgaggtgggagg

SEQ ID NO: 1141 - DNA, 23 bp, Homo sapiens
ctcaagcaatcctcccacctcgg

SEQ ID NO: 1142 - DNA, 23 bp, Homo sapiens
ctttgggaggccgaggtgggagg

SEQ ID NO: 1143 - DNA, 23 bp, Homo sapiens
ctcaagcaatcctcccacctcgg

SEQ ID NO: 1144 - DNA, 23 bp, Homo sapiens
taaaaacagaaaaattagccagg

SEQ ID NO: 1145 - DNA, 23 bp, Homo sapiens
tatttggaaaagaaaaatgttgg

SEQ ID NO: 1146 - DNA, 23 bp, Homo sapiens
aggtactcaggaggctgaggtgg

SEQ ID NO: 1147 - DNA, 23 bp, Homo sapiens
cccaggtactcaggaggctgagg

SEQ ID NO: 1148 - DNA, 23 bp, Homo sapiens
catttccttctctgtaaaatggg

SEQ ID NO: 1149 - DNA, 23 bp, Homo sapiens
ctaaaaatacaaaaattatccgg

SEQ ID NO: 1150 - DNA, 23 bp, Homo sapiens
tcgcccaggccggagtgcagtgg

SEQ ID NO: 1151 - DNA, 23 bp, Homo sapiens
ttttaccatgttggtcaggctgg

SEQ ID NO: 1152 - DNA, 23 bp, Homo sapiens
tactcaggaggctgaggtggagg

SEQ ID NO: 1153 - DNA, 23 bp, Homo sapiens
agtgctgggattacagacgttgg

SEQ ID NO: 1154 - DNA, 23 bp, Homo sapiens
cctctgcctcccaaagtgctggg

SEQ ID NO: 1155 - DNA, 23 bp, Homo sapiens
ctttgggaggctgaggctggagg

SEQ ID NO: 1156 - DNA, 23 bp, Homo sapiens
gtttaaaaaaaaagaaacacagg

SEQ ID NO: 1157 - DNA, 23 bp, Homo sapiens
gcgccactgcactccagcctggg

SEQ ID NO: 1158 - DNA, 23 bp, Homo sapiens
cgcgccactgcactccagcctgg

SEQ ID NO: 1159 - DNA, 23 bp, Homo sapiens
tttttattcatttttagagatgg

SEQ ID NO: 1160 - DNA, 23 bp, Homo sapiens
actttgggaggctgaggcagagg

SEQ ID NO: 1161 - DNA, 23 bp, Homo sapiens
cccaacactttgggaggctgagg

SEQ ID NO: 1162 - DNA, 23 bp, Homo sapiens
acctcggcctcccaaagtgctgg

SEQ ID NO: 1163 - DNA, 23 bp, Homo sapiens
agggtcttgctctgttgctcagg

SEQ ID NO: 1164 - DNA, 23 bp, Homo sapiens
gaaagggaagttggggaaggagg

SEQ ID NO: 1165 - DNA, 23 bp, Homo sapiens
ggagtcttgcactgtcacccagg

SEQ ID NO: 1166 - DNA, 23 bp, Homo sapiens
ccatttccttctctgtaaaatgg

SEQ ID NO: 1167 - DNA, 23 bp, Homo sapiens
ccattttacagagaaggaaatgg

SEQ ID NO: 1168 - DNA, 23 bp, Homo sapiens
ccagaccagcctgaccaacatgg

SEQ ID NO: 1169 - DNA, 23 bp, Homo sapiens
tttccccatgttggtcaggctgg

SEQ ID NO: 1170 - DNA, 23 bp, Homo sapiens
ggattacagctgtgagccaccgg

SEQ ID NO: 1171 - DNA, 23 bp, Homo sapiens
agcactttgggaggccgaggtgg

SEQ ID NO: 1172 - DNA, 23 bp, Homo sapiens
cgcttgaacccaggaggcagagg

SEQ ID NO: 1173 - DNA, 23 bp, Homo sapiens
cccagctactcaggaggctgagg

SEQ ID NO: 1174 - DNA, 23 bp, Homo sapiens
tctaaaaatgaataaaaataagg

SEQ ID NO: 1175 - DNA, 23 bp, Homo sapiens
gctactcaggaggctgaggcagg

SEQ ID NO: 1176 - DNA, 23 bp, Homo sapiens
caagaccagcctgaccaacatgg

SEQ ID NO: 1177 - DNA, 23 bp, Homo sapiens
acaaacaaaaaaaactcttttgg

SEQ ID NO: 1178 - DNA, 23 bp, Homo sapiens
cctcagcctcctgagtagctggg

SEQ ID NO: 1179 - DNA, 23 bp, Homo sapiens
acctgtaatcccagctactcagg

SEQ ID NO: 1180 - DNA, 23 bp, Homo sapiens
tcttgcactgtcacccaggctgg

SEQ ID NO: 1181 - DNA, 23 bp, Homo sapiens
ttttttttttagtagagacgggg

SEQ ID NO: 1182 - DNA, 23 bp, Homo sapiens
cctcagcctcctgagtagctggg

SEQ ID NO: 1183 - DNA, 23 bp, Homo sapiens
agaccagcctgaccaacatgggg

SEQ ID NO: 1184 - DNA, 23 bp, Homo sapiens
cagctgtaatcccagcactttgg

SEQ ID NO: 1185 - DNA, 23 bp, Homo sapiens
tttttttttttagtagagacggg

SEQ ID NO: 1186 - DNA, 23 bp, Homo sapiens
gcactttgggaggctgaggctgg

SEQ ID NO: 1187 - DNA, 23 bp, Homo sapiens
gcctgtagtcccagctactcagg

SEQ ID NO: 1188 - DNA, 23 bp, Homo sapiens
gcactttgggaggccaaggtggg

SEQ ID NO: 1189 - DNA, 23 bp, Homo sapiens
cgtctgtaatcccagcactttgg

SEQ ID NO: 1190 - DNA, 23 bp, Homo sapiens
tcttgctctgttgctcaggcagg

SEQ ID NO: 1191 - DNA, 23 bp, Homo sapiens
tgtaatcccaacactttgggagg

SEQ ID NO: 1192 - DNA, 23 bp, Homo sapiens
ctaaaaatgaataaaaataaggg

SEQ ID NO: 1193 - DNA, 23 bp, Homo sapiens
ttttctgtttttagtagagatgg

SEQ ID NO: 1194 - DNA, 23 bp, Homo sapiens
cccagcactttgggaggccgagg

SEQ ID NO: 1195 - DNA, 23 bp, Homo sapiens
tttaaaaaaaaagaaacacaggg

SEQ ID NO: 1196 - DNA, 23 bp, Homo sapiens
tgtggtcccaggtactcaggagg

SEQ ID NO: 1197 - DNA, 23 bp, Homo sapiens
agctgtaatcccagcactttggg

SEQ ID NO: 1198 - DNA, 23 bp, Homo sapiens
catgccactgcactccagcctgg

SEQ ID NO: 1199 - DNA, 23 bp, Homo sapiens
taaaaaaaaaaaaattagcctgg

SEQ ID NO: 1200 - DNA, 23 bp, Homo sapiens
atgccactgcactccagcctggg

SEQ ID NO: 1201 - DNA, 23 bp, Homo sapiens
accttggcctcccaaagtgctgg

SEQ ID NO: 1202 - DNA, 23 bp, Homo sapiens
cctcggcctcccaaagtgctggg

SEQ ID NO: 1203 - DNA, 23 bp, Homo sapiens
gtctgtaatcccagcactttggg

SEQ ID NO: 1204 - DNA, 23 bp, Homo sapiens
cccagcactttgggaggccaagg

SEQ ID NO: 1205 - DNA, 23 bp, Homo sapiens
cacctgtaatcccagcactttgg

SEQ ID NO: 1206 - DNA, 23 bp, Homo sapiens
ttgtttgtttgtttttgaagtgg

SEQ ID NO: 1207 - DNA, 23 bp, Homo sapiens
ttgcccaggctggagtgcagtgg

SEQ ID NO: 1208 - DNA, 23 bp, Homo sapiens
agcactttgggaggccaaggtgg

SEQ ID NO: 1209 - DNA, 23 bp, Homo sapiens
aaaaaaaaaaaaaattagccggg

SEQ ID NO: 1210 - DNA, 23 bp, Homo sapiens
tcacccaggctggagtgcagtgg

SEQ ID NO: 1211 - DNA, 23 bp, Homo sapiens
ttttttttttttagtagagacgg

SEQ ID NO: 1212 - DNA, 23 bp, Homo sapiens
ttgtatttttagtagagacaggg

SEQ ID NO: 1213 - DNA, 23 bp, Homo sapiens
aataaataaataaaataaatagg

SEQ ID NO: 1214 - DNA, 23 bp, Homo sapiens
tgtagtcccagctactcaggagg

SEQ ID NO: 1215 - DNA, 23 bp, Homo sapiens
ccttggcctcccaaagtgctggg

SEQ ID NO: 1216 - DNA, 23 bp, Homo sapiens
aaaaaaaaaaaaaaattagccgg

SEQ ID NO: 1217 - DNA, 23 bp, Homo sapiens
tctcactctgttgcccaggctgg

SEQ ID NO: 1218 - DNA, 23 bp, Homo sapiens
acctgtaatcccagcactttggg

SEQ ID NO: 1219 - DNA, 23 bp, Homo sapiens
tgtaatcccagcactttgggagg

SEQ ID NO: 1220 - DNA, 23 bp, Homo sapiens
tttgtatttttagtagagacagg

SEQ ID NO: 1221 - DNA, 23 bp, Homo sapiens
tcccaaagtgctgggattacagg

SEQ ID NO: 1222 - DNA, 23 bp, Homo sapiens
ttttttttttttttgaggcaggg

SEQ ID NO: 1223 - DNA, 23 bp, Homo sapiens
tttttttttttttttgaggcagg

SEQ ID NO: 1224 - DNA, 23 bp, Homo sapiens
aaaaaaaaaaaaaaaagtctggg

SEQ ID NO: 1225 - DNA, 23 bp, Homo sapiens
aaaaaaaaaaaaaaaaagtctgg

SEQ ID NO: 1226 - DNA, 23 bp, Homo sapiens
tttttttttttttttttttgagg

SEQ ID NO: 1227 - DNA, 23 bp, Homo sapiens
tccaaatctccaagcgggttggg

SEQ ID NO: 1228 - DNA, 23 bp, Homo sapiens
ccaaatctccaagcgggttgggg

SEQ ID NO: 1229 - DNA, 23 bp, Homo sapiens
gtccaaatctccaagcgggttgg

SEQ ID NO: 1230 - DNA, 23 bp, Homo sapiens
ccggctacagttgtgacccctgg

SEQ ID NO: 1231 - DNA, 23 bp, Homo sapiens
ccccaacccgcttggagatttgg

SEQ ID NO: 1232 - DNA, 23 bp, Homo sapiens
gccgggcaccccaacccgcttgg

SEQ ID NO: 1233 - DNA, 23 bp, Homo sapiens
cggctacagttgtgacccctggg

SEQ ID NO: 1234 - DNA, 23 bp, Homo sapiens
ctcaaggtcacgttgaccccagg

SEQ ID NO: 1235 - DNA, 23 bp, Homo sapiens
ccgggatgtgtcctccgagctgg

SEQ ID NO: 1236 - DNA, 23 bp, Homo sapiens
ttggggtgcccggcatctcaagg

SEQ ID NO: 1237 - DNA, 23 bp, Homo sapiens
aaagaattctgccagctcggagg

SEQ ID NO: 1238 - DNA, 23 bp, Homo sapiens
agcagctccaggacatcgctggg

SEQ ID NO: 1239 - DNA, 23 bp, Homo sapiens
tcaacgtgaccttgagatgccgg

SEQ ID NO: 1240 - DNA, 23 bp, Homo sapiens
gcttagggtggtatgaagctggg

SEQ ID NO: 1241 - DNA, 23 bp, Homo sapiens
cttcataccaccctaagccatgg

SEQ ID NO: 1242 - DNA, 23 bp, Homo sapiens
ccaggggtcacaactgtagccgg

SEQ ID NO: 1243 - DNA, 23 bp, Homo sapiens
gctgctaccgaaggccagactgg

SEQ ID NO: 1244 - DNA, 23 bp, Homo sapiens
ctgctaccgaaggccagactggg

SEQ ID NO: 1245 - DNA, 23 bp, Homo sapiens
tcaaggtcacgttgaccccaggg

SEQ ID NO: 1246 - DNA, 23 bp, Homo sapiens
ggcttagggtggtatgaagctgg

SEQ ID NO: 1247 - DNA, 23 bp, Homo sapiens
agaaggggagcgatctctccagg

SEQ ID NO: 1248 - DNA, 23 bp, Homo sapiens
gtcccagcccagcgatgtcctgg

SEQ ID NO: 1249 - DNA, 23 bp, Homo sapiens
ataccaccctaagccatggctgg

SEQ ID NO: 1250 - DNA, 23 bp, Homo sapiens
caacgtgaccttgagatgccggg

SEQ ID NO: 1251 - DNA, 23 bp, Homo sapiens
gagctcccagccatggcttaggg

SEQ ID NO: 1252 - DNA, 23 bp, Homo sapiens
tgctaccgaaggccagactgggg

SEQ ID NO: 1253 - DNA, 23 bp, Homo sapiens
gctaccgaaggccagactggggg

SEQ ID NO: 1254 - DNA, 23 bp, Homo sapiens
caaggtcacgttgaccccagggg

SEQ ID NO: 1255 - DNA, 23 bp, Homo sapiens
taccaccctaagccatggctggg

SEQ ID NO: 1256 - DNA, 23 bp, Homo sapiens
tccaagcgggttggggtgcccgg

SEQ ID NO: 1257 - DNA, 23 bp, Homo sapiens
gctccaggacatcgctgggctgg

SEQ ID NO: 1258 - DNA, 23 bp, Homo sapiens
cttagggtggtatgaagctgggg

SEQ ID NO: 1259 - DNA, 23 bp, Homo sapiens
ggctacagttgtgacccctgggg

SEQ ID NO: 1260 - DNA, 23 bp, Homo sapiens
ccagctcggaggacacatcccgg

SEQ ID NO: 1261 - DNA, 23 bp, Homo sapiens
agatcgctccccttctcttccgg

SEQ ID NO: 1262 - DNA, 23 bp, Homo sapiens
tgagctcccagccatggcttagg

SEQ ID NO: 1263 - DNA, 23 bp, Homo sapiens
cagcagctccaggacatcgctgg

SEQ ID NO: 1264 - DNA, 23 bp, Homo sapiens
agatttggacttttcaagcctgg

SEQ ID NO: 1265 - DNA, 23 bp, Homo sapiens
aggacacatcccggaagagaagg

SEQ ID NO: 1266 - DNA, 23 bp, Homo sapiens
cagactgggggccgggtgtctgg

SEQ ID NO: 1267 - DNA, 23 bp, Homo sapiens
actgaataaacggggctgcctgg

SEQ ID NO: 1268 - DNA, 23 bp, Homo sapiens
ggacacatcccggaagagaaggg

SEQ ID NO: 1269 - DNA, 23 bp, Homo sapiens
ctcccagccatggcttagggtgg

SEQ ID NO: 1270 - DNA, 23 bp, Homo sapiens
cgagctggcagaattctttctgg

SEQ ID NO: 1271 - DNA, 23 bp, Homo sapiens
aggaggtgactccagcccaaggg

SEQ ID NO: 1272 - DNA, 23 bp, Homo sapiens
cagacacccggcccccagtctgg

SEQ ID NO: 1273 - DNA, 23 bp, Homo sapiens
tagggtggtatgaagctgggggg

SEQ ID NO: 1274 - DNA, 23 bp, Homo sapiens
ttagggtggtatgaagctggggg

SEQ ID NO: 1275 - DNA, 23 bp, Homo sapiens
agcagcggtaacttcccccttgg

SEQ ID NO: 1276 - DNA, 23 bp, Homo sapiens
ctggccttcggtagcagcagcgg

SEQ ID NO: 1277 - DNA, 23 bp, Homo sapiens
gaaaagtccaaatctccaagcgg

SEQ ID NO: 1278 - DNA, 23 bp, Homo sapiens
agctggggggactgaataaacgg

SEQ ID NO: 1279 - DNA, 23 bp, Homo sapiens
gcagcggtaacttcccccttggg

SEQ ID NO: 1280 - DNA, 23 bp, Homo sapiens
agctggggggactgaataaacgg

SEQ ID NO: 1281 - DNA, 23 bp, Homo sapiens
aaaagtccaaatctccaagcggg

SEQ ID NO: 1282 - DNA, 23 bp, Homo sapiens
ctccaggacatcgctgggctggg

SEQ ID NO: 1283 - DNA, 23 bp, Homo sapiens
ccggcccccagtctggccttcgg

SEQ ID NO: 1284 - DNA, 23 bp, Homo sapiens
gacacatcccggaagagaagggg

SEQ ID NO: 1285 - DNA, 23 bp, Homo sapiens
ggaggtgactccagcccaagggg

SEQ ID NO: 1286 - DNA, 23 bp, Homo sapiens
cggtaacttcccccttgggctgg

SEQ ID NO: 1287 - DNA, 23 bp, Homo sapiens
cagaaagaattctgccagctcgg

SEQ ID NO: 1288 - DNA, 23 bp, Homo sapiens
gatcgctccccttctcttccggg

SEQ ID NO: 1289 - DNA, 23 bp, Homo sapiens
tggtgacaggtgaggtcctgggg

SEQ ID NO: 1290 - DNA, 23 bp, Homo sapiens
ctggtgacaggtgaggtcctggg

SEQ ID NO: 1291 - DNA, 23 bp, Homo sapiens
cagcgatgtcctggagctgctgg

SEQ ID NO: 1292 - DNA, 23 bp, Homo sapiens
ctggtgacaggtgaggtcctggg

SEQ ID NO: 1293 - DNA, 23 bp, Homo sapiens
gaggtgactccagcccaaggggg

SEQ ID NO: 1294 - DNA, 23 bp, Homo sapiens
gctggtgacaggtgaggtcctgg

SEQ ID NO: 1295 - DNA, 23 bp, Homo sapiens
ctgggctgggaccagacacccgg

SEQ ID NO: 1296 - DNA, 23 bp, Homo sapiens
ccgaaggccagactgggggccgg

SEQ ID NO: 1297 - DNA, 23 bp, Homo sapiens
caggtgaggtcctggggtcgggg

SEQ ID NO: 1298 - DNA, 23 bp, Homo sapiens
gctggcagaattctttctggagg

SEQ ID NO: 1299 - DNA, 23 bp, Homo sapiens
gccatggctgggagctcagccgg

SEQ ID NO: 1300 - DNA, 23 bp, Homo sapiens
ggcagaattctttctggaggagg

SEQ ID NO: 1301 - DNA, 23 bp, Homo sapiens
gttaccgctgctgctaccgaagg

SEQ ID NO: 1302 - DNA, 23 bp, Homo sapiens
cgaaggccagactgggggccggg

SEQ ID NO: 1303 - DNA, 23 bp, Homo sapiens
gccggctgagctcccagccatgg

SEQ ID NO: 1304 - DNA, 23 bp, Homo sapiens
acaggtgaggtcctggggtcggg

SEQ ID NO: 1305 - DNA, 23 bp, Homo sapiens
gaggaggtgactccagcccaagg

SEQ ID NO: 1306 - DNA, 23 bp, Homo sapiens
ggagctgctggtgacaggtgagg

SEQ ID NO: 1307 - DNA, 23 bp, Homo sapiens
gtcctggagctgctggtgacagg

SEQ ID NO: 1308 - DNA, 23 bp, Homo sapiens
cacctgtcaccagcagctccagg

SEQ ID NO: 1309 - DNA, 23 bp, Homo sapiens
gcgagcggaagacgctcacgcgg

SEQ ID NO: 1310 - DNA, 23 bp, Homo sapiens
ggaagacgctcacgcggccccgg

SEQ ID NO: 1311 - DNA, 23 bp, Homo sapiens
agagacggggtgagagtccgggg

SEQ ID NO: 1312 - DNA, 23 bp, Homo sapiens
agagagagaggtacagtgcgggg

SEQ ID NO: 1313 - DNA, 23 bp, Homo sapiens
agagagaggtacagtgcgggggg

SEQ ID NO: 1314 - DNA, 23 bp, Homo sapiens
cagagacggggtgagagtccggg

SEQ ID NO: 1315 - DNA, 23 bp, Homo sapiens
aaacagagcgagcgagcgagcgg

SEQ ID NO: 1316 - DNA, 23 bp, Homo sapiens
gtgggtggaacaagggagttggg

SEQ ID NO: 1317 - DNA, 23 bp, Homo sapiens
gacagatacagagacactagggg

SEQ ID NO: 1318 - DNA, 23 bp, Homo sapiens
gagagagaggtacagtgcggggg

SEQ ID NO: 1319 - DNA, 23 bp, Homo sapiens
gcagctcctctgcagagacgggg

SEQ ID NO: 1320 - DNA, 23 bp, Homo sapiens
acagatacagagacactaggggg

SEQ ID NO: 1321 - DNA, 23 bp, Homo sapiens
agtgggtggaacaagggagttgg

SEQ ID NO: 1322 - DNA, 23 bp, Homo sapiens
tggtgacaggtgaggtcctgggg

SEQ ID NO: 1323 - DNA, 23 bp, Homo sapiens
tgggtggaacaagggagttgggg

SEQ ID NO: 1324 - DNA, 23 bp, Homo sapiens
tctctgcagaggagctgccgcgg

SEQ ID NO: 1325 - DNA, 23 bp, Homo sapiens
ctggtgacaggtgaggtcctggg

SEQ ID NO: 1326 - DNA, 23 bp, Homo sapiens
gagagagagaggtacagtgcggg

SEQ ID NO: 1327 - DNA, 23 bp, Homo sapiens
gctggtgacaggtgaggtcctgg

SEQ ID NO: 1328 - DNA, 23 bp, Homo sapiens
gcagagacggggtgagagtccgg

SEQ ID NO: 1329 - DNA, 23 bp, Homo sapiens
caggtgaggtcctggggtcgggg

SEQ ID NO: 1330 - DNA, 23 bp, Homo sapiens
ctctcaccccgtctctgcagagg

SEQ ID NO: 1331 - DNA, 23 bp, Homo sapiens
agagagagagaggtacagtgcgg

SEQ ID NO: 1332 - DNA, 23 bp, Homo sapiens
acaggtgaggtcctggggtcggg

SEQ ID NO: 1333 - DNA, 23 bp, Homo sapiens
gggtggaacaagggagttggggg

SEQ ID NO: 1334 - DNA, 23 bp, Homo sapiens
ggcagctcctctgcagagacggg

SEQ ID NO: 1335 - DNA, 23 bp, Homo sapiens
gaggagaagtgggtggaacaagg

SEQ ID NO: 1336 - DNA, 23 bp, Homo sapiens
cacttctcctccccgaccccagg

SEQ ID NO: 1337 - DNA, 23 bp, Homo sapiens
gggagggacagagagatataggg

SEQ ID NO: 1338 - DNA, 23 bp, Homo sapiens
ggggagggacagagagatatagg

SEQ ID NO: 1339 - DNA, 23 bp, Homo sapiens
gacaggtgaggtcctggggtcgg

SEQ ID NO: 1340 - DNA, 23 bp, Homo sapiens
gtgaggtcctggggtcggggagg

SEQ ID NO: 1341 - DNA, 23 bp, Homo sapiens
ggagctgctggtgacaggtgagg

SEQ ID NO: 1342 - DNA, 23 bp, Homo sapiens
tggggtcggggaggagaagtggg

SEQ ID NO: 1343 - DNA, 23 bp, Homo sapiens
gtcctggagctgctggtgacagg

SEQ ID NO: 1344 - DNA, 23 bp, Homo sapiens
tggaacaagggagttgggggagg

SEQ ID NO: 1345 - DNA, 23 bp, Homo sapiens
cggcagctcctctgcagagacgg

SEQ ID NO: 1346 - DNA, 23 bp, Homo sapiens
aaagagagacagagcgaggcggg

SEQ ID NO: 1347 - DNA, 23 bp, Homo sapiens
ggaacaagggagttgggggaggg

SEQ ID NO: 1348 - DNA, 23 bp, Homo sapiens
gaaagagagacagagcgaggcgg

SEQ ID NO: 1349 - DNA, 23 bp, Homo sapiens
agggaaagagagacagagcgagg

SEQ ID NO: 1350 - DNA, 23 bp, Homo sapiens
ggtcggggaggagaagtgggtgg

SEQ ID NO: 1351 - DNA, 23 bp, Homo sapiens
ctggggtcggggaggagaagtgg

SEQ ID NO: 1352 - DNA, 23 bp, Homo sapiens
aggagaagtgggtggaacaaggg

SEQ ID NO: 1353 - DNA, 23 bp, Homo sapiens
aagacagatacagagacactagg

SEQ ID NO: 1354 - DNA, 23 bp, Homo sapiens
acagagaaagcgagagacagagg

SEQ ID NO: 1355 - DNA, 23 bp, Homo sapiens
agaggcagaaggagaaagggagg

SEQ ID NO: 1356 - DNA, 23 bp, Homo sapiens
aaagcgagagacagaggagaagg

SEQ ID NO: 1357 - DNA, 23 bp, Homo sapiens
ctagggggagagagagagacagg

SEQ ID NO: 1358 - DNA, 23 bp, Homo sapiens
cacctgtcaccagcagctccagg

SEQ ID NO: 1359 - DNA, 23 bp, Homo sapiens
agggaggcagagagagaggcagg

SEQ ID NO: 1360 - DNA, 23 bp, Homo sapiens
agagaggcaggcagagagagagg

SEQ ID NO: 1361 - DNA, 23 bp, Homo sapiens
agaaagaggcagaaggagaaagg

SEQ ID NO: 1362 - DNA, 23 bp, Homo sapiens
agggaggcagagagagaggcagg

SEQ ID NO: 1363 - DNA, 23 bp, Homo sapiens
agagggaggcagagagagggagg

SEQ ID NO: 1364 - DNA, 23 bp, Homo sapiens
aggcaggcagagagagaggcagg

SEQ ID NO: 1365 - DNA, 23 bp, Homo sapiens
gaaagaggcagaaggagaaaggg

SEQ ID NO: 1366 - DNA, 23 bp, Homo sapiens
aggcaggcagagagagagggagg

SEQ ID NO: 1367 - DNA, 23 bp, Homo sapiens
agacaggcagagagaaagagagg

SEQ ID NO: 1368 - DNA, 23 bp, Homo sapiens
tagggggagagagagagacaggg

SEQ ID NO: 1369 - DNA, 23 bp, Homo sapiens
agggggagagagagagacagggg

SEQ ID NO: 1370 - DNA, 23 bp, Homo sapiens
aggggagcagagagagagagagg

SEQ ID NO: 1371 - DNA, 23 bp, Homo sapiens
gagaggcaggcagagagagaggg

SEQ ID NO: 1372 - DNA, 23 bp, Homo sapiens
agaaagggaggcagagagagagg

SEQ ID NO: 1373 - DNA, 23 bp, Homo sapiens
aggcagacagagagagagacagg

SEQ ID NO: 1374 - DNA, 23 bp, Homo sapiens
agagagagggaggcagagagagg

SEQ ID NO: 1375 - DNA, 23 bp, Homo sapiens
agggaggcagagagagagggagg

SEQ ID NO: 1376 - DNA, 23 bp, Homo sapiens
agagagggaggcagagagagagg

SEQ ID NO: 1377 - DNA, 23 bp, Homo sapiens
gaaagggaggcagagagagaggg

SEQ ID NO: 1378 - DNA, 23 bp, Homo sapiens
gagagagagaaagaggcagaagg

SEQ ID NO: 1379 - DNA, 23 bp, Homo sapiens
gagagagggaggcagagagaggg

SEQ ID NO: 1380 - DNA, 23 bp, Homo sapiens
ggggggagagagagagaaagagg

SEQ ID NO: 1381 - DNA, 23 bp, Homo sapiens
gagagggaggcagagagagaggg

SEQ ID NO: 1382 - DNA, 23 bp, Homo sapiens
agaggcagaaagagagagagagg

SEQ ID NO: 1383 - DNA, 23 bp, Homo sapiens
gagcttcgtgctgtaccgcgagg

SEQ ID NO: 1384 - DNA, 23 bp, Homo sapiens
cgggggaacctagtccgcctggg

SEQ ID NO: 1385 - DNA, 23 bp, Homo sapiens
ggggtctaaggaccgttccgcgg

SEQ ID NO: 1386 - DNA, 23 bp, Homo sapiens
gttcccccgggtgtagtcggagg

SEQ ID NO: 1387 - DNA, 23 bp, Homo sapiens
gggggaacctagtccgcctgggg

SEQ ID NO: 1388 - DNA, 23 bp, Homo sapiens
agcttcgtgctgtaccgcgaggg

SEQ ID NO: 1389 - DNA, 23 bp, Homo sapiens
cgtgctgtaccgcgagggcgtgg

SEQ ID NO: 1390 - DNA, 23 bp, Homo sapiens
ctgcgctgcgacagcacgtaggg

SEQ ID NO: 1391 - DNA, 23 bp, Homo sapiens
taggttcccccgggtgtagtcgg

SEQ ID NO: 1392 - DNA, 23 bp, Homo sapiens
aaaagtgaccagcgcgcccaggg

SEQ ID NO: 1393 - DNA, 23 bp, Homo sapiens
gcgcgctggtcacttttgactgg

SEQ ID NO: 1394 - DNA, 23 bp, Homo sapiens
gcacgaagctcatgttccgcagg

SEQ ID NO: 1395 - DNA, 23 bp, Homo sapiens
gacagcacgtagggcgcggaggg

SEQ ID NO: 1396 - DNA, 23 bp, Homo sapiens
tgaaaggaagacgcgattagtgg

SEQ ID NO: 1397 - DNA, 23 bp, Homo sapiens
tgggccgacttcacgctgctggg

SEQ ID NO: 1398 - DNA, 23 bp, Homo sapiens
agcagcgtgaagtcggcccaggg

SEQ ID NO: 1399 - DNA, 23 bp, Homo sapiens
gctcaggggcggataccagcagg

SEQ ID NO: 1400 - DNA, 23 bp, Homo sapiens
caaaagtgaccagcgcgcccagg

SEQ ID NO: 1401 - DNA, 23 bp, Homo sapiens
ggaataaaagctggcgagcgcgg

SEQ ID NO: 1402 - DNA, 23 bp, Homo sapiens
cgcgcagcgcaggctcacgttgg

SEQ ID NO: 1403 - DNA, 23 bp, Homo sapiens
agcgccaccagcgacggccgcgg

SEQ ID NO: 1404 - DNA, 23 bp, Homo sapiens
ctgcgacagcacgtagggcgcgg

SEQ ID NO: 1405 - DNA, 23 bp, Homo sapiens
ccgggggaacctagtccgcctgg

SEQ ID NO: 1406 - DNA, 23 bp, Homo sapiens
caatcagcaggacacgggcgggg

SEQ ID NO: 1407 - DNA, 23 bp, Homo sapiens
ccattttacagagcgctgattgg

SEQ ID NO: 1408 - DNA, 23 bp, Homo sapiens
aacgtgagcctgcgctgcgcggg

SEQ ID NO: 1409 - DNA, 23 bp, Homo sapiens
caacgtgagcctgcgctgcgcgg

SEQ ID NO: 1410 - DNA, 23 bp, Homo sapiens
gctgcgctgcgacagcacgtagg

SEQ ID NO: 1411 - DNA, 23 bp, Homo sapiens
cgacagcacgtagggcgcggagg

SEQ ID NO: 1412 - DNA, 23 bp, Homo sapiens
cgtgctgtcgcagcgcagcgagg

SEQ ID NO: 1413 - DNA, 23 bp, Homo sapiens
ctgggccgacttcacgctgctgg

SEQ ID NO: 1414 - DNA, 23 bp, Homo sapiens
cagcagcgtgaagtcggcccagg

SEQ ID NO: 1415 - DNA, 23 bp, Homo sapiens
gctcctccgactacacccggggg

SEQ ID NO: 1416 - DNA, 23 bp, Homo sapiens
gctggctgagctccgcggaacgg

SEQ ID NO: 1417 - DNA, 23 bp, Homo sapiens
gctgtaccgcgagggcgtggcgg

SEQ ID NO: 1418 - DNA, 23 bp, Homo sapiens
cgaagctcatgttccgcaggcgg

SEQ ID NO: 1419 - DNA, 23 bp, Homo sapiens
ggctcctccgactacacccgggg

SEQ ID NO: 1420 - DNA, 23 bp, Homo sapiens
agagtctgcttccacgttgtggg

SEQ ID NO: 1421 - DNA, 23 bp, Homo sapiens
ctggctcctccgactacacccgg

SEQ ID NO: 1422 - DNA, 23 bp, Homo sapiens
caaagttgagggggagtcgatgg

SEQ ID NO: 1423 - DNA, 23 bp, Homo sapiens
caggcggactaggttcccccggg

SEQ ID NO: 1424 - DNA, 23 bp, Homo sapiens
ggacacgggcggggacaataagg

SEQ ID NO: 1425 - DNA, 23 bp, Homo sapiens
cggagtggcggtactgcagcggg

SEQ ID NO: 1426 - DNA, 23 bp, Homo sapiens
ggagtggcggtactgcagcgggg

SEQ ID NO: 1427 - DNA, 23 bp, Homo sapiens
agtcagaaccgcgctcctgctgg

SEQ ID NO: 1428 - DNA, 23 bp, Homo sapiens
ccaggcggactaggttcccccgg

SEQ ID NO: 1429 - DNA, 23 bp, Homo sapiens
cctcatctccctgggcgcgctgg

SEQ ID NO: 1430 - DNA, 23 bp, Homo sapiens
gcggagtggcggtactgcagcgg

SEQ ID NO: 1431 - DNA, 23 bp, Homo sapiens
tggctcctccgactacacccggg

SEQ ID NO: 1432 - DNA, 23 bp, Homo sapiens
tcgatggaggcttcaactcctgg

SEQ ID NO: 1433 - DNA, 23 bp, Homo sapiens
gaacctagtccgcctggggctgg

SEQ ID NO: 1434 - DNA, 23 bp, Homo sapiens
ttggcgccaggacccaccaccgg

SEQ ID NO: 1435 - DNA, 23 bp, Homo sapiens
cgtgtgatagtagcagctgtagg

SEQ ID NO: 1436 - DNA, 23 bp, Homo sapiens
gtcgcagcgcagcgaggtgctgg

SEQ ID NO: 1437 - DNA, 23 bp, Homo sapiens
ccaatcagcaggacacgggcggg

SEQ ID NO: 1438 - DNA, 23 bp, Homo sapiens
agaacaaagctcccacaacgtgg

SEQ ID NO: 1439 - DNA, 23 bp, Homo sapiens
cagagtctgcttccacgttgtgg

SEQ ID NO: 1440 - DNA, 23 bp, Homo sapiens
ccaatcagcgctctgtaaaatgg

SEQ ID NO: 1441 - DNA, 23 bp, Homo sapiens
gacacgggcggggacaataaggg

SEQ ID NO: 1442 - DNA, 23 bp, Homo sapiens
ccgggcagcgccaccagcgacgg

SEQ ID NO: 1443 - DNA, 23 bp, Homo sapiens
gctgccgcggccgtcgctggtgg

SEQ ID NO: 1444 - DNA, 23 bp, Homo sapiens
cgatggaggcttcaactcctggg

SEQ ID NO: 1445 - DNA, 23 bp, Homo sapiens
agcttctccgccactcaggttgg

SEQ ID NO: 1446 - DNA, 23 bp, Homo sapiens
cccgagacttccaacctgagtgg

SEQ ID NO: 1447 - DNA, 23 bp, Homo sapiens
ggcgcccagcagcgtgaagtcgg

SEQ ID NO: 1448 - DNA, 23 bp, Homo sapiens
gactagactcctggatctgaggg

SEQ ID NO: 1449 - DNA, 23 bp, Homo sapiens
cggccagccccaggcggactagg

SEQ ID NO: 1450 - DNA, 23 bp, Homo sapiens
gattcgaaccctctgtcttctgg

SEQ ID NO: 1451 - DNA, 23 bp, Homo sapiens
cacaacgtggaagcagactctgg

SEQ ID NO: 1452 - DNA, 23 bp, Homo sapiens
gtagcagctgtaggtgccggggg

SEQ ID NO: 1453 - DNA, 23 bp, Homo sapiens
gcgaggtgctggtcatcagctgg

SEQ ID NO: 1454 - DNA, 23 bp, Homo sapiens
atagtagcagctgtaggtgccgg

SEQ ID NO: 1455 - DNA, 23 bp, Homo sapiens
gagctggaggactagactcctgg

SEQ ID NO: 1456 - DNA, 23 bp, Homo sapiens
ggctgcaggactagacccctggg

SEQ ID NO: 1457 - DNA, 23 bp, Homo sapiens
agttgagggggagtcgatggagg

SEQ ID NO: 1458 - DNA, 23 bp, Homo sapiens
acagggcacagcggggtctaagg

SEQ ID NO: 1459 - DNA, 23 bp, Homo sapiens
ctactactacagtgagtagacgg

SEQ ID NO: 1460 - DNA, 23 bp, Homo sapiens
accaatcagcaggacacgggcgg

SEQ ID NO: 1461 - DNA, 23 bp, Homo sapiens
gctcccggaccccaaagtctggg

SEQ ID NO: 1462 - DNA, 23 bp, Homo sapiens
ccactcaggttggaagtctcggg

SEQ ID NO: 1463 - DNA, 23 bp, Homo sapiens
gccactcaggttggaagtctcgg

SEQ ID NO: 1464 - DNA, 23 bp, Homo sapiens
acgtggaagcagactctggtggg

SEQ ID NO: 1465 - DNA, 23 bp, Homo sapiens
ggagctgccgcggccgtcgctgg

SEQ ID NO: 1466 - DNA, 23 bp, Homo sapiens
agtagcagctgtaggtgccgggg

SEQ ID NO: 1467 - DNA, 23 bp, Homo sapiens
agctcccggaccccaaagtctgg

SEQ ID NO: 1468 - DNA, 23 bp, Homo sapiens
cagtgagtagacggcagtgctgg

SEQ ID NO: 1469 - DNA, 23 bp, Homo sapiens
ccatcttacagagtgctgattgg

SEQ ID NO: 1470 - DNA, 23 bp, Homo sapiens
gcgctgcccgggccggtggtggg

SEQ ID NO: 1471 - DNA, 23 bp, Homo sapiens
ccaatcagcactctgtaagatgg

SEQ ID NO: 1472 - DNA, 23 bp, Homo sapiens
tagtagcagctgtaggtgccggg

SEQ ID NO: 1473 - DNA, 23 bp, Homo sapiens
cgaggtgctggtcatcagctggg

SEQ ID NO: 1474 - DNA, 23 bp, Homo sapiens
gggctgcaggactagacccctgg

SEQ ID NO: 1475 - DNA, 23 bp, Homo sapiens
ggtccctaagtccaccccagggg

SEQ ID NO: 1476 - DNA, 23 bp, Homo sapiens
gagacttccaacctgagtggcgg

SEQ ID NO: 1477 - DNA, 23 bp, Homo sapiens
ttcaacccaggaagtccagctgg

SEQ ID NO: 1478 - DNA, 23 bp, Homo sapiens
tagtgagacgtgaagccagctgg

SEQ ID NO: 1479 - DNA, 23 bp, Homo sapiens
agtgagtagacggcagtgctggg

SEQ ID NO: 1480 - DNA, 23 bp, Homo sapiens
tgtaaaatggaccaatcagcagg

SEQ ID NO: 1481 - DNA, 23 bp, Homo sapiens
tgcgctgcgcgggccgcctgcgg

SEQ ID NO: 1482 - DNA, 23 bp, Homo sapiens
gcaggcggcccgcgcagcgcagg

SEQ ID NO: 1483 - DNA, 23 bp, Homo sapiens
aactttgagactgtagagtcagg

SEQ ID NO: 1484 - DNA, 23 bp, Homo sapiens
cagcccctggggtggacttaggg

SEQ ID NO: 1485 - DNA, 23 bp, Homo sapiens
actctacagtctcaaagttgagg

SEQ ID NO: 1486 - DNA, 23 bp, Homo sapiens
ggcggataccagcaggagcgcgg

SEQ ID NO: 1487 - DNA, 23 bp, Homo sapiens
aacctgagtggcggagaagctgg

SEQ ID NO: 1488 - DNA, 23 bp, Homo sapiens
tggacttcctgggttgaatgggg

SEQ ID NO: 1489 - DNA, 23 bp, Homo sapiens
ggactagactcctggatctgagg

SEQ ID NO: 1490 - DNA, 23 bp, Homo sapiens
tccaggtccccattcaacccagg

SEQ ID NO: 1491 - DNA, 23 bp, Homo sapiens
gcggggccgccacgccctcgcgg

SEQ ID NO: 1492 - DNA, 23 bp, Homo sapiens
gccaggacccaccaccggcccgg

SEQ ID NO: 1493 - DNA, 23 bp, Homo sapiens
gactagacccctgggtctgaagg

SEQ ID NO: 1494 - DNA, 23 bp, Homo sapiens
gtactggggcccgggaatcctgg

SEQ ID NO: 1495 - DNA, 23 bp, Homo sapiens
ccggctccgcccgcagactctgg

SEQ ID NO: 1496 - DNA, 23 bp, Homo sapiens
ccagagtctgcgggcggagccgg

SEQ ID NO: 1497 - DNA, 23 bp, Homo sapiens
gtctcgggctgcagtgctcctgg

SEQ ID NO: 1498 - DNA, 23 bp, Homo sapiens
acctgagtggcggagaagctggg

SEQ ID NO: 1499 - DNA, 23 bp, Homo sapiens
ctacagtctcaaagttgaggggg

SEQ ID NO: 1500 - DNA, 23 bp, Homo sapiens
gagttcagggcccagactttggg

SEQ ID NO: 1501 - DNA, 23 bp, Homo sapiens
gctggacttcctgggttgaatgg

SEQ ID NO: 1502 - DNA, 23 bp, Homo sapiens
ctggacttcctgggttgaatggg

SEQ ID NO: 1503 - DNA, 23 bp, Homo sapiens
tggaccaatcagcaggacacggg

SEQ ID NO: 1504 - DNA, 23 bp, Homo sapiens
accgccactccgcgcagccctgg

SEQ ID NO: 1505 - DNA, 23 bp, Homo sapiens
tactggggcccgggaatcctggg

SEQ ID NO: 1506 - DNA, 23 bp, Homo sapiens
caggtccctaagtccaccccagg

SEQ ID NO: 1507 - DNA, 23 bp, Homo sapiens
ttccgcggagctcagccagcagg

SEQ ID NO: 1508 - DNA, 23 bp, Homo sapiens
cgtggaagcagactctggtgggg

SEQ ID NO: 1509 - DNA, 23 bp, Homo sapiens
aacgtggaagcagactctggtgg

SEQ ID NO: 1510 - DNA, 23 bp, Homo sapiens
cgtcgctggtggcgctgcccggg

SEQ ID NO: 1511 - DNA, 23 bp, Homo sapiens
ccgtcgctggtggcgctgcccgg

SEQ ID NO: 1512 - DNA, 23 bp, Homo sapiens
cctggactgctggatcaggaagg

SEQ ID NO: 1513 - DNA, 23 bp, Homo sapiens
cccgggccggtggtgggtcctgg

SEQ ID NO: 1514 - DNA, 23 bp, Homo sapiens
gctgtaggtgccgggggcgcggg

SEQ ID NO: 1515 - DNA, 23 bp, Homo sapiens
ggtctgagggcggaggtcctggg

SEQ ID NO: 1516 - DNA, 23 bp, Homo sapiens
aggtccctaagtccaccccaggg

SEQ ID NO: 1517 - DNA, 23 bp, Homo sapiens
cagagtctgcgggcggagccggg

SEQ ID NO: 1518 - DNA, 23 bp, Homo sapiens
tctcgggctgcagtgctcctggg

SEQ ID NO: 1519 - DNA, 23 bp, Homo sapiens
gaagtcggcccagggctgcgcgg

SEQ ID NO: 1520 - DNA, 23 bp, Homo sapiens
cccgggaatcctgggtctgaggg

SEQ ID NO: 1521 - DNA, 23 bp, Homo sapiens
tcggaggagccagagtctgcggg

SEQ ID NO: 1522 - DNA, 23 bp, Homo sapiens
tctacagtctcaaagttgagggg

SEQ ID NO: 1523 - DNA, 23 bp, Homo sapiens
ctctacagtctcaaagttgaggg

SEQ ID NO: 1524 - DNA, 23 bp, Homo sapiens
agttcagggcccagactttgggg

SEQ ID NO: 1525 - DNA, 23 bp, Homo sapiens
tgaagccagctggacttcctggg

SEQ ID NO: 1526 - DNA, 23 bp, Homo sapiens
ctggaaagaagctacagcacagg

SEQ ID NO: 1527 - DNA, 23 bp, Homo sapiens
tagactcctggatctgagggagg

SEQ ID NO: 1528 - DNA, 23 bp, Homo sapiens
aagtctgggccctgaactccagg

SEQ ID NO: 1529 - DNA, 23 bp, Homo sapiens
atggaccaatcagcaggacacgg

SEQ ID NO: 1530 - DNA, 23 bp, Homo sapiens
ccgccactccgcgcagccctggg

SEQ ID NO: 1531 - DNA, 23 bp, Homo sapiens
agctgtaggtgccgggggcgcgg

SEQ ID NO: 1532 - DNA, 23 bp, Homo sapiens
ccttcctgatccagcagtccagg

SEQ ID NO: 1533 - DNA, 23 bp, Homo sapiens
ctgcattcctggggcggaggagg

SEQ ID NO: 1534 - DNA, 23 bp, Homo sapiens
tagacccctgggtctgaaggagg

SEQ ID NO: 1535 - DNA, 23 bp, Homo sapiens
tcccagcttctccgccactcagg

SEQ ID NO: 1536 - DNA, 23 bp, Homo sapiens
tttcccaaggagtagctgaaagg

SEQ ID NO: 1537 - DNA, 23 bp, Homo sapiens
gaaccctctgtcttctggcttgg

SEQ ID NO: 1538 - DNA, 23 bp, Homo sapiens
cttacaagaggattgtaaaatgg

SEQ ID NO: 1539 - DNA, 23 bp, Homo sapiens
gcagctcctctgcagagacgggg

SEQ ID NO: 1540 - DNA, 23 bp, Homo sapiens
ctcctccgccccaggaatgcagg

SEQ ID NO: 1541 - DNA, 23 bp, Homo sapiens
ggtatccgcccctgagccccagg

SEQ ID NO: 1542 - DNA, 23 bp, Homo sapiens
tagtagtagcagctacagaaagg

SEQ ID NO: 1543 - DNA, 23 bp, Homo sapiens
tttcagctactccttgggaaagg

SEQ ID NO: 1544 - DNA, 23 bp, Homo sapiens
ggtggcgctgcccgggccggtgg

SEQ ID NO: 1545 - DNA, 23 bp, Homo sapiens
ccaggacccaccaccggcccggg

SEQ ID NO: 1546 - DNA, 23 bp, Homo sapiens
cccaggaatcctgggtctgaggg

SEQ ID NO: 1547 - DNA, 23 bp, Homo sapiens
ggggcctggactgctggatcagg

SEQ ID NO: 1548 - DNA, 23 bp, Homo sapiens
ccagcccctggggtggacttagg

SEQ ID NO: 1549 - DNA, 23 bp, Homo sapiens
tagtccgcctggggctggccggg

SEQ ID NO: 1550 - DNA, 23 bp, Homo sapiens
cgggctggtcctcatctccctgg

SEQ ID NO: 1551 - DNA, 23 bp, Homo sapiens
ctagtccgcctggggctggccgg

SEQ ID NO: 1552 - DNA, 23 bp, Homo sapiens
cttcctttcagctactccttggg

SEQ ID NO: 1553 - DNA, 23 bp, Homo sapiens
gtaagacagaaaagttctccagg

SEQ ID NO: 1554 - DNA, 23 bp, Homo sapiens
cggcccagggctgcgcggagtgg

SEQ ID NO: 1555 - DNA, 23 bp, Homo sapiens
ctgctgggcgcccgcgcccccgg

SEQ ID NO: 1556 - DNA, 23 bp, Homo sapiens
ggcctgcattcctggggcggagg

SEQ ID NO: 1557 - DNA, 23 bp, Homo sapiens
ctcgggctgcagtgctcctgggg

SEQ ID NO: 1558 - DNA, 23 bp, Homo sapiens
agctcagccagcaggactgtggg

SEQ ID NO: 1559 - DNA, 23 bp, Homo sapiens
gaacttttctgtcttacaagagg

SEQ ID NO: 1560 - DNA, 23 bp, Homo sapiens
ggcgctgcccgggccggtggtgg

SEQ ID NO: 1561 - DNA, 23 bp, Homo sapiens
gtctgagggcggaggtcctgggg

SEQ ID NO: 1562 - DNA, 23 bp, Homo sapiens
gggtctgagggcggaggtcctgg

SEQ ID NO: 1563 - DNA, 23 bp, Homo sapiens
cccagggctgcgcggagtggcgg

SEQ ID NO: 1564 - DNA, 23 bp, Homo sapiens
aggaggcgggccgggcctcaggg

SEQ ID NO: 1565 - DNA, 23 bp, Homo sapiens
cctaagtccaccccaggggctgg

SEQ ID NO: 1566 - DNA, 23 bp, Homo sapiens
gctactccttgggaaaggcctgg

SEQ ID NO: 1567 - DNA, 23 bp, Homo sapiens
tctctgcagaggagctgccgcgg

SEQ ID NO: 1568 - DNA, 23 bp, Homo sapiens
gtgctggtcatcagctgggaagg

SEQ ID NO: 1569 - DNA, 23 bp, Homo sapiens
ggctggaaacctggagttcaggg

SEQ ID NO: 1570 - DNA, 23 bp, Homo sapiens
agggcccagactttggggtccgg

SEQ ID NO: 1571 - DNA, 23 bp, Homo sapiens
agctgatggcccctctctcccgg

SEQ ID NO: 1572 - DNA, 23 bp, Homo sapiens
ccagcgcgcccagggagatgagg

SEQ ID NO: 1573 - DNA, 23 bp, Homo sapiens
ctacagcacagggcacagcgggg

SEQ ID NO: 1574 - DNA, 23 bp, Homo sapiens
ggagttcagggcccagactttgg

SEQ ID NO: 1575 - DNA, 23 bp, Homo sapiens
agagaggggccatcagctcccgg

SEQ ID NO: 1576 - DNA, 23 bp, Homo sapiens
gctggtggcgctgcccgggccgg

SEQ ID NO: 1577 - DNA, 23 bp, Homo sapiens
ggctgggtcccaggaatcctggg

SEQ ID NO: 1578 - DNA, 23 bp, Homo sapiens
gaggagccagagtctgcgggcgg

SEQ ID NO: 1579 - DNA, 23 bp, Homo sapiens
gcgggcggagccgggagagaggg

SEQ ID NO: 1580 - DNA, 23 bp, Homo sapiens
ggtcctggggcctgcattcctgg

SEQ ID NO: 1581 - DNA, 23 bp, Homo sapiens
ggtcatcagctgggaaggtgagg

SEQ ID NO: 1582 - DNA, 23 bp, Homo sapiens
gcctggagtcctgggtctgaggg

SEQ ID NO: 1583 - DNA, 23 bp, Homo sapiens
ggtctgagggaggaggtactggg

SEQ ID NO: 1584 - DNA, 23 bp, Homo sapiens
gtcggaggagccagagtctgcgg

SEQ ID NO: 1585 - DNA, 23 bp, Homo sapiens
ctgtgctgtagcttctttccagg

SEQ ID NO: 1586 - DNA, 23 bp, Homo sapiens
tcctgggttgaatggggacctgg

SEQ ID NO: 1587 - DNA, 23 bp, Homo sapiens
gacaataagggaataaaagctgg

SEQ ID NO: 1588 - DNA, 23 bp, Homo sapiens
ctctcaccccgtctctgcagagg

SEQ ID NO: 1589 - DNA, 23 bp, Homo sapiens
gggcccagactttggggtccggg

SEQ ID NO: 1590 - DNA, 23 bp, Homo sapiens
tggaaagaagctacagcacaggg

SEQ ID NO: 1591 - DNA, 23 bp, Homo sapiens
gtcctggggcctgcattcctggg

SEQ ID NO: 1592 - DNA, 23 bp, Homo sapiens
ccctcagacccaggattcccggg

SEQ ID NO: 1593 - DNA, 23 bp, Homo sapiens
gctcagccagcaggactgtgggg

SEQ ID NO: 1594 - DNA, 23 bp, Homo sapiens
ggacctccgccctcagacccagg

SEQ ID NO: 1595 - DNA, 23 bp, Homo sapiens
aggaatcctgggtctgagggagg

SEQ ID NO: 1596 - DNA, 23 bp, Homo sapiens
cctctcctccttcagacccaggg

SEQ ID NO: 1597 - DNA, 23 bp, Homo sapiens
tcccaggaatcctgggtctgagg

SEQ ID NO: 1598 - DNA, 23 bp, Homo sapiens
aactccaggtttccagcccctgg

SEQ ID NO: 1599 - DNA, 23 bp, Homo sapiens
tgcagtgctcctggggctcaggg

SEQ ID NO: 1600 - DNA, 23 bp, Homo sapiens
aggaaaggacagtccagcccagg

SEQ ID NO: 1601 - DNA, 23 bp, Homo sapiens
cccgcccgtgtcctgctgattgg

SEQ ID NO: 1602 - DNA, 23 bp, Homo sapiens
gctcctgggtctgagggcggagg

SEQ ID NO: 1603 - DNA, 23 bp, Homo sapiens
cttcctggacccaggactccagg

SEQ ID NO: 1604 - DNA, 23 bp, Homo sapiens
gtctgagggaggaggtactgggg

SEQ ID NO: 1605 - DNA, 23 bp, Homo sapiens
caccccaggggctggaaacctgg

SEQ ID NO: 1606 - DNA, 23 bp, Homo sapiens
ggactgctggatcaggaaggagg

SEQ ID NO: 1607 - DNA, 23 bp, Homo sapiens
ctttggggtccgggagctgatgg

SEQ ID NO: 1608 - DNA, 23 bp, Homo sapiens
ctgcagccccacagtcctgctgg

SEQ ID NO: 1609 - DNA, 23 bp, Homo sapiens
ggcggagaagctgggaccctggg

SEQ ID NO: 1610 - DNA, 23 bp, Homo sapiens
ggcagctcctctgcagagacggg

SEQ ID NO: 1611 - DNA, 23 bp, Homo sapiens
gcccgggaatcctgggtctgagg

SEQ ID NO: 1612 - DNA, 23 bp, Homo sapiens
gactgctggatcaggaaggaggg

SEQ ID NO: 1613 - DNA, 23 bp, Homo sapiens
actcctgggtccaggaagaaggg

SEQ ID NO: 1614 - DNA, 23 bp, Homo sapiens
acttccaagccagaagacagagg

SEQ ID NO: 1615 - DNA, 23 bp, Homo sapiens
attcctggggcggaggaggcggg

SEQ ID NO: 1616 - DNA, 23 bp, Homo sapiens
gccccaggaatgcaggccccagg

SEQ ID NO: 1617 - DNA, 23 bp, Homo sapiens
tccctcagacccaggattcccgg

SEQ ID NO: 1618 - DNA, 23 bp, Homo sapiens
tccctcagacccaggattcctgg

SEQ ID NO: 1619 - DNA, 23 bp, Homo sapiens
gggctgggtcccaggaatcctgg

SEQ ID NO: 1620 - DNA, 23 bp, Homo sapiens
gcctctcctccttcagacccagg

SEQ ID NO: 1621 - DNA, 23 bp, Homo sapiens
gggtctgagggaggaggtactgg

SEQ ID NO: 1622 - DNA, 23 bp, Homo sapiens
gagctcagccagcaggactgtgg

SEQ ID NO: 1623 - DNA, 23 bp, Homo sapiens
gcctgggctcctgggtctgaggg

SEQ ID NO: 1624 - DNA, 23 bp, Homo sapiens
gaggaggcgggccgggcctcagg

SEQ ID NO: 1625 - DNA, 23 bp, Homo sapiens
ccctcagacccaggattcctggg

SEQ ID NO: 1626 - DNA, 23 bp, Homo sapiens
ctggagtcctgggtccaggaagg

SEQ ID NO: 1627 - DNA, 23 bp, Homo sapiens
ctctcctccttcagacccagggg

SEQ ID NO: 1628 - DNA, 23 bp, Homo sapiens
gggaatcctgggtctgagggagg

SEQ ID NO: 1629 - DNA, 23 bp, Homo sapiens
caggtttccagcccctggggtgg

SEQ ID NO: 1630 - DNA, 23 bp, Homo sapiens
cagggagatgaggaccagcccgg

SEQ ID NO: 1631 - DNA, 23 bp, Homo sapiens
agctacagcacagggcacagcgg

SEQ ID NO: 1632 - DNA, 23 bp, Homo sapiens
cttccaagccagaagacagaggg

SEQ ID NO: 1633 - DNA, 23 bp, Homo sapiens
cggcccgcctcctccgccccagg

SEQ ID NO: 1634 - DNA, 23 bp, Homo sapiens
tggagtcctgggtctgagggagg

SEQ ID NO: 1635 - DNA, 23 bp, Homo sapiens
gggctggaaacctggagttcagg

SEQ ID NO: 1636 - DNA, 23 bp, Homo sapiens
tgcgggcggagccgggagagagg

SEQ ID NO: 1637 - DNA, 23 bp, Homo sapiens
ctccaggtttccagcccctgggg

SEQ ID NO: 1638 - DNA, 23 bp, Homo sapiens
tggcggagaagctgggaccctgg

SEQ ID NO: 1639 - DNA, 23 bp, Homo sapiens
ccgcctggggctggccgggctgg

SEQ ID NO: 1640 - DNA, 23 bp, Homo sapiens
aactcctgggtccaggaagaagg

SEQ ID NO: 1641 - DNA, 23 bp, Homo sapiens
cgggcggagccgggagagagggg

SEQ ID NO: 1642 - DNA, 23 bp, Homo sapiens
gcagtgctcctggggctcagggg

SEQ ID NO: 1643 - DNA, 23 bp, Homo sapiens
gctacagcacagggcacagcggg

SEQ ID NO: 1644 - DNA, 23 bp, Homo sapiens
tggggcggaggaggcgggccggg

SEQ ID NO: 1645 - DNA, 23 bp, Homo sapiens
actcctggatctgagggaggagg

SEQ ID NO: 1646 - DNA, 23 bp, Homo sapiens
tccctcagacccaggactccagg

SEQ ID NO: 1647 - DNA, 23 bp, Homo sapiens
agccccttcttcctggacccagg

SEQ ID NO: 1648 - DNA, 23 bp, Homo sapiens
ctgcagtgctcctggggctcagg

SEQ ID NO: 1649 - DNA, 23 bp, Homo sapiens
gtcctgctggctgagctccgcgg

SEQ ID NO: 1650 - DNA, 23 bp, Homo sapiens
cggcagctcctctgcagagacgg

SEQ ID NO: 1651 - DNA, 23 bp, Homo sapiens
gcccctcctccctcagatccagg

SEQ ID NO: 1652 - DNA, 23 bp, Homo sapiens
actgctggatcaggaaggagggg

SEQ ID NO: 1653 - DNA, 23 bp, Homo sapiens
aggcttcaactcctgggtccagg

SEQ ID NO: 1654 - DNA, 23 bp, Homo sapiens
tcctggggcctgcattcctgggg

SEQ ID NO: 1655 - DNA, 23 bp, Homo sapiens
tgggctcctgggtctgagggcgg

SEQ ID NO: 1656 - DNA, 23 bp, Homo sapiens
gtacctcctccctcagacccagg

SEQ ID NO: 1657 - DNA, 23 bp, Homo sapiens
gggctggtcctcatctccctggg

SEQ ID NO: 1658 - DNA, 23 bp, Homo sapiens
cattcctggggcggaggaggcgg

SEQ ID NO: 1659 - DNA, 23 bp, Homo sapiens
ctcctggatctgagggaggaggg

SEQ ID NO: 1660 - DNA, 23 bp, Homo sapiens
tgggtccaggaagaaggggctgg

SEQ ID NO: 1661 - DNA, 23 bp, Homo sapiens
ctggatcaggaaggaggggctgg

SEQ ID NO: 1662 - DNA, 23 bp, Homo sapiens
ctcctgggtccaggaagaagggg

SEQ ID NO: 1663 - DNA, 23 bp, Homo sapiens
ggaccagcccggccagccccagg

SEQ ID NO: 1664 - DNA, 23 bp, Homo sapiens
ttctttccaggcctttcccaagg

SEQ ID NO: 1665 - DNA, 23 bp, Homo sapiens
cgcaggctcacgttggcgccagg

SEQ ID NO: 1666 - DNA, 23 bp, Homo sapiens
gtcatcagctgggaaggtgaggg

SEQ ID NO: 1667 - DNA, 23 bp, Homo sapiens
ctggggcggaggaggcgggccgg

SEQ ID NO: 1668 - DNA, 23 bp, Homo sapiens
agggaggaggtactggggcccgg

SEQ ID NO: 1669 - DNA, 23 bp, Homo sapiens
actccaggtttccagcccctggg

SEQ ID NO: 1670 - DNA, 23 bp, Homo sapiens
cagcaggactgtggggctgcagg

SEQ ID NO: 1671 - DNA, 23 bp, Homo sapiens
ggactgtggggctgcaggaaagg

SEQ ID NO: 1672 - DNA, 23 bp, Homo sapiens
gccctcagacccaggagcccagg

SEQ ID NO: 1673 - DNA, 23 bp, Homo sapiens
gggaggaggtactggggcccggg

SEQ ID NO: 1674 - DNA, 23 bp, Homo sapiens
agtcctgggtccaggaaggaggg

SEQ ID NO: 1675 - DNA, 23 bp, Homo sapiens
ccctgggtctgaaggaggagagg

SEQ ID NO: 1676 - DNA, 23 bp, Homo sapiens
tggatcaggaaggaggggctggg

SEQ ID NO: 1677 - DNA, 23 bp, Homo sapiens
ggaaaggacagtccagcccaggg

SEQ ID NO: 1678 - DNA, 23 bp, Homo sapiens
aaggtgagggccctgaggcccgg

SEQ ID NO: 1679 - DNA, 23 bp, Homo sapiens
agcccctccttcctggacccagg

SEQ ID NO: 1680 - DNA, 23 bp, Homo sapiens
atcctgggtctgagggaggaggg

SEQ ID NO: 1681 - DNA, 23 bp, Homo sapiens
aatcctgggtctgagggaggagg

SEQ ID NO: 1682 - DNA, 23 bp, Homo sapiens
gtcctgggtccaggaaggagggg

SEQ ID NO: 1683 - DNA, 23 bp, Homo sapiens
ggtctgaaggaggagaggctggg

SEQ ID NO: 1684 - DNA, 23 bp, Homo sapiens
gggtccaggaagaaggggctggg

SEQ ID NO: 1685 - DNA, 23 bp, Homo sapiens
aggccccagccccttcttcctgg

SEQ ID NO: 1686 - DNA, 23 bp, Homo sapiens
tcttcctttcagctactccttgg

SEQ ID NO: 1687 - DNA, 23 bp, Homo sapiens
ggctgggggcctggagtcctggg

SEQ ID NO: 1688 - DNA, 23 bp, Homo sapiens
ggcctggagtcctgggtctgagg

SEQ ID NO: 1689 - DNA, 23 bp, Homo sapiens
agtcctgggtctgagggaggagg

SEQ ID NO: 1690 - DNA, 23 bp, Homo sapiens
gtgaagccagctggacttcctgg

SEQ ID NO: 1691 - DNA, 23 bp, Homo sapiens
ggcctgggctcctgggtctgagg

SEQ ID NO: 1692 - DNA, 23 bp, Homo sapiens
tggggcctgcattcctggggcgg

SEQ ID NO: 1693 - DNA, 23 bp, Homo sapiens
gggctgggggcctggagtcctgg

SEQ ID NO: 1694 - DNA, 23 bp, Homo sapiens
tgggtccaggaaggaggggctgg

SEQ ID NO: 1695 - DNA, 23 bp, Homo sapiens
ggtccaggaagaaggggctgggg

SEQ ID NO: 1696 - DNA, 23 bp, Homo sapiens
tctgaaggaggagaggctggggg

SEQ ID NO: 1697 - DNA, 23 bp, Homo sapiens
gatctgagggaggaggggctggg

SEQ ID NO: 1698 - DNA, 23 bp, Homo sapiens
ggggctggggcctggactgctgg

SEQ ID NO: 1699 - DNA, 23 bp, Homo sapiens
gtgctcctggggctcaggggcgg

SEQ ID NO: 1700 - DNA, 23 bp, Homo sapiens
ggctgggggcctgggctcctggg

SEQ ID NO: 1701 - DNA, 23 bp, Homo sapiens
gagtcctgggtccaggaaggagg

SEQ ID NO: 1702 - DNA, 23 bp, Homo sapiens
gggcctggagtcctgggtccagg

SEQ ID NO: 1703 - DNA, 23 bp, Homo sapiens
gtctgaaggaggagaggctgggg

SEQ ID NO: 1704 - DNA, 23 bp, Homo sapiens
gggtctgaaggaggagaggctgg

SEQ ID NO: 1705 - DNA, 23 bp, Homo sapiens
tcctggatctgagggaggagggg

SEQ ID NO: 1706 - DNA, 23 bp, Homo sapiens
gggaggaggggctgggtcccagg

SEQ ID NO: 1707 - DNA, 23 bp, Homo sapiens
gggtccaggaaggaggggctggg

SEQ ID NO: 1708 - DNA, 23 bp, Homo sapiens
tctgagggaggaggggctgcagg

SEQ ID NO: 1709 - DNA, 23 bp, Homo sapiens
ggaggagaggctgggggcctggg

SEQ ID NO: 1710 - DNA, 23 bp, Homo sapiens
gatcaggaaggaggggctggggg

SEQ ID NO: 1711 - DNA, 23 bp, Homo sapiens
ctgggaaggtgagggccctgagg

SEQ ID NO: 1712 - DNA, 23 bp, Homo sapiens
aggaggagaggctgggggcctgg

SEQ ID NO: 1713 - DNA, 23 bp, Homo sapiens
aggctgggggcctgggctcctgg

SEQ ID NO: 1714 - DNA, 23 bp, Homo sapiens
ggtccaggaaggaggggctgggg

SEQ ID NO: 1715 - DNA, 23 bp, Homo sapiens
gagaagctgggaccctgggctgg

SEQ ID NO: 1716 - DNA, 23 bp, Homo sapiens
ccagcccggccagccccaggcgg

SEQ ID NO: 1717 - DNA, 23 bp, Homo sapiens
gctcctcctccctcagacccagg

SEQ ID NO: 1718 - DNA, 23 bp, Homo sapiens
ggcccccagcccctccttcctgg

SEQ ID NO: 1719 - DNA, 23 bp, Homo sapiens
gtccaggaaggaggggctggggg

SEQ ID NO: 1720 - DNA, 23 bp, Homo sapiens
gcccctcctccctcagacccagg

SEQ ID NO: 1721 - DNA, 23 bp, Homo sapiens
ggaaggaggggctgggggcctgg

SEQ ID NO: 1722 - DNA, 23 bp, Homo sapiens
tctgagggaggaggagctggagg

SEQ ID NO: 1723 - DNA, 23 bp, Homo sapiens
ggatcaggaaggaggggctgggg

SEQ ID NO: 1724 - DNA, 23 bp, Homo sapiens
tcctgggtctgagggaggagggg

SEQ ID NO: 1725 - DNA, 23 bp, Homo sapiens
gggtctgagggaggaggagctgg

SEQ ID NO: 1726 - DNA, 23 bp, Homo sapiens
ggatctgagggaggaggggctgg

SEQ ID NO: 1727 - DNA, 23 bp, Homo sapiens
aggaagaaggggctggggcctgg

SEQ ID NO: 1728 - DNA, 23 bp, Homo sapiens
cgggggaacctagtccgcctggg

SEQ ID NO: 1729 - DNA, 23 bp, Homo sapiens
ggggtctaaggaccgttccgcgg

SEQ ID NO: 1730 - DNA, 23 bp, Homo sapiens
gttcccccgggtgtagtcggagg

SEQ ID NO: 1731 - DNA, 23 bp, Homo sapiens
gggggaacctagtccgcctgggg

SEQ ID NO: 1732 - DNA, 23 bp, Homo sapiens
taggttcccccgggtgtagtcgg

SEQ ID NO: 1733 - DNA, 23 bp, Homo sapiens
aaaagtgaccagcgcgcccaggg

SEQ ID NO: 1734 - DNA, 23 bp, Homo sapiens
gcgcgctggtcacttttgactgg

SEQ ID NO: 1735 - DNA, 23 bp, Homo sapiens
tgaaaggaagacgcgattagtgg

SEQ ID NO: 1736 - DNA, 23 bp, Homo sapiens
gctcaggggcggataccagcagg

SEQ ID NO: 1737 - DNA, 23 bp, Homo sapiens
caaaagtgaccagcgcgcccagg

SEQ ID NO: 1738 - DNA, 23 bp, Homo sapiens
ggaataaaagctggcgagcgcgg

SEQ ID NO: 1739 - DNA, 23 bp, Homo sapiens
ccgggggaacctagtccgcctgg

SEQ ID NO: 1740 - DNA, 23 bp, Homo sapiens
caatcagcaggacacgggcgggg

SEQ ID NO: 1741 - DNA, 23 bp, Homo sapiens
ccattttacagagcgctgattgg

SEQ ID NO: 1742 - DNA, 23 bp, Homo sapiens
gctcctccgactacacccggggg

SEQ ID NO: 1743 - DNA, 23 bp, Homo sapiens
gctggctgagctccgcggaacgg

SEQ ID NO: 1744 - DNA, 23 bp, Homo sapiens
ggctcctccgactacacccgggg

SEQ ID NO: 1745 - DNA, 23 bp, Homo sapiens
agagtctgcttccacgttgtggg

SEQ ID NO: 1746 - DNA, 23 bp, Homo sapiens
caggcggactaggttcccccggg

SEQ ID NO: 1747 - DNA, 23 bp, Homo sapiens
ctggctcctccgactacacccgg

SEQ ID NO: 1748 - DNA, 23 bp, Homo sapiens
ggacacgggcggggacaataagg

SEQ ID NO: 1749 - DNA, 23 bp, Homo sapiens
agtcagaaccgcgctcctgctgg

SEQ ID NO: 1750 - DNA, 23 bp, Homo sapiens
ccaggcggactaggttcccccgg

SEQ ID NO: 1751 - DNA, 23 bp, Homo sapiens
cctcatctccctgggcgcgctgg

SEQ ID NO: 1752 - DNA, 23 bp, Homo sapiens
tggctcctccgactacacccggg

SEQ ID NO: 1753 - DNA, 23 bp, Homo sapiens
gaacctagtccgcctggggctgg

SEQ ID NO: 1754 - DNA, 23 bp, Homo sapiens
ccaatcagcaggacacgggcggg

SEQ ID NO: 1755 - DNA, 23 bp, Homo sapiens
agaacaaagctcccacaacgtgg

SEQ ID NO: 1756 - DNA, 23 bp, Homo sapiens
cagagtctgcttccacgttgtgg

SEQ ID NO: 1757 - DNA, 23 bp, Homo sapiens
ccaatcagcgctctgtaaaatgg

SEQ ID NO: 1758 - DNA, 23 bp, Homo sapiens
gacacgggcggggacaataaggg

SEQ ID NO: 1759 - DNA, 23 bp, Homo sapiens
agcttctccgccactcaggttgg

SEQ ID NO: 1760 - DNA, 23 bp, Homo sapiens
cccgagacttccaacctgagtgg

SEQ ID NO: 1761 - DNA, 23 bp, Homo sapiens
cggccagccccaggcggactagg

SEQ ID NO: 1762 - DNA, 23 bp, Homo sapiens
gattcgaaccctctgtcttctgg

SEQ ID NO: 1763 - DNA, 23 bp, Homo sapiens
cacaacgtggaagcagactctgg

SEQ ID NO: 1764 - DNA, 23 bp, Homo sapiens
acagggcacagcggggtctaagg

SEQ ID NO: 1765 - DNA, 23 bp, Homo sapiens
ctactactacagtgagtagacgg

SEQ ID NO: 1766 - DNA, 23 bp, Homo sapiens
accaatcagcaggacacgggcgg

SEQ ID NO: 1767 - DNA, 23 bp, Homo sapiens
ccactcaggttggaagtctcggg

SEQ ID NO: 1768 - DNA, 23 bp, Homo sapiens
gccactcaggttggaagtctcgg

SEQ ID NO: 1769 - DNA, 23 bp, Homo sapiens
acgtggaagcagactctggtggg

SEQ ID NO: 1770 - DNA, 23 bp, Homo sapiens
cagtgagtagacggcagtgctgg

SEQ ID NO: 1771 - DNA, 23 bp, Homo sapiens
ccatcttacagagtgctgattgg

SEQ ID NO: 1772 - DNA, 23 bp, Homo sapiens
ccaatcagcactctgtaagatgg

SEQ ID NO: 1773 - DNA, 23 bp, Homo sapiens
gagacttccaacctgagtggcgg

SEQ ID NO: 1774 - DNA, 23 bp, Homo sapiens
tagtgagacgtgaagccagctgg

SEQ ID NO: 1775 - DNA, 23 bp, Homo sapiens
agtgagtagacggcagtgctggg

SEQ ID NO: 1776 - DNA, 23 bp, Homo sapiens
tgtaaaatggaccaatcagcagg

SEQ ID NO: 1777 - DNA, 23 bp, Homo sapiens
ggcggataccagcaggagcgcgg

SEQ ID NO: 1778 - DNA, 23 bp, Homo sapiens
aacctgagtggcggagaagctgg

SEQ ID NO: 1779 - DNA, 23 bp, Homo sapiens
tggacttcctgggttgaatgggg

SEQ ID NO: 1780 - DNA, 23 bp, Homo sapiens
tccaggtccccattcaacccagg

SEQ ID NO: 1781 - DNA, 23 bp, Homo sapiens
ccggctccgcccgcagactctgg

SEQ ID NO: 1782 - DNA, 23 bp, Homo sapiens
ccagagtctgcgggcggagccgg

SEQ ID NO: 1783 - DNA, 23 bp, Homo sapiens
gtctcgggctgcagtgctcctgg

SEQ ID NO: 1784 - DNA, 23 bp, Homo sapiens
acctgagtggcggagaagctggg

SEQ ID NO: 1785 - DNA, 23 bp, Homo sapiens
gctggacttcctgggttgaatgg

SEQ ID NO: 1786 - DNA, 23 bp, Homo sapiens
tggaccaatcagcaggacacggg

SEQ ID NO: 1787 - DNA, 23 bp, Homo sapiens
ctggacttcctgggttgaatggg

SEQ ID NO: 1788 - DNA, 23 bp, Homo sapiens
ttccgcggagctcagccagcagg

SEQ ID NO: 1789 - DNA, 23 bp, Homo sapiens
cgtggaagcagactctggtgggg

SEQ ID NO: 1790 - DNA, 23 bp, Homo sapiens
aacgtggaagcagactctggtgg

SEQ ID NO: 1791 - DNA, 23 bp, Homo sapiens
cagagtctgcgggcggagccggg

SEQ ID NO: 1792 - DNA, 23 bp, Homo sapiens
tctcgggctgcagtgctcctggg

SEQ ID NO: 1793 - DNA, 23 bp, Homo sapiens
tcggaggagccagagtctgcggg

SEQ ID NO: 1794 - DNA, 23 bp, Homo sapiens
tgaagccagctggacttcctggg

SEQ ID NO: 1795 - DNA, 23 bp, Homo sapiens
ctggaaagaagctacagcacagg

SEQ ID NO: 1796 - DNA, 23 bp, Homo sapiens
atggaccaatcagcaggacacgg

SEQ ID NO: 1797 - DNA, 23 bp, Homo sapiens
tcccagcttctccgccactcagg

SEQ ID NO: 1798 - DNA, 23 bp, Homo sapiens
tttcccaaggagtagctgaaagg

SEQ ID NO: 1799 - DNA, 23 bp, Homo sapiens
gaaccctctgtcttctggcttgg

SEQ ID NO: 1800 - DNA, 23 bp, Homo sapiens
cttacaagaggattgtaaaatgg

SEQ ID NO: 1801 - DNA, 23 bp, Homo sapiens
ggtatccgcccctgagccccagg

SEQ ID NO: 1802 - DNA, 23 bp, Homo sapiens
tagtagtagcagctacagaaagg

SEQ ID NO: 1803 - DNA, 23 bp, Homo sapiens
tttcagctactccttgggaaagg

SEQ ID NO: 1804 - DNA, 23 bp, Homo sapiens
tagtccgcctggggctggccggg

SEQ ID NO: 1805 - DNA, 23 bp, Homo sapiens
cgggctggtcctcatctccctgg

SEQ ID NO: 1806 - DNA, 23 bp, Homo sapiens
ctagtccgcctggggctggccgg

SEQ ID NO: 1807 - DNA, 23 bp, Homo sapiens
cttcctttcagctactccttggg

SEQ ID NO: 1808 - DNA, 23 bp, Homo sapiens
gtaagacagaaaagttctccagg

SEQ ID NO: 1809 - DNA, 23 bp, Homo sapiens
ctcgggctgcagtgctcctgggg

SEQ ID NO: 1810 - DNA, 23 bp, Homo sapiens
agctcagccagcaggactgtggg

SEQ ID NO: 1811 - DNA, 23 bp, Homo sapiens
gaacttttctgtcttacaagagg

SEQ ID NO: 1812 - DNA, 23 bp, Homo sapiens
gctactccttgggaaaggcctgg

SEQ ID NO: 1813 - DNA, 23 bp, Homo sapiens
ccagcgcgcccagggagatgagg

SEQ ID NO: 1814 - DNA, 23 bp, Homo sapiens
ctacagcacagggcacagcgggg

SEQ ID NO: 1815 - DNA, 23 bp, Homo sapiens
gaggagccagagtctgcgggcgg

SEQ ID NO: 1816 - DNA, 23 bp, Homo sapiens
gtcggaggagccagagtctgcgg

SEQ ID NO: 1817 - DNA, 23 bp, Homo sapiens
ctgtgctgtagcttctttccagg

SEQ ID NO: 1818 - DNA, 23 bp, Homo sapiens
gacaataagggaataaaagctgg

SEQ ID NO: 1819 - DNA, 23 bp, Homo sapiens
tcctgggttgaatggggacctgg

SEQ ID NO: 1820 - DNA, 23 bp, Homo sapiens
tggaaagaagctacagcacaggg

SEQ ID NO: 1821 - DNA, 23 bp, Homo sapiens
gctcagccagcaggactgtgggg

SEQ ID NO: 1822 - DNA, 23 bp, Homo sapiens
tgcagtgctcctggggctcaggg

SEQ ID NO: 1823 - DNA, 23 bp, Homo sapiens
aggaaaggacagtccagcccagg

SEQ ID NO: 1824 - DNA, 23 bp, Homo sapiens
cccgcccgtgtcctgctgattgg

SEQ ID NO: 1825 - DNA, 23 bp, Homo sapiens
ggcggagaagctgggaccctggg

SEQ ID NO: 1826 - DNA, 23 bp, Homo sapiens
ctgcagccccacagtcctgctgg

SEQ ID NO: 1827 - DNA, 23 bp, Homo sapiens
acttccaagccagaagacagagg

SEQ ID NO: 1828 - DNA, 23 bp, Homo sapiens
gagctcagccagcaggactgtgg

SEQ ID NO: 1829 - DNA, 23 bp, Homo sapiens
cagggagatgaggaccagcccgg

SEQ ID NO: 1830 - DNA, 23 bp, Homo sapiens
agctacagcacagggcacagcgg

SEQ ID NO: 1831 - DNA, 23 bp, Homo sapiens
cttccaagccagaagacagaggg

SEQ ID NO: 1832 - DNA, 23 bp, Homo sapiens
tggcggagaagctgggaccctgg

SEQ ID NO: 1833 - DNA, 23 bp, Homo sapiens
ccgcctggggctggccgggctgg

SEQ ID NO: 1834 - DNA, 23 bp, Homo sapiens
gcagtgctcctggggctcagggg

SEQ ID NO: 1835 - DNA, 23 bp, Homo sapiens
gctacagcacagggcacagcggg

SEQ ID NO: 1836 - DNA, 23 bp, Homo sapiens
ctgcagtgctcctggggctcagg

SEQ ID NO: 1837 - DNA, 23 bp, Homo sapiens
gtcctgctggctgagctccgcgg

SEQ ID NO: 1838 - DNA, 23 bp, Homo sapiens
gggctggtcctcatctccctggg

SEQ ID NO: 1839 - DNA, 23 bp, Homo sapiens
ggaccagcccggccagccccagg

SEQ ID NO: 1840 - DNA, 23 bp, Homo sapiens
ttctttccaggcctttcccaagg

SEQ ID NO: 1841 - DNA, 23 bp, Homo sapiens
ggactgtggggctgcaggaaagg

SEQ ID NO: 1842 - DNA, 23 bp, Homo sapiens
cagcaggactgtggggctgcagg

SEQ ID NO: 1843 - DNA, 23 bp, Homo sapiens
ggaaaggacagtccagcccaggg

SEQ ID NO: 1844 - DNA, 23 bp, Homo sapiens
tcttcctttcagctactccttgg

SEQ ID NO: 1845 - DNA, 23 bp, Homo sapiens
gtgaagccagctggacttcctgg

SEQ ID NO: 1846 - DNA, 23 bp, Homo sapiens
gtgctcctggggctcaggggcgg

SEQ ID NO: 1847 - DNA, 23 bp, Homo sapiens
gagaagctgggaccctgggctgg

SEQ ID NO: 1848 - DNA, 23 bp, Homo sapiens
ccagcccggccagccccaggcgg

SEQ ID NO: 1849 - DNA, 23 bp, Homo sapiens
caaagttgagggggagtcgatgg

SEQ ID NO: 1850 - DNA, 23 bp, Homo sapiens
tcgatggaggcttcaactcctgg

SEQ ID NO: 1851 - DNA, 23 bp, Homo sapiens
cgatggaggcttcaactcctggg

SEQ ID NO: 1852 - DNA, 23 bp, Homo sapiens
gactagactcctggatctgaggg

SEQ ID NO: 1853 - DNA, 23 bp, Homo sapiens
ggctgcaggactagacccctggg

SEQ ID NO: 1854 - DNA, 23 bp, Homo sapiens
gagctggaggactagactcctgg

SEQ ID NO: 1855 - DNA, 23 bp, Homo sapiens
agttgagggggagtcgatggagg

SEQ ID NO: 1856 - DNA, 23 bp, Homo sapiens
gctcccggaccccaaagtctggg

SEQ ID NO: 1857 - DNA, 23 bp, Homo sapiens
agctcccggaccccaaagtctgg

SEQ ID NO: 1858 - DNA, 23 bp, Homo sapiens
ggtccctaagtccaccccagggg

SEQ ID NO: 1859 - DNA, 23 bp, Homo sapiens
gggctgcaggactagacccctgg

SEQ ID NO: 1860 - DNA, 23 bp, Homo sapiens
cagcccctggggtggacttaggg

SEQ ID NO: 1861 - DNA, 23 bp, Homo sapiens
actctacagtctcaaagttgagg

SEQ ID NO: 1862 - DNA, 23 bp, Homo sapiens
aactttgagactgtagagtcagg

SEQ ID NO: 1863 - DNA, 23 bp, Homo sapiens
ggactagactcctggatctgagg

SEQ ID NO: 1864 - DNA, 23 bp, Homo sapiens
gtactggggcccgggaatcctgg

SEQ ID NO: 1865 - DNA, 23 bp, Homo sapiens
gactagacccctgggtctgaagg

SEQ ID NO: 1866 - DNA, 23 bp, Homo sapiens
ccggctccgcccgcagactctgg

SEQ ID NO: 1867 - DNA, 23 bp, Homo sapiens
ccagagtctgcgggcggagccgg

SEQ ID NO: 1868 - DNA, 23 bp, Homo sapiens
gagttcagggcccagactttggg

SEQ ID NO: 1869 - DNA, 23 bp, Homo sapiens
ctacagtctcaaagttgaggggg

SEQ ID NO: 1870 - DNA, 23 bp, Homo sapiens
tactggggcccgggaatcctggg

SEQ ID NO: 1871 - DNA, 23 bp, Homo sapiens
caggtccctaagtccaccccagg

SEQ ID NO: 1872 - DNA, 23 bp, Homo sapiens
cctggactgctggatcaggaagg

SEQ ID NO: 1873 - DNA, 23 bp, Homo sapiens
ggtctgagggcggaggtcctggg

SEQ ID NO: 1874 - DNA, 23 bp, Homo sapiens
cagagtctgcgggcggagccggg

SEQ ID NO: 1875 - DNA, 23 bp, Homo sapiens
aggtccctaagtccaccccaggg

SEQ ID NO: 1876 - DNA, 23 bp, Homo sapiens
tctacagtctcaaagttgagggg

SEQ ID NO: 1877 - DNA, 23 bp, Homo sapiens
tcggaggagccagagtctgcggg

SEQ ID NO: 1878 - DNA, 23 bp, Homo sapiens
ctctacagtctcaaagttgaggg

SEQ ID NO: 1879 - DNA, 23 bp, Homo sapiens
cccgggaatcctgggtctgaggg

SEQ ID NO: 1880 - DNA, 23 bp, Homo sapiens
agttcagggcccagactttgggg

SEQ ID NO: 1881 - DNA, 23 bp, Homo sapiens
tagactcctggatctgagggagg

SEQ ID NO: 1882 - DNA, 23 bp, Homo sapiens
aagtctgggccctgaactccagg

SEQ ID NO: 1883 - DNA, 23 bp, Homo sapiens
ccttcctgatccagcagtccagg

SEQ ID NO: 1884 - DNA, 23 bp, Homo sapiens
tagacccctgggtctgaaggagg

SEQ ID NO: 1885 - DNA, 23 bp, Homo sapiens
ctgcattcctggggcggaggagg

SEQ ID NO: 1886 - DNA, 23 bp, Homo sapiens
ctcctccgccccaggaatgcagg

SEQ ID NO: 1887 - DNA, 23 bp, Homo sapiens
ggggcctggactgctggatcagg

SEQ ID NO: 1888 - DNA, 23 bp, Homo sapiens
cccaggaatcctgggtctgaggg

SEQ ID NO: 1889 - DNA, 23 bp, Homo sapiens
ccagcccctggggtggacttagg

SEQ ID NO: 1890 - DNA, 23 bp, Homo sapiens
ggcctgcattcctggggcggagg

SEQ ID NO: 1891 - DNA, 23 bp, Homo sapiens
gtctgagggcggaggtcctgggg

SEQ ID NO: 1892 - DNA, 23 bp, Homo sapiens
gggtctgagggcggaggtcctgg

SEQ ID NO: 1893 - DNA, 23 bp, Homo sapiens
cctaagtccaccccaggggctgg

SEQ ID NO: 1894 - DNA, 23 bp, Homo sapiens
aggaggcgggccgggcctcaggg

SEQ ID NO: 1895 - DNA, 23 bp, Homo sapiens
gtgctggtcatcagctgggaagg

SEQ ID NO: 1896 - DNA, 23 bp, Homo sapiens
ggctggaaacctggagttcaggg

SEQ ID NO: 1897 - DNA, 23 bp, Homo sapiens
agggcccagactttggggtccgg

SEQ ID NO: 1898 - DNA, 23 bp, Homo sapiens
agctgatggcccctctctcccgg

SEQ ID NO: 1899 - DNA, 23 bp, Homo sapiens
ggagttcagggcccagactttgg

SEQ ID NO: 1900 - DNA, 23 bp, Homo sapiens
agagaggggccatcagctcccgg

SEQ ID NO: 1901 - DNA, 23 bp, Homo sapiens
ggctgggtcccaggaatcctggg

SEQ ID NO: 1902 - DNA, 23 bp, Homo sapiens
gcgggcggagccgggagagaggg

SEQ ID NO: 1903 - DNA, 23 bp, Homo sapiens
gaggagccagagtctgcgggcgg

SEQ ID NO: 1904 - DNA, 23 bp, Homo sapiens
gtcggaggagccagagtctgcgg

SEQ ID NO: 1905 - DNA, 23 bp, Homo sapiens
ggtctgagggaggaggtactggg

SEQ ID NO: 1906 - DNA, 23 bp, Homo sapiens
ggtcctggggcctgcattcctgg

SEQ ID NO: 1907 - DNA, 23 bp, Homo sapiens
ggtcatcagctgggaaggtgagg

SEQ ID NO: 1908 - DNA, 23 bp, Homo sapiens
gcctggagtcctgggtctgaggg

SEQ ID NO: 1909 - DNA, 23 bp, Homo sapiens
gggcccagactttggggtccggg

SEQ ID NO: 1910 - DNA, 23 bp, Homo sapiens
gtcctggggcctgcattcctggg

SEQ ID NO: 1911 - DNA, 23 bp, Homo sapiens
ccctcagacccaggattcccggg

SEQ ID NO: 1912 - DNA, 23 bp, Homo sapiens
tcccaggaatcctgggtctgagg

SEQ ID NO: 1913 - DNA, 23 bp, Homo sapiens
ggacctccgccctcagacccagg

SEQ ID NO: 1914 - DNA, 23 bp, Homo sapiens
cctctcctccttcagacccaggg

SEQ ID NO: 1915 - DNA, 23 bp, Homo sapiens
aggaatcctgggtctgagggagg

SEQ ID NO: 1916 - DNA, 23 bp, Homo sapiens
aactccaggtttccagcccctgg

SEQ ID NO: 1917 - DNA, 23 bp, Homo sapiens
gtctgagggaggaggtactgggg

SEQ ID NO: 1918 - DNA, 23 bp, Homo sapiens
ggactgctggatcaggaaggagg

SEQ ID NO: 1919 - DNA, 23 bp, Homo sapiens
gctcctgggtctgagggcggagg

SEQ ID NO: 1920 - DNA, 23 bp, Homo sapiens
ctttggggtccgggagctgatgg

SEQ ID NO: 1921 - DNA, 23 bp, Homo sapiens
cttcctggacccaggactccagg

SEQ ID NO: 1922 - DNA, 23 bp, Homo sapiens
caccccaggggctggaaacctgg

SEQ ID NO: 1923 - DNA, 23 bp, Homo sapiens
gcccgggaatcctgggtctgagg

SEQ ID NO: 1924 - DNA, 23 bp, Homo sapiens
gactgctggatcaggaaggaggg

SEQ ID NO: 1925 - DNA, 23 bp, Homo sapiens
actcctgggtccaggaagaaggg

SEQ ID NO: 1926 - DNA, 23 bp, Homo sapiens
tccctcagacccaggattcctgg

SEQ ID NO: 1927 - DNA, 23 bp, Homo sapiens
tccctcagacccaggattcccgg

SEQ ID NO: 1928 - DNA, 23 bp, Homo sapiens
gggtctgagggaggaggtactgg

SEQ ID NO: 1929 - DNA, 23 bp, Homo sapiens
gggctgggtcccaggaatcctgg

SEQ ID NO: 1930 - DNA, 23 bp, Homo sapiens
gcctctcctccttcagacccagg

SEQ ID NO: 1931 - DNA, 23 bp, Homo sapiens
gccccaggaatgcaggccccagg

SEQ ID NO: 1932 - DNA, 23 bp, Homo sapiens
attcctggggcggaggaggcggg

SEQ ID NO: 1933 - DNA, 23 bp, Homo sapiens
gggaatcctgggtctgagggagg

SEQ ID NO: 1934 - DNA, 23 bp, Homo sapiens
gcctgggctcctgggtctgaggg

SEQ ID NO: 1935 - DNA, 23 bp, Homo sapiens
gaggaggcgggccgggcctcagg

SEQ ID NO: 1936 - DNA, 23 bp, Homo sapiens
ctggagtcctgggtccaggaagg

SEQ ID NO: 1937 - DNA, 23 bp, Homo sapiens
ctctcctccttcagacccagggg

SEQ ID NO: 1938 - DNA, 23 bp, Homo sapiens
ccctcagacccaggattcctggg

SEQ ID NO: 1939 - DNA, 23 bp, Homo sapiens
caggtttccagcccctggggtgg

SEQ ID NO: 1940 - DNA, 23 bp, Homo sapiens
tggagtcctgggtctgagggagg

SEQ ID NO: 1941 - DNA, 23 bp, Homo sapiens
tgcgggcggagccgggagagagg

SEQ ID NO: 1942 - DNA, 23 bp, Homo sapiens
gggctggaaacctggagttcagg

SEQ ID NO: 1943 - DNA, 23 bp, Homo sapiens
ctccaggtttccagcccctgggg

SEQ ID NO: 1944 - DNA, 23 bp, Homo sapiens
cggcccgcctcctccgccccagg

SEQ ID NO: 1945 - DNA, 23 bp, Homo sapiens
cgggcggagccgggagagagggg

SEQ ID NO: 1946 - DNA, 23 bp, Homo sapiens
aactcctgggtccaggaagaagg

SEQ ID NO: 1947 - DNA, 23 bp, Homo sapiens
tggggcggaggaggcgggccggg

SEQ ID NO: 1948 - DNA, 23 bp, Homo sapiens
tccctcagacccaggactccagg

SEQ ID NO: 1949 - DNA, 23 bp, Homo sapiens
agccccttcttcctggacccagg

SEQ ID NO: 1950 - DNA, 23 bp, Homo sapiens
actcctggatctgagggaggagg

SEQ ID NO: 1951 - DNA, 23 bp, Homo sapiens
gcccctcctccctcagatccagg

SEQ ID NO: 1952 - DNA, 23 bp, Homo sapiens
aggcttcaactcctgggtccagg

SEQ ID NO: 1953 - DNA, 23 bp, Homo sapiens
actgctggatcaggaaggagggg

SEQ ID NO: 1954 - DNA, 23 bp, Homo sapiens
tgggctcctgggtctgagggcgg

SEQ ID NO: 1955 - DNA, 23 bp, Homo sapiens
tcctggggcctgcattcctgggg

SEQ ID NO: 1956 - DNA, 23 bp, Homo sapiens
gtacctcctccctcagacccagg

SEQ ID NO: 1957 - DNA, 23 bp, Homo sapiens
tgggtccaggaagaaggggctgg

SEQ ID NO: 1958 - DNA, 23 bp, Homo sapiens
ctggatcaggaaggaggggctgg

SEQ ID NO: 1959 - DNA, 23 bp, Homo sapiens
ctcctgggtccaggaagaagggg

SEQ ID NO: 1960 - DNA, 23 bp, Homo sapiens
ctcctggatctgagggaggaggg

SEQ ID NO: 1961 - DNA, 23 bp, Homo sapiens
cattcctggggcggaggaggcgg

SEQ ID NO: 1962 - DNA, 23 bp, Homo sapiens
gtcatcagctgggaaggtgaggg

SEQ ID NO: 1963 - DNA, 23 bp, Homo sapiens
ctggggcggaggaggcgggccgg

SEQ ID NO: 1964 - DNA, 23 bp, Homo sapiens
agggaggaggtactggggcccgg

SEQ ID NO: 1965 - DNA, 23 bp, Homo sapiens
actccaggtttccagcccctggg

SEQ ID NO: 1966 - DNA, 23 bp, Homo sapiens
tggatcaggaaggaggggctggg

SEQ ID NO: 1967 - DNA, 23 bp, Homo sapiens
gggaggaggtactggggcccggg

SEQ ID NO: 1968 - DNA, 23 bp, Homo sapiens
gccctcagacccaggagcccagg

SEQ ID NO: 1969 - DNA, 23 bp, Homo sapiens
ccctgggtctgaaggaggagagg

SEQ ID NO: 1970 - DNA, 23 bp, Homo sapiens
agtcctgggtccaggaaggaggg

SEQ ID NO: 1971 - DNA, 23 bp, Homo sapiens
atcctgggtctgagggaggaggg

SEQ ID NO: 1972 - DNA, 23 bp, Homo sapiens
agcccctccttcctggacccagg

SEQ ID NO: 1973 - DNA, 23 bp, Homo sapiens
aatcctgggtctgagggaggagg

SEQ ID NO: 1974 - DNA, 23 bp, Homo sapiens
aaggtgagggccctgaggcccgg

SEQ ID NO: 1975 - DNA, 23 bp, Homo sapiens
gtcctgggtccaggaaggagggg

SEQ ID NO: 1976 - DNA, 23 bp, Homo sapiens
ggtctgaaggaggagaggctggg

SEQ ID NO: 1977 - DNA, 23 bp, Homo sapiens
gggtccaggaagaaggggctggg

SEQ ID NO: 1978 - DNA, 23 bp, Homo sapiens
aggccccagccccttcttcctgg

SEQ ID NO: 1979 - DNA, 23 bp, Homo sapiens
ggctgggggcctggagtcctggg

SEQ ID NO: 1980 - DNA, 23 bp, Homo sapiens
ggcctggagtcctgggtctgagg

SEQ ID NO: 1981 - DNA, 23 bp, Homo sapiens
agtcctgggtctgagggaggagg

SEQ ID NO: 1982 - DNA, 23 bp, Homo sapiens
tgggtccaggaaggaggggctgg

SEQ ID NO: 1983 - DNA, 23 bp, Homo sapiens
tggggcctgcattcctggggcgg

SEQ ID NO: 1984 - DNA, 23 bp, Homo sapiens
ggtccaggaagaaggggctgggg

SEQ ID NO: 1985 - DNA, 23 bp, Homo sapiens
gggctgggggcctggagtcctgg

SEQ ID NO: 1986 - DNA, 23 bp, Homo sapiens
ggcctgggctcctgggtctgagg

SEQ ID NO: 1987 - DNA, 23 bp, Homo sapiens
tctgaaggaggagaggctggggg

SEQ ID NO: 1988 - DNA, 23 bp, Homo sapiens
ggggctggggcctggactgctgg

SEQ ID NO: 1989 - DNA, 23 bp, Homo sapiens
gatctgagggaggaggggctggg

SEQ ID NO: 1990 - DNA, 23 bp, Homo sapiens
gtctgaaggaggagaggctgggg

SEQ ID NO: 1991 - DNA, 23 bp, Homo sapiens
gggtctgaaggaggagaggctgg

SEQ ID NO: 1992 - DNA, 23 bp, Homo sapiens
gggcctggagtcctgggtccagg

SEQ ID NO: 1993 - DNA, 23 bp, Homo sapiens
ggctgggggcctgggctcctggg

SEQ ID NO: 1994 - DNA, 23 bp, Homo sapiens
gagtcctgggtccaggaaggagg

SEQ ID NO: 1995 - DNA, 23 bp, Homo sapiens
tcctggatctgagggaggagggg

SEQ ID NO: 1996 - DNA, 23 bp, Homo sapiens
gggtccaggaaggaggggctggg

SEQ ID NO: 1997 - DNA, 23 bp, Homo sapiens
gggaggaggggctgggtcccagg

SEQ ID NO: 1998 - DNA, 23 bp, Homo sapiens
tctgagggaggaggggctgcagg

SEQ ID NO: 1999 - DNA, 23 bp, Homo sapiens
ggaggagaggctgggggcctggg

SEQ ID NO: 2000 - DNA, 23 bp, Homo sapiens
gatcaggaaggaggggctggggg

SEQ ID NO: 2001 - DNA, 23 bp, Homo sapiens
ctgggaaggtgagggccctgagg

SEQ ID NO: 2002 - DNA, 23 bp, Homo sapiens
aggaggagaggctgggggcctgg

SEQ ID NO: 2003 - DNA, 23 bp, Homo sapiens
ggtccaggaaggaggggctgggg

SEQ ID NO: 2004 - DNA, 23 bp, Homo sapiens
aggctgggggcctgggctcctgg

SEQ ID NO: 2005 - DNA, 23 bp, Homo sapiens
gtccaggaaggaggggctggggg

SEQ ID NO: 2006 - DNA, 23 bp, Homo sapiens
ggcccccagcccctccttcctgg

SEQ ID NO: 2007 - DNA, 23 bp, Homo sapiens
gctcctcctccctcagacccagg

SEQ ID NO: 2008 - DNA, 23 bp, Homo sapiens
tctgagggaggaggagctggagg

SEQ ID NO: 2009 - DNA, 23 bp, Homo sapiens
ggatcaggaaggaggggctgggg

SEQ ID NO: 2010 - DNA, 23 bp, Homo sapiens
ggaaggaggggctgggggcctgg

SEQ ID NO: 2011 - DNA, 23 bp, Homo sapiens
gcccctcctccctcagacccagg

SEQ ID NO: 2012 - DNA, 23 bp, Homo sapiens
tcctgggtctgagggaggagggg

SEQ ID NO: 2013 - DNA, 23 bp, Homo sapiens
gggtctgagggaggaggagctgg

SEQ ID NO: 2014 - DNA, 23 bp, Homo sapiens
ggatctgagggaggaggggctgg

SEQ ID NO: 2015 - DNA, 23 bp, Homo sapiens
aggaagaaggggctggggcctgg

SEQ ID NO: 2016 - DNA, 20 bp, Artificial Sequence
  primer
ctccatcggagaaggacagc

SEQ ID NO: 2017 - DNA, 22 bp, Artificial Sequence
  primer
aggtcctgaaagtccattgtcc